European Patent Application EP 4 144 864 A1, published March 8, 2023. Title: An in vitro method for diagnosis for ischemic vascular diseases and related complications. Applicant: Prostem Cardiology B.V. The sequence listing filed with the application follows.

SEQUENCE LISTING (1348 sequences)

SEQ ID NO: 1 - DNA, 25 bp, Artificial Sequence
  >Female | AK125911 | 16928030
cattttggccaacagtcgaagacgg

SEQ ID NO: 2 - DNA, 25 bp, Artificial Sequence
  >Female | AK125911 | 16928030
cacagcttattcaagaagactccac

SEQ ID NO: 3 - DNA, 25 bp, Artificial Sequence
  >Female | AK125911 | 16928030
tgtttcacagcttattcaagaagac

SEQ ID NO: 4 - DNA, 25 bp, Artificial Sequence
  >Female | AK125911 | 16928030
tgcagagccacgatccaggcagtgg

SEQ ID NO: 5 - DNA, 25 bp, Artificial Sequence
  >Female | AK125911 | 16928030
tctcactgggttgtgggttctggcc

SEQ ID NO: 6 - DNA, 25 bp, Artificial Sequence
  >Female | AK125911 | 16928030
tggcacagcgcagtctcactgggtt

SEQ ID NO: 7 - DNA, 25 bp, Artificial Sequence
  >Female | AK125911 | 16928030
ctcttctgtcggttgcgggcactca

SEQ ID NO: 8 - DNA, 25 bp, Artificial Sequence
  >Female | AK125911 | 16928030
aggtgaggtccgtcttctcccagcg

SEQ ID NO: 9 - DNA, 25 bp, Artificial Sequence
  >Female | AK125911 | 16928030
tgtaggtgaggtccgtcttctccca

SEQ ID NO: 10 - DNA, 25 bp, Artificial Sequence
  >Female | AK125911 | 16928030
gtggcatcctagtgtcctgctccca

SEQ ID NO: 11 - DNA, 25 bp, Artificial Sequence
  >Female | AK125911 | 16928030
aggtggcatcctagtgtcctgctcc

SEQ ID NO: 12 - DNA, 25 bp, Artificial Sequence
  >Female | AK125911 | 16928030
tctttgcatgatgacggaggctctg

SEQ ID NO: 13 - DNA, 25 bp, Artificial Sequence
  >Female | AK125911 | 16928030
taaaggctgcctgagtgactgaaca

SEQ ID NO: 14 - DNA, 25 bp, Artificial Sequence
  >Female | AK125911 | 16928030
caactgccatgggaaccgaaggatc

SEQ ID NO: 15 - DNA, 25 bp, Artificial Sequence
  >Female | AK125911 | 16928030
cctcagtaaaggtgagtggcgtcac

SEQ ID NO: 16 - DNA, 25 bp, Artificial Sequence
  >Female | AK125911 | 16928030
tcatcatagtcgaagtggacatccc

SEQ ID NO: 17 - DNA, 25 bp, Artificial Sequence
  >Female | AK125911 | 16928030
tggtcatccccgatagtccaggtct

SEQ ID NO: 18 - DNA, 25 bp, Artificial Sequence
  >Female | AK125911 | 16928030
catataggtgttgaacgcccctgca

SEQ ID NO: 19 - DNA, 25 bp, Artificial Sequence
  >Female | AK125911 | 16928030
tcattggtgtctatcccagcctggg

SEQ ID NO: 20 - DNA, 25 bp, Artificial Sequence
  >Female | AK125911 | 16928030
catatgctgcagtcacagtggccag

SEQ ID NO: 21 - DNA, 25 bp, Artificial Sequence
  >Female | AK125911 | 16928030
gacacatgctgagggcatatgctgc

SEQ ID NO: 22 - DNA, 25 bp, Artificial Sequence
  >Female | AK125911 | 16928030
tttgaagaaaaagagctcgcctcgg

SEQ ID NO: 23 - DNA, 25 bp, Artificial Sequence
  >Female | AK125911 | 16928030
cgagaacctcctacctgtgcctgag

SEQ ID NO: 24 - DNA, 25 bp, Artificial Sequence
  >Female | AK125911 | 16928030
gagggttgaacgcaccaacacgagg

SEQ ID NO: 25 - DNA, 25 bp, Artificial Sequence
  >Female | AK125911 | 16928030
tctgccagttgaggatggaaatccc

SEQ ID NO: 26 - DNA, 25 bp, Artificial Sequence
  >Female | AK125911 | 16928030
tgtgaagtccctggcatctgcaatg

SEQ ID NO: 27 - DNA, 25 bp, Artificial Sequence
  >Female | AK125911 | 16928030
tctgtaaactagtgcacgggtgagg

SEQ ID NO: 28 - DNA, 25 bp, Artificial Sequence
  >Female | AK125911 | 16928030
caggactggcttttcaccgtcgtac

SEQ ID NO: 29 - DNA, 25 bp, Artificial Sequence
  >Female | AK125911 | 16928030
agaccaaggcagcatggaccgggaa

SEQ ID NO: 30 - DNA, 25 bp, Artificial Sequence
  >Female | AK125911 | 16928030
agagggcacccctctccagtcagtg

SEQ ID NO: 31 - DNA, 25 bp, Artificial Sequence
  >Female | AK125911 | 16928030
aagagccagacttcctgtggcaggc

SEQ ID NO: 32 - DNA, 25 bp, Artificial Sequence
  >Female | AK125911 | 16928030
gagccttcaccttcacagggtcaaa

SEQ ID NO: 33 - DNA, 25 bp, Artificial Sequence
  >Female | AK299689 | 17069388
gaggatcggcctgtctagttaagag

SEQ ID NO: 34 - DNA, 25 bp, Artificial Sequence
  >Female | AK299689 | 17069388
tgcgtcccactgtgcaggtctgttt

SEQ ID NO: 35 - DNA, 25 bp, Artificial Sequence
  >Female | AK299689 | 17069388
gctcgcgcccgcctttgttagtttc

SEQ ID NO: 36 - DNA, 25 bp, Artificial Sequence
  >Female | AK299689 | 17069388
ggcgctgactgccagagatcctcgt

SEQ ID NO: 37 - DNA, 25 bp, Artificial Sequence
  >Female | AK299689 | 17069388
agaggcagatgagcgagcagcgtcc

SEQ ID NO: 38 - DNA, 25 bp, Artificial Sequence
  >Female | AK299689 | 17069388
cgaggtctgtactgaatggtcccaa

SEQ ID NO: 39 - DNA, 25 bp, Artificial Sequence
  >Female | AK299689 | 17069388
gagagtccacctacttccaaataaa

SEQ ID NO: 40 - DNA, 25 bp, Artificial Sequence
  >Female | AK299689 | 17069388
tgtaatcgtccatcatgccatgggc

SEQ ID NO: 41 - DNA, 25 bp, Artificial Sequence
  >Female | AK299689 | 17069388
tactggaagtcaacgatgcagcctg

SEQ ID NO: 42 - DNA, 25 bp, Artificial Sequence
  >Female | AK299689 | 17069388
ggtctgcagtgagtacggctccaca

SEQ ID NO: 43 - DNA, 25 bp, Artificial Sequence
  >Female | AK299689 | 17069388
taacaggcatacacaaaacccacca

SEQ ID NO: 44 - DNA, 25 bp, Artificial Sequence
  >Female | AK299689 | 17069388
ggaaatactgatcacataacaggca

SEQ ID NO: 45 - DNA, 25 bp, Artificial Sequence
  >Female | AK299689 | 17069388
gagtgtgtatcaagtccacctatga

SEQ ID NO: 46 - DNA, 25 bp, Artificial Sequence
  >Female | AK299689 | 17069388
ggctttaactcaacatgatcctggt

SEQ ID NO: 47 - DNA, 25 bp, Artificial Sequence
  >Female | AK299689 | 17069388
gaagcacagtctagcctctggaagg

SEQ ID NO: 48 - DNA, 25 bp, Artificial Sequence
  >Female | AK299689 | 17069388
caaaggctgtgaccaaaatgctcca

SEQ ID NO: 49 - DNA, 25 bp, Artificial Sequence
  >Female | AK299689 | 17069388
tattcaataatttgcagcatctgga

SEQ ID NO: 50 - DNA, 25 bp, Artificial Sequence
  >Female | AK299689 | 17069388
gtctgtttggtgtaaggcgagctcc

SEQ ID NO: 51 - DNA, 25 bp, Artificial Sequence
  >Female | AK299689 | 17069388
gatgccctccccacagaaatgagtg

SEQ ID NO: 52 - DNA, 25 bp, Artificial Sequence
  >Female | BC039373 | 16779021
gtagatccagattccttttgttttc

SEQ ID NO: 53 - DNA, 25 bp, Artificial Sequence
  >Female | BC039373 | 16779021
gctagggtttcctgatggtgccaaa

SEQ ID NO: 54 - DNA, 25 bp, Artificial Sequence
  >Female | BC039373 | 16779021
gtaaaccgagacttctgtaacagac

SEQ ID NO: 55 - DNA, 25 bp, Artificial Sequence
  >Female | BC039373 | 16779021
cacttaacgtggtcttaacatggca

SEQ ID NO: 56 - DNA, 25 bp, Artificial Sequence
  >Female | BC039373 | 16779021
taagtacgtgtaagatgttagccct

SEQ ID NO: 57 - DNA, 25 bp, Artificial Sequence
  >Female | BC039373 | 16779021
caaagacattacagattggcaccac

SEQ ID NO: 58 - DNA, 25 bp, Artificial Sequence
  >Female | BC039373 | 16779021
tgaaagttctgtcccagtgagtcct

SEQ ID NO: 59 - DNA, 25 bp, Artificial Sequence
  >Female | BC039373 | 16779021
tagactgaacaaaaacggcgggtgc

SEQ ID NO: 60 - DNA, 25 bp, Artificial Sequence
  >Female | BC039373 | 16779021
gatcacagttaaccacacgccagtg

SEQ ID NO: 61 - DNA, 25 bp, Artificial Sequence
  >Female | BC039373 | 16779021
catttcggactttgaggacgcagat

SEQ ID NO: 62 - DNA, 25 bp, Artificial Sequence
  >Female | BC039373 | 16779021
tattaacccaagcacaaacaccatg

SEQ ID NO: 63 - DNA, 25 bp, Artificial Sequence
  >Female | BC039373 | 16779021
gaaaagctgtgatctgtgaccagaa

SEQ ID NO: 64 - DNA, 25 bp, Artificial Sequence
  >Female | BC039373 | 16779021
gaaatgccttctgcggtgctggcaa

SEQ ID NO: 65 - DNA, 25 bp, Artificial Sequence
  >Female | BC039373 | 16779021
gatgattctcacatgtttgctgatg

SEQ ID NO: 66 - DNA, 25 bp, Artificial Sequence
  >Female | BC039373 | 16779021
gaatgtgccacgaggaacgatgcat

SEQ ID NO: 67 - DNA, 25 bp, Artificial Sequence
  >Female | BC039373 | 16779021
tttgccatggtgaaatgtgacttcc

SEQ ID NO: 68 - DNA, 25 bp, Artificial Sequence
  >Female | BC039373 | 16779021
gtatatagtttagctctccttccag

SEQ ID NO: 69 - DNA, 25 bp, Artificial Sequence
  >Female | BC039373 | 16779021
aaatgttctcgtagtaacaggtagc

SEQ ID NO: 70 - DNA, 25 bp, Artificial Sequence
  >Female | BC039373 | 16779021
tcactttagcccaaatgctgggaaa

SEQ ID NO: 71 - DNA, 25 bp, Artificial Sequence
  >Female | BC039373 | 16779021
tagtgttccagaaaataggctttgg

SEQ ID NO: 72 - DNA, 25 bp, Artificial Sequence
  >Female | ENST00000468156 | 16861376
aagccatgaaacctctgcgcggaga

SEQ ID NO: 73 - DNA, 25 bp, Artificial Sequence
  >Female | ENST00000468156 | 16861376
agctcgcccagtccgcgaagggtaa

SEQ ID NO: 74 - DNA, 25 bp, Artificial Sequence
  >Female | ENST00000468156 | 16861376
tagttcacggttcttccaatagcgg

SEQ ID NO: 75 - DNA, 25 bp, Artificial Sequence
  >Female | ENST00000468156 | 16861376
gatgaaaacggtcaccgtgggtgcc

SEQ ID NO: 76 - DNA, 25 bp, Artificial Sequence
  >Female | ENST00000468156 | 16861376
ggctgtatcgcttctcggagcggaa

SEQ ID NO: 77 - DNA, 25 bp, Artificial Sequence
  >Female | ENST00000468156 | 16861376
tccagttccatgcaggaagcagggc

SEQ ID NO: 78 - DNA, 25 bp, Artificial Sequence
  >Female | ENST00000468156 | 16861376
cagcttgctgtagaacttgtcgtca

SEQ ID NO: 79 - DNA, 25 bp, Artificial Sequence
  >Female | ENST00000468156 | 16861376
ggcagccgtcatctacagggtagga

SEQ ID NO: 80 - DNA, 25 bp, Artificial Sequence
  >Female | ENST00000468156 | 16861376
gagtgtcccagatagagagtcctca

SEQ ID NO: 81 - DNA, 25 bp, Artificial Sequence
  >Female | ENST00000468156 | 16861376
tatctcgggtatgactgagggcaaa

SEQ ID NO: 82 - DNA, 25 bp, Artificial Sequence
  >Female | ENST00000468156 | 16861376
taatgatgggtctgtctctcgtcag

SEQ ID NO: 83 - DNA, 25 bp, Artificial Sequence
  >Female | ENST00000468156 | 16861376
gtcctcatactcaccaaggcgggcg

SEQ ID NO: 84 - DNA, 25 bp, Artificial Sequence
  >Female | ENST00000468156 | 16861376
cctctggtcgtaggcttcttgtgag

SEQ ID NO: 85 - DNA, 25 bp, Artificial Sequence
  >Female | ENST00000468156 | 16861376
cgcttcaggaaagagcggaccgtgt

SEQ ID NO: 86 - DNA, 25 bp, Artificial Sequence
  >Female | ENST00000468156 | 16861376
gttgtaccggccgagcttgctgcgc

SEQ ID NO: 87 - DNA, 25 bp, Artificial Sequence
  >Female | ENST00000468156 | 16861376
ctacatacatgacggtgccccggcg

SEQ ID NO: 88 - DNA, 25 bp, Artificial Sequence
  >Female | ENST00000468156 | 16861376
cgtggtctccgaggctccactgtgc

SEQ ID NO: 89 - DNA, 25 bp, Artificial Sequence
  >Female | ENST00000468156 | 16861376
agagcgtggtctccgaggctccact

SEQ ID NO: 90 - DNA, 25 bp, Artificial Sequence
  >Female | ENST00000468156 | 16861376
tccagggactgagatcgtttcgagt

SEQ ID NO: 91 - DNA, 25 bp, Artificial Sequence
  >Female | ENST00000468156 | 16861376
cctccagggactgagatcgtttcga

SEQ ID NO: 92 - DNA, 25 bp, Artificial Sequence
  >Female | ENST00000468156 | 16861376
ttcgaagcgcacaggccgcgtgcct

SEQ ID NO: 93 - DNA, 25 bp, Artificial Sequence
  >Female | ENST00000468156 | 16861376
gctactccttctggcgggaactctt

SEQ ID NO: 94 - DNA, 25 bp, Artificial Sequence
  >Female | ENST00000468156 | 16861376
tagccaggcttgaaatctgtgagac

SEQ ID NO: 95 - DNA, 25 bp, Artificial Sequence
  >Female | ENST00000468156 | 16861376
gacaccaatccagtagccaggcttg

SEQ ID NO: 96 - DNA, 25 bp, Artificial Sequence
  >Female | ENST00000468156 | 16861376
tttccccagtggctcatcatagcgg

SEQ ID NO: 97 - DNA, 25 bp, Artificial Sequence
  >Female | ENST00000468156 | 16861376
ggcattcgaagtagcgtttcccatt

SEQ ID NO: 98 - DNA, 25 bp, Artificial Sequence
  >Female | ENST00000468156 | 16861376
ttggcctggcattcgaagtagcgtt

SEQ ID NO: 99 - DNA, 25 bp, Artificial Sequence
  >Female | ENST00000468156 | 16861376
tgctggcttgacaaaggcgccatac

SEQ ID NO: 100 - DNA, 25 bp, Artificial Sequence
  >Female | ENST00000468156 | 16861376
taatgcatgagtctcaaaaatcaat

SEQ ID NO: 101 - DNA, 25 bp, Artificial Sequence
  >Female | ENST00000468156 | 16861376
tagtgaatttaatgcatgagtctca

SEQ ID NO: 102 - DNA, 25 bp, Artificial Sequence
  >Female | ENST00000468156 | 16861376
ctagtgaatttaatgcatgagtctc

SEQ ID NO: 103 - DNA, 25 bp, Artificial Sequence
  >Female | ENST00000493991 | 16763818
tcaggtcaggtcagccattcagtgc

SEQ ID NO: 104 - DNA, 25 bp, Artificial Sequence
  >Female | ENST00000493991 | 16763818
tgtgaccggtactcgataacagtct

SEQ ID NO: 105 - DNA, 25 bp, Artificial Sequence
  >Female | ENST00000493991 | 16763818
cagaaaaccttcatggcgtccaagg

SEQ ID NO: 106 - DNA, 25 bp, Artificial Sequence
  >Female | ENST00000493991 | 16763818
gcaaaggcggacatgtcgatgccag

SEQ ID NO: 107 - DNA, 25 bp, Artificial Sequence
  >Female | ENST00000493991 | 16763818
cattagcaccatctttgccagaggg

SEQ ID NO: 108 - DNA, 25 bp, Artificial Sequence
  >Female | ENST00000493991 | 16763818
tgcagaccagtgaagccacggtgtc

SEQ ID NO: 109 - DNA, 25 bp, Artificial Sequence
  >Female | ENST00000493991 | 16763818
tccagctggtcctgagggtcccatg

SEQ ID NO: 110 - DNA, 25 bp, Artificial Sequence
  >Female | ENST00000493991 | 16763818
tccttgcttgccagttggaccagcg

SEQ ID NO: 111 - DNA, 25 bp, Artificial Sequence
  >Female | ENST00000493991 | 16763818
gctgtctcctcgagcacctttggga

SEQ ID NO: 112 - DNA, 25 bp, Artificial Sequence
  >Female | ENST00000493991 | 16763818
taggaccagtcactccagtaggacc

SEQ ID NO: 113 - DNA, 25 bp, Artificial Sequence
  >Female | ENST00000493991 | 16763818
ttctcgccattagcaccagctgggc

SEQ ID NO: 114 - DNA, 25 bp, Artificial Sequence
  >Female | ENST00000493991 | 16763818
gctaggatcctaatgcccagcagtc

SEQ ID NO: 115 - DNA, 25 bp, Artificial Sequence
  >Female | ENST00000493991 | 16763818
tttgggcccagcgataccagctgct

SEQ ID NO: 116 - DNA, 25 bp, Artificial Sequence
  >Female | ENST00000493991 | 16763818
ggagagccacgttcacctgggaaac

SEQ ID NO: 117 - DNA, 25 bp, Artificial Sequence
  >Female | ENST00000493991 | 16763818
tgagctgagccagtgttccagagac

SEQ ID NO: 118 - DNA, 25 bp, Artificial Sequence
  >Female | ENST00000493991 | 16763818
tcttgacctgggaaaccgcggttgc

SEQ ID NO: 119 - DNA, 25 bp, Artificial Sequence
  >Female | ENST00000493991 | 16763818
ctttgaagccagcaataccaggttc

SEQ ID NO: 120 - DNA, 25 bp, Artificial Sequence
  >Female | ENST00000493991 | 16763818
cagagcctcctcaggtttcttctca

SEQ ID NO: 121 - DNA, 25 bp, Artificial Sequence
  >Female | ENST00000493991 | 16763818
tggctgaccatcgttgcctcgggca

SEQ ID NO: 122 - DNA, 25 bp, Artificial Sequence
  >Female | ENST00000493991 | 16763818
agcagggccagtccgtcctctttca

SEQ ID NO: 123 - DNA, 25 bp, Artificial Sequence
  >Female | ENST00000493991 | 16763818
cattgggcccggagatccgttctca

SEQ ID NO: 124 - DNA, 25 bp, Artificial Sequence
  >Female | ENST00000493991 | 16763818
tagcaccgtccaggcctggataacc

SEQ ID NO: 125 - DNA, 25 bp, Artificial Sequence
  >Female | ENST00000493991 | 16763818
cacaatcaaggaaggcggcagcttc

SEQ ID NO: 126 - DNA, 25 bp, Artificial Sequence
  >Female | ENST00000493991 | 16763818
gaaggacccctctagtgtctcaggc

SEQ ID NO: 127 - DNA, 25 bp, Artificial Sequence
  >Female | ENST00000493991 | 16763818
gaggcagtctttcacgtcttcacag

SEQ ID NO: 128 - DNA, 25 bp, Artificial Sequence
  >Female | ENST00000493991 | 16763818
gaatagcagggactagtctcctcca

SEQ ID NO: 129 - DNA, 25 bp, Artificial Sequence
  >Female | ENST00000493991 | 16763818
tatccctggaaacagcctggtggca

SEQ ID NO: 130 - DNA, 25 bp, Artificial Sequence
  >Female | ENST00000493991 | 16763818
tgacaccgaaggacagcggcgacga

SEQ ID NO: 131 - DNA, 25 bp, Artificial Sequence
  >Female | ENST00000531175 | 16731259
cgggacacttgtgcctggcagcgac

SEQ ID NO: 132 - DNA, 25 bp, Artificial Sequence
  >Female | ENST00000531175 | 16731259
ctgtacaatcggtggctcgcgctga

SEQ ID NO: 133 - DNA, 25 bp, Artificial Sequence
  >Female | ENST00000531175 | 16731259
gggccttccacttttcaattcaaca

SEQ ID NO: 134 - DNA, 25 bp, Artificial Sequence
  >Female | ENST00000531175 | 16731259
caactgatctgctcatgggccttcc

SEQ ID NO: 135 - DNA, 25 bp, Artificial Sequence
  >Female | ENST00000531175 | 16731259
tataattgtgcccatggccatttgg

SEQ ID NO: 136 - DNA, 25 bp, Artificial Sequence
  >Female | ENST00000531175 | 16731259
tactttcttcgaacactgctggcaa

SEQ ID NO: 137 - DNA, 25 bp, Artificial Sequence
  >Female | ENST00000531175 | 16731259
cacaagttagcaacatacaagcaca

SEQ ID NO: 138 - DNA, 25 bp, Artificial Sequence
  >Female | ENST00000531175 | 16731259
gactttcaacagatcaacatccaag

SEQ ID NO: 139 - DNA, 25 bp, Artificial Sequence
  >Female | ENST00000531175 | 16731259
tgcacatttgccttcatcccagaga

SEQ ID NO: 140 - DNA, 25 bp, Artificial Sequence
  >Female | ENST00000531175 | 16731259
tgataggctctccatattaaacggc

SEQ ID NO: 141 - DNA, 25 bp, Artificial Sequence
  >Female | ENST00000531175 | 16731259
tgagatcagccagattcataaccat

SEQ ID NO: 142 - DNA, 25 bp, Artificial Sequence
  >Female | ENST00000531175 | 16731259
ttgagatcagccagattcataacca

SEQ ID NO: 143 - DNA, 25 bp, Artificial Sequence
  >Female | ENST00000531175 | 16731259
catctgcaaagtatggcacatccat

SEQ ID NO: 144 - DNA, 25 bp, Artificial Sequence
  >Female | ENST00000531175 | 16731259
cataaggcaagatacagtgccaccc

SEQ ID NO: 145 - DNA, 25 bp, Artificial Sequence
  >Female | ENST00000531175 | 16731259
tcagaaatcacacaacaatcaaagt

SEQ ID NO: 146 - DNA, 25 bp, Artificial Sequence
  >Female | ENST00000531175 | 16731259
tataaacagctacattttcagtcgt

SEQ ID NO: 147 - DNA, 25 bp, Artificial Sequence
  >Female | ENST00000531175 | 16731259
gaagaactttctggaggttgtccca

SEQ ID NO: 148 - DNA, 25 bp, Artificial Sequence
  >Female | ENST00000531175 | 16731259
taagattcacctactcgaagtcaca

SEQ ID NO: 149 - DNA, 25 bp, Artificial Sequence
  >Female | ENST00000531175 | 16731259
tcagtggtgggaacaaggtttcctc

SEQ ID NO: 150 - DNA, 25 bp, Artificial Sequence
  >Female | ENST00000531175 | 16731259
gatgctctgggtaaacactggaagg

SEQ ID NO: 151 - DNA, 25 bp, Artificial Sequence
  >Female | ENST00000531175 | 16731259
caggccgtcatgttgggagatgctc

SEQ ID NO: 152 - DNA, 25 bp, Artificial Sequence
  >Female | ENST00000531175 | 16731259
tgctcactctgctgaagcaggccgt

SEQ ID NO: 153 - DNA, 25 bp, Artificial Sequence
  >Female | ENST00000531175 | 16731259
caccccttggatgtgtacacgacat

SEQ ID NO: 154 - DNA, 25 bp, Artificial Sequence
  >Female | ENST00000531175 | 16731259
cacagatcacgagatatatggcaga

SEQ ID NO: 155 - DNA, 25 bp, Artificial Sequence
  >Female | NM_001102398 | 16683280
taatggcactgattacagaggaatc

SEQ ID NO: 156 - DNA, 25 bp, Artificial Sequence
  >Female | NM_001102398 | 16683280
gactggtgagaaacgaagtacaccc

SEQ ID NO: 157 - DNA, 25 bp, Artificial Sequence
  >Female | NM_001102398 | 16683280
ggaaaaggtcttgcaaatgtcccta

SEQ ID NO: 158 - DNA, 25 bp, Artificial Sequence
  >Female | NM_001102398 | 16683280
tacaaggctgacataattgcccact

SEQ ID NO: 159 - DNA, 25 bp, Artificial Sequence
  >Female | NM_001102398 | 16683280
catgacatgtcaggtcagggcagcc

SEQ ID NO: 160 - DNA, 25 bp, Artificial Sequence
  >Female | NM_001102398 | 16683280
gcatatttgtatcggtctcaccagg

SEQ ID NO: 161 - DNA, 25 bp, Artificial Sequence
  >Female | NM_001102398 | 16683280
tcatgatttaacagtgtgcccagct

SEQ ID NO: 162 - DNA, 25 bp, Artificial Sequence
  >Female | NM_001102398 | 16683280
tgcaagcccaataatgtccaagagc

SEQ ID NO: 163 - DNA, 25 bp, Artificial Sequence
  >Female | NM_001102398 | 16683280
gaaccacggcctctctgctgttgag

SEQ ID NO: 164 - DNA, 25 bp, Artificial Sequence
  >Female | NM_001102398 | 16683280
tcatagccgtagtaatctggagggt

SEQ ID NO: 165 - DNA, 25 bp, Artificial Sequence
  >Female | NM_001102398 | 16683280
ggtggcttggctaagactatttcaa

SEQ ID NO: 166 - DNA, 25 bp, Artificial Sequence
  >Female | NM_001102398 | 16683280
tacgagccagacaaagattaacttc

SEQ ID NO: 167 - DNA, 25 bp, Artificial Sequence
  >Female | NM_001102398 | 16683280
tatttcttctgtcaccgtagtagcc

SEQ ID NO: 168 - DNA, 25 bp, Artificial Sequence
  >Female | NM_001102398 | 16683280
tctgtcaccgtagtagccaagtttc

SEQ ID NO: 169 - DNA, 25 bp, Artificial Sequence
  >Female | NM_001102398 | 16683280
ttacttttccactcatcagccggcg

SEQ ID NO: 170 - DNA, 25 bp, Artificial Sequence
  >Female | NM_001102398 | 16683280
ttgatgatagagaataacgtccacc

SEQ ID NO: 171 - DNA, 25 bp, Artificial Sequence
  >Female | NM_001102398 | 16683280
tcggaatggatccaacaaaaagtct

SEQ ID NO: 172 - DNA, 25 bp, Artificial Sequence
  >Female | NM_001102398 | 16683280
cactccaaggtgtttaccagggcga

SEQ ID NO: 173 - DNA, 25 bp, Artificial Sequence
  >Female | NM_001102398 | 16683280
aatgcataccctctattctgaccgg

SEQ ID NO: 174 - DNA, 25 bp, Artificial Sequence
  >Female | NM_001102398 | 16683280
taagacgtagatcccaaatgggtcc

SEQ ID NO: 175 - DNA, 25 bp, Artificial Sequence
  >Female | NM_001102398 | 16683280
caattccaggttgcacgccagagta

SEQ ID NO: 176 - DNA, 25 bp, Artificial Sequence
  >Female | NM_001102398 | 16683280
cgcttcatcaggtccctttgtggac

SEQ ID NO: 177 - DNA, 25 bp, Artificial Sequence
  >Female | NM_001102398 | 16683280
tttgtggactcttgcaccttgctcc

SEQ ID NO: 178 - DNA, 25 bp, Artificial Sequence
  >Female | NM_001102398 | 16683280
ccacttgttgatatgtgactgtatc

SEQ ID NO: 179 - DNA, 25 bp, Artificial Sequence
  >Female | NM_001102398 | 16683280
gtgactgtatctagactgtctttgc

SEQ ID NO: 180 - DNA, 25 bp, Artificial Sequence
  >Female | NM_001102398 | 16683280
ttctgaaactctgccacaagcagtt

SEQ ID NO: 181 - DNA, 25 bp, Artificial Sequence
  >Female | NM_001102398 | 16683280
agacatttctgagtaacgaccttac

SEQ ID NO: 182 - DNA, 25 bp, Artificial Sequence
  >Female | NM_001102398 | 16683280
gtagtacagacagagctccttcttc

SEQ ID NO: 183 - DNA, 25 bp, Artificial Sequence
  >Female | NM_001102398 | 16683280
tcatcaagatcgacataagctacca

SEQ ID NO: 184 - DNA, 25 bp, Artificial Sequence
  >Female | NM_001102398 | 16683280
gaggcctgcctctatcagtgtcttg

SEQ ID NO: 185 - DNA, 25 bp, Artificial Sequence
  >Female | NM_001102398 | 16683280
tgtaccgcattaccattcacctgat

SEQ ID NO: 186 - DNA, 25 bp, Artificial Sequence
  >Female | NM_001102398 | 16683280
aaaacgactagaaatggcgcgcgcg

SEQ ID NO: 187 - DNA, 25 bp, Artificial Sequence
  >Female | NM_001113490 | 17113427
taaagcctctgtcgggtaaacacca

SEQ ID NO: 188 - DNA, 25 bp, Artificial Sequence
  >Female | NM_001113490 | 17113427
ccattaatcacaagggaggccagaa

SEQ ID NO: 189 - DNA, 25 bp, Artificial Sequence
  >Female | NM_001113490 | 17113427
gagtattggagtggaacacaggccc

SEQ ID NO: 190 - DNA, 25 bp, Artificial Sequence
  >Female | NM_001113490 | 17113427
caaacgatgtggtccaggaccggta

SEQ ID NO: 191 - DNA, 25 bp, Artificial Sequence
  >Female | NM_001113490 | 17113427
cacagccggagctgaagttggtgcc

SEQ ID NO: 192 - DNA, 25 bp, Artificial Sequence
  >Female | NM_001113490 | 17113427
tcagtttgggtactgcagtctcggc

SEQ ID NO: 193 - DNA, 25 bp, Artificial Sequence
  >Female | NM_001113490 | 17113427
gacatattcagcacggtagtctcca

SEQ ID NO: 194 - DNA, 25 bp, Artificial Sequence
  >Female | NM_001113490 | 17113427
catgggtgcttatctcagggctctc

SEQ ID NO: 195 - DNA, 25 bp, Artificial Sequence
  >Female | NM_001113490 | 17113427
gaaatggacatcagagacttcgctg

SEQ ID NO: 196 - DNA, 25 bp, Artificial Sequence
  >Female | NM_001113490 | 17113427
ggcatccttctcaataatctgggca

SEQ ID NO: 197 - DNA, 25 bp, Artificial Sequence
  >Female | NM_001113490 | 17113427
gcatccttctcaataatctgggcat

SEQ ID NO: 198 - DNA, 25 bp, Artificial Sequence
  >Female | NM_001113490 | 17113427
catgtcaaggcaacgcttattggcc

SEQ ID NO: 199 - DNA, 25 bp, Artificial Sequence
  >Female | NM_001113490 | 17113427
catagctggtgttaggagagtgact

SEQ ID NO: 200 - DNA, 25 bp, Artificial Sequence
  >Female | NM_001113490 | 17113427
tattctgaaacgttggtgggctgac

SEQ ID NO: 201 - DNA, 25 bp, Artificial Sequence
  >Female | NM_001113490 | 17113427
cagtcgtgtccggagacggtgctct

SEQ ID NO: 202 - DNA, 25 bp, Artificial Sequence
  >Female | NM_001113490 | 17113427
actcagggcctgatctcggatttcg

SEQ ID NO: 203 - DNA, 25 bp, Artificial Sequence
  >Female | NM_001113490 | 17113427
ctcattggtagaacgggcagtggcc

SEQ ID NO: 204 - DNA, 25 bp, Artificial Sequence
  >Female | NM_001113490 | 17113427
caaagagctgcgagatggtttttct

SEQ ID NO: 205 - DNA, 25 bp, Artificial Sequence
  >Female | NM_001113490 | 17113427
gaaatcatgcatcctccgaatctcg

SEQ ID NO: 206 - DNA, 25 bp, Artificial Sequence
  >Female | NM_001113490 | 17113427
gaggttctcatatgcctccgagacg

SEQ ID NO: 207 - DNA, 25 bp, Artificial Sequence
  >Female | NM_001113490 | 17113427
tctggaaacaatggcaaaagggtct

SEQ ID NO: 208 - DNA, 25 bp, Artificial Sequence
  >Female | NM_001113490 | 17113427
agattgtagcaagggcaaggacccc

SEQ ID NO: 209 - DNA, 25 bp, Artificial Sequence
  >Female | NM_001113490 | 17113427
gatgctcactatagaagtgccctgg

SEQ ID NO: 210 - DNA, 25 bp, Artificial Sequence
  >Female | NM_001113490 | 17113427
taacaggtggatgggccttaactcc

SEQ ID NO: 211 - DNA, 25 bp, Artificial Sequence
  >Female | NM_001113490 | 17113427
tagaaggcagctccaacactggcat

SEQ ID NO: 212 - DNA, 25 bp, Artificial Sequence
  >Female | NM_001113490 | 17113427
gagagagagaaattgggcacctggg

SEQ ID NO: 213 - DNA, 25 bp, Artificial Sequence
  >Female | NM_001113490 | 17113427
gagagagaaattgggcacctgggct

SEQ ID NO: 214 - DNA, 25 bp, Artificial Sequence
  >Female | NM_001113490 | 17113427
aattcttgcttatgagcagctccag

SEQ ID NO: 215 - DNA, 25 bp, Artificial Sequence
  >Female | NM_001113490 | 17113427
gccaagagtccaaccactggtcact

SEQ ID NO: 216 - DNA, 25 bp, Artificial Sequence
  >Female | NM_001113490 | 17113427
tctcagccttccttctaaggagaca

SEQ ID NO: 217 - DNA, 25 bp, Artificial Sequence
  >Female | NM_001113490 | 17113427
ggagacaaaagctctttcactctgc

SEQ ID NO: 218 - DNA, 25 bp, Artificial Sequence
  >Female | NM_001113490 | 17113427
gaagacaaggtgacgactctctgct

SEQ ID NO: 219 - DNA, 25 bp, Artificial Sequence
  >Female | NM_001113490 | 17113427
gggtctaccagtttaggcagccaga

SEQ ID NO: 220 - DNA, 25 bp, Artificial Sequence
  >Female | NM_001265577 | 16845809
tcaggacattctggcggtcaggaca

SEQ ID NO: 221 - DNA, 25 bp, Artificial Sequence
  >Female | NM_001265577 | 16845809
cattcctccggttgctagggcacag

SEQ ID NO: 222 - DNA, 25 bp, Artificial Sequence
  >Female | NM_001265577 | 16845809
gaaggaaagtgacgctctgtccccg

SEQ ID NO: 223 - DNA, 25 bp, Artificial Sequence
  >Female | NM_001265577 | 16845809
tgagatgcttggcaataccctaggc

SEQ ID NO: 224 - DNA, 25 bp, Artificial Sequence
  >Female | NM_001265577 | 16845809
ctcgcaacgcgcttcttcttgcagg

SEQ ID NO: 225 - DNA, 25 bp, Artificial Sequence
  >Female | NM_001265577 | 16845809
aaactgggctttgagggaggctcct

SEQ ID NO: 226 - DNA, 25 bp, Artificial Sequence
  >Female | NM_001265577 | 16845809
atagtccgggtcacagggccagtgt

SEQ ID NO: 227 - DNA, 25 bp, Artificial Sequence
  >Female | NM_001265577 | 16845809
caaactctgtgatcatgtcgggcgt

SEQ ID NO: 228 - DNA, 25 bp, Artificial Sequence
  >Female | NM_001265577 | 16845809
tgcttagaacggtccccatccagtt

SEQ ID NO: 229 - DNA, 25 bp, Artificial Sequence
  >Female | NM_001265577 | 16845809
tgagaagtggcccacgactggcttg

SEQ ID NO: 230 - DNA, 25 bp, Artificial Sequence
  >Female | NM_001265577 | 16845809
gaagagttcccttccatggccctct

SEQ ID NO: 231 - DNA, 25 bp, Artificial Sequence
  >Female | NM_001265577 | 16845809
tggtggtcccgacttgggagatcct

SEQ ID NO: 232 - DNA, 25 bp, Artificial Sequence
  >Female | NM_001265577 | 16845809
gcatactggctgatgtgacagtcca

SEQ ID NO: 233 - DNA, 25 bp, Artificial Sequence
  >Female | NM_001265577 | 16845809
ttcgcatgggtgctggatgcccgct

SEQ ID NO: 234 - DNA, 25 bp, Artificial Sequence
  >Female | NM_001265577 | 16845809
gtgctgcgtgcggttacggttcccc

SEQ ID NO: 235 - DNA, 25 bp, Artificial Sequence
  >Female | NM_001265577 | 16845809
tccacggtggtcaggtacatgatgc

SEQ ID NO: 236 - DNA, 25 bp, Artificial Sequence
  >Female | NM_001265577 | 16845809
tgccaccccatttcaggccagggaa

SEQ ID NO: 237 - DNA, 25 bp, Artificial Sequence
  >Female | NM_001265577 | 16845809
ccatcgggctcctcagggttaaaca

SEQ ID NO: 238 - DNA, 25 bp, Artificial Sequence
  >Female | NM_001265577 | 16845809
tttcgtcggttctccgccgctggcg

SEQ ID NO: 239 - DNA, 25 bp, Artificial Sequence
  >Female | NM_015080 | 16739924
caggctgctgctcgtggaatctaga

SEQ ID NO: 240 - DNA, 25 bp, Artificial Sequence
  >Female | NM_015080 | 16739924
aaggagtcctccgtgataatgggca

SEQ ID NO: 241 - DNA, 25 bp, Artificial Sequence
  >Female | NM_015080 | 16739924
cccattgtagtagaggccggacacc

SEQ ID NO: 242 - DNA, 25 bp, Artificial Sequence
  >Female | NM_015080 | 16739924
taaagggaccttgcttcgctcactg

SEQ ID NO: 243 - DNA, 25 bp, Artificial Sequence
  >Female | NM_015080 | 16739924
cttactatggcgttgggctcgtcga

SEQ ID NO: 244 - DNA, 25 bp, Artificial Sequence
  >Female | NM_015080 | 16739924
ccacgtgtaggtgatgagcgctccc

SEQ ID NO: 245 - DNA, 25 bp, Artificial Sequence
  >Female | NM_015080 | 16739924
ggtccggagccaacaaaatcaactg

SEQ ID NO: 246 - DNA, 25 bp, Artificial Sequence
  >Female | NM_015080 | 16739924
gatcattgcagacagggcctccata

SEQ ID NO: 247 - DNA, 25 bp, Artificial Sequence
  >Female | NM_015080 | 16739924
gaacatattcttgctcagaccgcca

SEQ ID NO: 248 - DNA, 25 bp, Artificial Sequence
  >Female | NM_015080 | 16739924
tgagttccccttcatcaaggacggg

SEQ ID NO: 249 - DNA, 25 bp, Artificial Sequence
  >Female | NM_015080 | 16739924
aatgaagtcattgccgttgcccgag

SEQ ID NO: 250 - DNA, 25 bp, Artificial Sequence
  >Female | NM_015080 | 16739924
caagaacggcgtgctgcgactattc

SEQ ID NO: 251 - DNA, 25 bp, Artificial Sequence
  >Female | NM_015080 | 16739924
taataggcgatgactaaccggctgc

SEQ ID NO: 252 - DNA, 25 bp, Artificial Sequence
  >Female | NM_015080 | 16739924
taggttgatgaccagccagacagcc

SEQ ID NO: 253 - DNA, 25 bp, Artificial Sequence
  >Female | NM_015080 | 16739924
ttttgttggctggtgcacatcgccg

SEQ ID NO: 254 - DNA, 25 bp, Artificial Sequence
  >Female | NM_015080 | 16739924
gctgtttaacgtcaggtgagccgga

SEQ ID NO: 255 - DNA, 25 bp, Artificial Sequence
  >Female | NM_015080 | 16739924
tacttgacggtgctcagcgtaagcg

SEQ ID NO: 256 - DNA, 25 bp, Artificial Sequence
  >Female | NM_015690 | 16891029
tctgcggttgcctagaaacgacgct

SEQ ID NO: 257 - DNA, 25 bp, Artificial Sequence
  >Female | NM_015690 | 16891029
gctcctcaggccaagggacggattc

SEQ ID NO: 258 - DNA, 25 bp, Artificial Sequence
  >Female | NM_015690 | 16891029
tctccaatcatctccaacacgtggt

SEQ ID NO: 259 - DNA, 25 bp, Artificial Sequence
  >Female | NM_015690 | 16891029
aaaggtatccctctttgtgcaacac

SEQ ID NO: 260 - DNA, 25 bp, Artificial Sequence
  >Female | NM_015690 | 16891029
tccataagaagtatgagggagtcag

SEQ ID NO: 261 - DNA, 25 bp, Artificial Sequence
  >Female | NM_015690 | 16891029
caattttgggatgaacttcagggcc

SEQ ID NO: 262 - DNA, 25 bp, Artificial Sequence
  >Female | NM_015690 | 16891029
aatctctcgttgcaaattcctcagc

SEQ ID NO: 263 - DNA, 25 bp, Artificial Sequence
  >Female | NM_015690 | 16891029
cacaatgttgggatgccgcagaccc

SEQ ID NO: 264 - DNA, 25 bp, Artificial Sequence
  >Female | NM_015690 | 16891029
tgaaagagctctccctcagcatagt

SEQ ID NO: 265 - DNA, 25 bp, Artificial Sequence
  >Female | NM_015690 | 16891029
gtacagggctgacaccaactgggca

SEQ ID NO: 266 - DNA, 25 bp, Artificial Sequence
  >Female | NM_015690 | 16891029
tattggtgctcatagcccgggcaaa

SEQ ID NO: 267 - DNA, 25 bp, Artificial Sequence
  >Female | NM_015690 | 16891029
tcaattctgaggctaagatcccggc

SEQ ID NO: 268 - DNA, 25 bp, Artificial Sequence
  >Female | NM_015690 | 16891029
tgggaatgctcgttcacaatctggg

SEQ ID NO: 269 - DNA, 25 bp, Artificial Sequence
  >Female | NM_015690 | 16891029
gatacctagaaagacgtccgctgca

SEQ ID NO: 270 - DNA, 25 bp, Artificial Sequence
  >Female | NM_015690 | 16891029
gaacaccagtgaccaacggataggg

SEQ ID NO: 271 - DNA, 25 bp, Artificial Sequence
  >Female | NM_015690 | 16891029
tcccggcagaaggaatacaaggcaa

SEQ ID NO: 272 - DNA, 25 bp, Artificial Sequence
  >Female | NM_015690 | 16891029
gtaagaaggtcccataccaagattg

SEQ ID NO: 273 - DNA, 25 bp, Artificial Sequence
  >Female | NM_015690 | 16891029
tccagattgaaggtacaggcaaagt

SEQ ID NO: 274 - DNA, 25 bp, Artificial Sequence
  >Female | NM_015690 | 16891029
taaaaggctttggagatggcccggc

SEQ ID NO: 275 - DNA, 25 bp, Artificial Sequence
  >Female | NM_015690 | 16891029
ggcagtcccacaggagcagtgcata

SEQ ID NO: 276 - DNA, 25 bp, Artificial Sequence
  >Female | NM_015690 | 16891029
ggctgctgtcttcagttagctgatt

SEQ ID NO: 277 - DNA, 25 bp, Artificial Sequence
  >Female | NM_015690 | 16891029
cataaacagggattccaaggccagg

SEQ ID NO: 278 - DNA, 25 bp, Artificial Sequence
  >Female | NM_015690 | 16891029
cacaaggcaggttttggagccgaaa

SEQ ID NO: 279 - DNA, 25 bp, Artificial Sequence
  >Female | NM_015690 | 16891029
taaagagagtagcaacgtcactgcc

SEQ ID NO: 280 - DNA, 25 bp, Artificial Sequence
  >Female | NM_015690 | 16891029
ccatgggctggaggtcaaaggtcac

SEQ ID NO: 281 - DNA, 25 bp, Artificial Sequence
  >Female | NM_015690 | 16891029
caactacctggtggagtcaaccgaa

SEQ ID NO: 282 - DNA, 25 bp, Artificial Sequence
  >Female | NM_015690 | 16891029
gttccaaggctatcacaggcacagt

SEQ ID NO: 283 - DNA, 25 bp, Artificial Sequence
  >Female | NM_015690 | 16891029
tgtatgtctgctgaaacccagggaa

SEQ ID NO: 284 - DNA, 25 bp, Artificial Sequence
  >Female | NM_015690 | 16891029
gaaagctccccttcctgtgcagatg

SEQ ID NO: 285 - DNA, 25 bp, Artificial Sequence
  >Female | NM_015690 | 16891029
gatacttccatgctgggacaggcag

SEQ ID NO: 286 - DNA, 25 bp, Artificial Sequence
  >Female | NM_015690 | 16891029
tataaggaggtcagcatccatgtcc

SEQ ID NO: 287 - DNA, 25 bp, Artificial Sequence
  >Female | NM_015690 | 16891029
cagatgggctgcaacttctgagtcc

SEQ ID NO: 288 - DNA, 25 bp, Artificial Sequence
  >Female | NM_015690 | 16891029
tcaacggaagatggtagcagcagac

SEQ ID NO: 289 - DNA, 25 bp, Artificial Sequence
  >Female | NM_015690 | 16891029
gatagtttctcactggcacccaggg

SEQ ID NO: 290 - DNA, 25 bp, Artificial Sequence
  >Female | NM_016328 | 17047164
tgtaatcccagtaagattgccagcc

SEQ ID NO: 291 - DNA, 25 bp, Artificial Sequence
  >Female | NM_016328 | 17047164
tgatttaaacaactggccggtgggc

SEQ ID NO: 292 - DNA, 25 bp, Artificial Sequence
  >Female | NM_016328 | 17047164
gatctcgtctttgcgggtgaacgcg

SEQ ID NO: 293 - DNA, 25 bp, Artificial Sequence
  >Female | NM_016328 | 17047164
cacctcggcgttcagtttggacagc

SEQ ID NO: 294 - DNA, 25 bp, Artificial Sequence
  >Female | NM_016328 | 17047164
tccgcagaaggtacacatctgagcc

SEQ ID NO: 295 - DNA, 25 bp, Artificial Sequence
  >Female | NM_016328 | 17047164
tcatactcggctggccttcggaagg

SEQ ID NO: 296 - DNA, 25 bp, Artificial Sequence
  >Female | NM_016328 | 17047164
caacagtcggagaagtcttgggcac

SEQ ID NO: 297 - DNA, 25 bp, Artificial Sequence
  >Female | NM_016328 | 17047164
catggacgttctggatgagaggccc

SEQ ID NO: 298 - DNA, 25 bp, Artificial Sequence
  >Female | NM_016328 | 17047164
gttaaacaggatctgcacacactcc

SEQ ID NO: 299 - DNA, 25 bp, Artificial Sequence
  >Female | NM_016328 | 17047164
cacaggcaatcttccggtagggcac

SEQ ID NO: 300 - DNA, 25 bp, Artificial Sequence
  >Female | NM_016328 | 17047164
tgtgaaaattcgctcatcaaacatc

SEQ ID NO: 301 - DNA, 25 bp, Artificial Sequence
  >Female | NM_016328 | 17047164
agcaaggtcaaggacggtggcccta

SEQ ID NO: 302 - DNA, 25 bp, Artificial Sequence
  >Female | NM_016328 | 17047164
aaacttggagtacggcaccttgacg

SEQ ID NO: 303 - DNA, 25 bp, Artificial Sequence
  >Female | NM_016328 | 17047164
gacctgctcccttagtgtgttggcg

SEQ ID NO: 304 - DNA, 25 bp, Artificial Sequence
  >Female | NM_016328 | 17047164
ccaggttctgggagccgaaggtaca

SEQ ID NO: 305 - DNA, 25 bp, Artificial Sequence
  >Female | NM_016328 | 17047164
cccgagtctgttggcgtcatcttca

SEQ ID NO: 306 - DNA, 25 bp, Artificial Sequence
  >Female | NM_016328 | 17047164
tagtttataagggaccagcaccggc

SEQ ID NO: 307 - DNA, 25 bp, Artificial Sequence
  >Female | NM_016328 | 17047164
ccttggcatcattgcagatttctgc

SEQ ID NO: 308 - DNA, 25 bp, Artificial Sequence
  >Female | NM_016328 | 17047164
gagtgccggagtccaaatcggtgca

SEQ ID NO: 309 - DNA, 25 bp, Artificial Sequence
  >Female | NM_016328 | 17047164
gatgtgaattcctgcctgagtgcct

SEQ ID NO: 310 - DNA, 25 bp, Artificial Sequence
  >Female | NM_016328 | 17047164
taattaagaggtcccgggagctgca

SEQ ID NO: 311 - DNA, 25 bp, Artificial Sequence
  >Female | NM_016328 | 17047164
actaaaaggcatcgatacatatccg

SEQ ID NO: 312 - DNA, 25 bp, Artificial Sequence
  >Female | NM_144639 | 16958674
gaatgagattcatgagccctggccc

SEQ ID NO: 313 - DNA, 25 bp, Artificial Sequence
  >Female | NM_144639 | 16958674
taaaatgaggctgtggtggcaccct

SEQ ID NO: 314 - DNA, 25 bp, Artificial Sequence
  >Female | NM_144639 | 16958674
tgaggcagtgtcaccaccaaggtgc

SEQ ID NO: 315 - DNA, 25 bp, Artificial Sequence
  >Female | NM_144639 | 16958674
tggtctggcagatgatctcataggc

SEQ ID NO: 316 - DNA, 25 bp, Artificial Sequence
  >Female | NM_144639 | 16958674
cattggagacatcccagctgagcat

SEQ ID NO: 317 - DNA, 25 bp, Artificial Sequence
  >Female | NM_144639 | 16958674
gacatcccagctgagcatcagcctg

SEQ ID NO: 318 - DNA, 25 bp, Artificial Sequence
  >Female | NM_144639 | 16958674
ctccgttgtgaagggcgacccaggt

SEQ ID NO: 319 - DNA, 25 bp, Artificial Sequence
  >Female | NM_144639 | 16958674
caggcatctcccacgaagttctgca

SEQ ID NO: 320 - DNA, 25 bp, Artificial Sequence
  >Female | NM_144639 | 16958674
cgtcgtaaatgttggaggtctccct

SEQ ID NO: 321 - DNA, 25 bp, Artificial Sequence
  >Female | NM_144639 | 16958674
cacgtcatggtgatctcggctcagg

SEQ ID NO: 322 - DNA, 25 bp, Artificial Sequence
  >Female | NM_144639 | 16958674
tacaggatccttgcctgggagccca

SEQ ID NO: 323 - DNA, 25 bp, Artificial Sequence
  >Female | NM_144639 | 16958674
gatccagcggatgttgtccatgtac

SEQ ID NO: 324 - DNA, 25 bp, Artificial Sequence
  >Female | NM_144639 | 16958674
tactgcagcttcacagacaccttca

SEQ ID NO: 325 - DNA, 25 bp, Artificial Sequence
  >Female | NM_144639 | 16958674
gatgtggccagttcgtctgtgaccg

SEQ ID NO: 326 - DNA, 25 bp, Artificial Sequence
  >Female | NM_144639 | 16958674
gcacacccagcggaaaggcccaaat

SEQ ID NO: 327 - DNA, 25 bp, Artificial Sequence
  >Female | NM_144639 | 16958674
cacataggaagggtagcggaactct

SEQ ID NO: 328 - DNA, 25 bp, Artificial Sequence
  >Female | NM_144639 | 16958674
gggtagcggaactctgtcctgccag

SEQ ID NO: 329 - DNA, 25 bp, Artificial Sequence
  >Female | NM_144639 | 16958674
gcattgccgtagtcccagaagaaga

SEQ ID NO: 330 - DNA, 25 bp, Artificial Sequence
  >Female | NM_144639 | 16958674
tcctcggccaacctgttgatggctg

SEQ ID NO: 331 - DNA, 25 bp, Artificial Sequence
  >Female | NM_144639 | 16958674
caccacgttgccatggtaaccaagg

SEQ ID NO: 332 - DNA, 25 bp, Artificial Sequence
  >Female | NM_144639 | 16958674
ttgccatggtaaccaaggctgagca

SEQ ID NO: 333 - DNA, 25 bp, Artificial Sequence
  >Female | NM_144639 | 16958674
ggaaaggacacacagtcccagggca

SEQ ID NO: 334 - DNA, 25 bp, Artificial Sequence
  >Female | NM_144639 | 16958674
gcagcggtccaagctgtcagtcact

SEQ ID NO: 335 - DNA, 25 bp, Artificial Sequence
  >Female | NM_144639 | 16958674
cctgtggcgtttctcaagggctgct

SEQ ID NO: 336 - DNA, 25 bp, Artificial Sequence
  >Female | NM_144639 | 16958674
caggtaccgacgtgcagcattcaac

SEQ ID NO: 337 - DNA, 25 bp, Artificial Sequence
  >Female | NM_144639 | 16958674
acagtgccatgaacgattccctggg

SEQ ID NO: 338 - DNA, 25 bp, Artificial Sequence
  >Female | NM_144639 | 16958674
gaccgatgtagcagtagctacctgc

SEQ ID NO: 339 - DNA, 25 bp, Artificial Sequence
  >Female | NM_144639 | 16958674
aaggcaaagagcttctcatactccg

SEQ ID NO: 340 - DNA, 25 bp, Artificial Sequence
  >Female | NM_144639 | 16958674
gagcttctcatactccgtccgggag

SEQ ID NO: 341 - DNA, 25 bp, Artificial Sequence
  >Female | NM_144639 | 16958674
gaaagaggccaagtgggtgcccact

SEQ ID NO: 342 - DNA, 25 bp, Artificial Sequence
  >Female | NM_144639 | 16958674
catcttcgacaagtagaacatggtc

SEQ ID NO: 343 - DNA, 25 bp, Artificial Sequence
  >Female | NM_144639 | 16958674
taatcatgtgcatgatggcggcagc

SEQ ID NO: 344 - DNA, 25 bp, Artificial Sequence
  >Female | NM_144639 | 16958674
gggcaaaaccggtacatgtagatgt

SEQ ID NO: 345 - DNA, 25 bp, Artificial Sequence
  >Female | NM_144639 | 16958674
tgtgtccgtacagttgcagctcctg

SEQ ID NO: 346 - DNA, 25 bp, Artificial Sequence
  >Female | NM_144973 | 16762944
gataccctggatcccttcgaatgag

SEQ ID NO: 347 - DNA, 25 bp, Artificial Sequence
  >Female | NM_144973 | 16762944
catacattcgagtgatggcaggaca

SEQ ID NO: 348 - DNA, 25 bp, Artificial Sequence
  >Female | NM_144973 | 16762944
taatagcatttacgtagtggcagaa

SEQ ID NO: 349 - DNA, 25 bp, Artificial Sequence
  >Female | NM_144973 | 16762944
gaacccatggtggaaaacttgctca

SEQ ID NO: 350 - DNA, 25 bp, Artificial Sequence
  >Female | NM_144973 | 16762944
gatgctcaatctcctagccgtggtg

SEQ ID NO: 351 - DNA, 25 bp, Artificial Sequence
  >Female | NM_144973 | 16762944
cctgagttatcgtgaccaatctgaa

SEQ ID NO: 352 - DNA, 25 bp, Artificial Sequence
  >Female | NM_144973 | 16762944
tgggatgatcactgacctatacgga

SEQ ID NO: 353 - DNA, 25 bp, Artificial Sequence
  >Female | NM_144973 | 16762944
cagaaatagtccacagcattgagag

SEQ ID NO: 354 - DNA, 25 bp, Artificial Sequence
  >Female | NM_144973 | 16762944
gagaccctgagcgttggcaacataa

SEQ ID NO: 355 - DNA, 25 bp, Artificial Sequence
  >Female | NM_144973 | 16762944
taaatgtgaccacaaagccgacttc

SEQ ID NO: 356 - DNA, 25 bp, Artificial Sequence
  >Female | NM_144973 | 16762944
ggtctgacagtttgggttgcctcag

SEQ ID NO: 357 - DNA, 25 bp, Artificial Sequence
  >Female | NM_144973 | 16762944
gaagtaaagtgacagaaaccccatc

SEQ ID NO: 358 - DNA, 25 bp, Artificial Sequence
  >Female | NM_144973 | 16762944
gaaacgaaacaatcaggctgggcat

SEQ ID NO: 359 - DNA, 25 bp, Artificial Sequence
  >Female | NM_144973 | 16762944
gcaccccaggaaggtagaccacata

SEQ ID NO: 360 - DNA, 25 bp, Artificial Sequence
  >Female | NM_144973 | 16762944
gaatgctggcgaaggcgttctttcc

SEQ ID NO: 361 - DNA, 25 bp, Artificial Sequence
  >Female | NM_144973 | 16762944
tatcaatccgagtgtcaaagacccg

SEQ ID NO: 362 - DNA, 25 bp, Artificial Sequence
  >Female | NM_144973 | 16762944
caatgagctggtttatttgcttgta

SEQ ID NO: 363 - DNA, 25 bp, Artificial Sequence
  >Female | NM_144973 | 16762944
tgggtaagcataggcacagaagaat

SEQ ID NO: 364 - DNA, 25 bp, Artificial Sequence
  >Female | NM_144973 | 16762944
ggttagcaaagacctctcggagctg

SEQ ID NO: 365 - DNA, 25 bp, Artificial Sequence
  >Female | NM_144973 | 16762944
caaaagtgtggtgatgccttctgcc

SEQ ID NO: 366 - DNA, 25 bp, Artificial Sequence
  >Female | NM_144973 | 16762944
taaaatttcagtgacctccctggag

SEQ ID NO: 367 - DNA, 25 bp, Artificial Sequence
  >Female | NM_144973 | 16762944
tattctgaggatagtgggcgagaac

SEQ ID NO: 368 - DNA, 25 bp, Artificial Sequence
  >Female | NM_144973 | 16762944
gacgatctgcttctagccattggta

SEQ ID NO: 369 - DNA, 25 bp, Artificial Sequence
  >Female | NM_144973 | 16762944
tcgatcccgcacagcacgaagtagt

SEQ ID NO: 370 - DNA, 25 bp, Artificial Sequence
  >Female | NM_198082 | 16850156
caacacgtaggtgaaagcacaggca

SEQ ID NO: 371 - DNA, 25 bp, Artificial Sequence
  >Female | NM_198082 | 16850156
cagtccataatgttgtagttacgga

SEQ ID NO: 372 - DNA, 25 bp, Artificial Sequence
  >Female | NM_198082 | 16850156
ccaggtaggtgcgtgcttctggacc

SEQ ID NO: 373 - DNA, 25 bp, Artificial Sequence
  >Female | NM_198082 | 16850156
caatgggactagaacgacaggagca

SEQ ID NO: 374 - DNA, 25 bp, Artificial Sequence
  >Female | NM_198082 | 16850156
gattggcgaccatgctcctcagggt

SEQ ID NO: 375 - DNA, 25 bp, Artificial Sequence
  >Female | NM_198082 | 16850156
ccaaaggtgggctgcgatccaaagg

SEQ ID NO: 376 - DNA, 25 bp, Artificial Sequence
  >Female | NM_198082 | 16850156
gtgcatcacttctggattcctcttg

SEQ ID NO: 377 - DNA, 25 bp, Artificial Sequence
  >Female | NM_198082 | 16850156
ggcccagctctgcacggagcctgtt

SEQ ID NO: 378 - DNA, 25 bp, Artificial Sequence
  >Female | NM_198082 | 16850156
ctgaccggaggtgcaggaaaagctc

SEQ ID NO: 379 - DNA, 25 bp, Artificial Sequence
  >Female | NM_198082 | 16850156
gaaagacaaaaagagtcgctgctcc

SEQ ID NO: 380 - DNA, 25 bp, Artificial Sequence
  >Female | NM_198082 | 16850156
gaactagcgcctggaactgtggaac

SEQ ID NO: 381 - DNA, 25 bp, Artificial Sequence
  >Female | NM_198082 | 16850156
caacagtctagggtacgaagtcagg

SEQ ID NO: 382 - DNA, 25 bp, Artificial Sequence
  >Female | NM_198082 | 16850156
cctgagtgccagtccagaggatact

SEQ ID NO: 383 - DNA, 25 bp, Artificial Sequence
  >Female | NM_198082 | 16850156
cagtcgtctctgtcgaggtgcggac

SEQ ID NO: 384 - DNA, 25 bp, Artificial Sequence
  >Female | NM_198082 | 16850156
tcatctgggcaatcgcgtttcgcaa

SEQ ID NO: 385 - DNA, 25 bp, Artificial Sequence
  >Female | NM_198082 | 16850156
tggtctcgttccagggtcacggcct

SEQ ID NO: 386 - DNA, 25 bp, Artificial Sequence
  >Female | NM_198082 | 16850156
cagggcctctgacttttggatctgg

SEQ ID NO: 387 - DNA, 25 bp, Artificial Sequence
  >Female | NM_198082 | 16850156
tgagcaatttgagcatcccaggcag

SEQ ID NO: 388 - DNA, 25 bp, Artificial Sequence
  >Female | NM_198082 | 16850156
tctccttggcggtgtcagcctgtct

SEQ ID NO: 389 - DNA, 25 bp, Artificial Sequence
  >Female | NM_198082 | 16850156
tcctggttagctgcacagagtgaag

SEQ ID NO: 390 - DNA, 25 bp, Artificial Sequence
  >Female | NM_198082 | 16850156
tcctctccagctcggcgttggtggc

SEQ ID NO: 391 - DNA, 25 bp, Artificial Sequence
  >Female | NM_198082 | 16850156
tgtcagcctgcagacggaattcgtg

SEQ ID NO: 392 - DNA, 25 bp, Artificial Sequence
  >Female | NM_213596 | 16769889
tgaattcaagggctttcaccccagg

SEQ ID NO: 393 - DNA, 25 bp, Artificial Sequence
  >Female | NM_213596 | 16769889
gagaagtctcactcaacacgggcag

SEQ ID NO: 394 - DNA, 25 bp, Artificial Sequence
  >Female | NM_213596 | 16769889
gacccgtcacctgcaagtctgggaa

SEQ ID NO: 395 - DNA, 25 bp, Artificial Sequence
  >Female | NM_213596 | 16769889
tgttgatgaagtctacaggagccct

SEQ ID NO: 396 - DNA, 25 bp, Artificial Sequence
  >Female | NM_213596 | 16769889
gccggtcggagatcagcttgtccaa

SEQ ID NO: 397 - DNA, 25 bp, Artificial Sequence
  >Female | NM_213596 | 16769889
gttggccatactccggtggatggca

SEQ ID NO: 398 - DNA, 25 bp, Artificial Sequence
  >Female | NM_213596 | 16769889
ccttgcgggaggagccgctcatctt

SEQ ID NO: 399 - DNA, 25 bp, Artificial Sequence
  >Female | NM_213596 | 16769889
gagacaggttgtgccgcaccgagtt

SEQ ID NO: 400 - DNA, 25 bp, Artificial Sequence
  >Female | NM_213596 | 16769889
tcttcagggccatggcgatcagaca

SEQ ID NO: 401 - DNA, 25 bp, Artificial Sequence
  >Female | NM_213596 | 16769889
gaaagggtctcaggctgacagccca

SEQ ID NO: 402 - DNA, 25 bp, Artificial Sequence
  >Female | NM_213596 | 16769889
gggtgcagttcttgagatgaatgca

SEQ ID NO: 403 - DNA, 25 bp, Artificial Sequence
  >Female | NM_213596 | 16769889
caggtgagtacagatgcggcgggtc

SEQ ID NO: 404 - DNA, 25 bp, Artificial Sequence
  >Female | NM_213596 | 16769889
ggtcctgcaggccagatgagggctg

SEQ ID NO: 405 - DNA, 25 bp, Artificial Sequence
  >Female | NM_213596 | 16769889
gtggctcccacatgcaggtcggcca

SEQ ID NO: 406 - DNA, 25 bp, Artificial Sequence
  >Female | NM_213596 | 16769889
gtgagccacgacagcgactgcaggt

SEQ ID NO: 407 - DNA, 25 bp, Artificial Sequence
  >Female | NM_213596 | 16769889
ggtgattttgccctgagtttcgaat

SEQ ID NO: 408 - DNA, 25 bp, Artificial Sequence
  >Female | NM_213596 | 16769889
cattatggatgaggtgtcactttct

SEQ ID NO: 409 - DNA, 25 bp, Artificial Sequence
  >Female | TCONS_00015170-XLOC_007214 | 17081037
tgaaatacagttggctgctcccgct

SEQ ID NO: 410 - DNA, 25 bp, Artificial Sequence
  >Female | TCONS_00015170-XLOC_007214 | 17081037
catgctggctgctgctgtgtaataa

SEQ ID NO: 411 - DNA, 25 bp, Artificial Sequence
  >Female | TCONS_00015170-XLOC_007214 | 17081037
tggtcaagcacattcaggacatcgc

SEQ ID NO: 412 - DNA, 25 bp, Artificial Sequence
  >Female | TCONS_00015170-XLOC_007214 | 17081037
gaataatttccaacgcaaccatcca

SEQ ID NO: 413 - DNA, 25 bp, Artificial Sequence
  >Female | TCONS_00015170-XLOC_007214 | 17081037
tccaaattttgacccacagcgtgtt

SEQ ID NO: 414 - DNA, 25 bp, Artificial Sequence
  >Female | TCONS_00015170-XLOC_007214 | 17081037
ggcattgcggtgactcagttcctca

SEQ ID NO: 415 - DNA, 25 bp, Artificial Sequence
  >Female | TCONS_00015170-XLOC_007214 | 17081037
tagattaacttgtgtgaagcactga

SEQ ID NO: 416 - DNA, 25 bp, Artificial Sequence
  >Female | TCONS_00015170-XLOC_007214 | 17081037
tatggtgtctttaggtccaacctca

SEQ ID NO: 417 - DNA, 25 bp, Artificial Sequence
  >Female | TCONS_00015170-XLOC_007214 | 17081037
tctccctacatgttgtcagaaaaag

SEQ ID NO: 418 - DNA, 25 bp, Artificial Sequence
  >Female | TCONS_00015170-XLOC_007214 | 17081037
caaggtttctaacagcccagttctg

SEQ ID NO: 419 - DNA, 25 bp, Artificial Sequence
  >Female | TCONS_00015170-XLOC_007214 | 17081037
actgttttcagcttgggtgagtcac

SEQ ID NO: 420 - DNA, 25 bp, Artificial Sequence
  >Female | TCONS_00015170-XLOC_007214 | 17081037
ggcccgattacccacagaaagtaca

SEQ ID NO: 421 - DNA, 25 bp, Artificial Sequence
  >Female | TCONS_00015170-XLOC_007214 | 17081037
catcatccacatagggtctccaaaa

SEQ ID NO: 422 - DNA, 25 bp, Artificial Sequence
  >Female | TCONS_00015170-XLOC_007214 | 17081037
ggctttcctggaaccattcacaagg

SEQ ID NO: 423 - DNA, 25 bp, Artificial Sequence
  >Female | TCONS_00015170-XLOC_007214 | 17081037
ctctggccaaaaaagggtctggcac

SEQ ID NO: 424 - DNA, 25 bp, Artificial Sequence
  >Female | TCONS_00015170-XLOC_007214 | 17081037
aaaatatctccggactatggctagg

SEQ ID NO: 425 - DNA, 25 bp, Artificial Sequence
  >Female | TCONS_00015170-XLOC_007214 | 17081037
cattatgtaacagtccagggaggct

SEQ ID NO: 426 - DNA, 25 bp, Artificial Sequence
  >Female | TCONS_00015170-XLOC_007214 | 17081037
catcgctgtctgtctggagggtgcc

SEQ ID NO: 427 - DNA, 25 bp, Artificial Sequence
  >Female | TCONS_00015170-XLOC_007214 | 17081037
caccttgaatgctatcagggaagct

SEQ ID NO: 428 - DNA, 25 bp, Artificial Sequence
  >Female | TCONS_00015170-XLOC_007214 | 17081037
tgttctttgctgtccttgccagtgt

SEQ ID NO: 429 - DNA, 25 bp, Artificial Sequence
  >Female | TCONS_00015170-XLOC_007214 | 17081037
tcctgaactcacatcagaagcatgc

SEQ ID NO: 430 - DNA, 25 bp, Artificial Sequence
  >Female | TCONS_00015170-XLOC_007214 | 17081037
taagcaggtggtaccagcagggttc

SEQ ID NO: 431 - DNA, 25 bp, Artificial Sequence
  >Female | TCONS_00015170-XLOC_007214 | 17081037
ggatagcagatatttcttaaacagg

SEQ ID NO: 432 - DNA, 25 bp, Artificial Sequence
  >Female | TCONS_00015170-XLOC_007214 | 17081037
gatagcagatatttcttaaacagga

SEQ ID NO: 433 - DNA, 25 bp, Artificial Sequence
  >Female | TCONS_00015170-XLOC_007214 | 17081037
atagcagatatttcttaaacaggac

SEQ ID NO: 434 - DNA, 25 bp, Artificial Sequence
  >Female | AK094845 | 16770033
tctttgctgggaactgtggaacacc

SEQ ID NO: 435 - DNA, 25 bp, Artificial Sequence
  >Female | AK094845 | 16770033
tgaacagcccactctatgtaaaggc

SEQ ID NO: 436 - DNA, 25 bp, Artificial Sequence
  >Female | AK094845 | 16770033
cagaccgtgggctagaaagactcaa

SEQ ID NO: 437 - DNA, 25 bp, Artificial Sequence
  >Female | AK094845 | 16770033
cgccgaatgggcttgtagacacaaa

SEQ ID NO: 438 - DNA, 25 bp, Artificial Sequence
  >Female | AK094845 | 16770033
aaatgccataaggatgacagtcacc

SEQ ID NO: 439 - DNA, 25 bp, Artificial Sequence
  >Female | AK094845 | 16770033
aaacaggttacttcctaatggcagc

SEQ ID NO: 440 - DNA, 25 bp, Artificial Sequence
  >Female | AK094845 | 16770033
ggttaggcaattcatccactcactg

SEQ ID NO: 441 - DNA, 25 bp, Artificial Sequence
  >Female | AK094845 | 16770033
tgtgcaaacagctgtaaacagatcc

SEQ ID NO: 442 - DNA, 25 bp, Artificial Sequence
  >Female | AK094845 | 16770033
tgtaaacagatcctctctccagttg

SEQ ID NO: 443 - DNA, 25 bp, Artificial Sequence
  >Female | AK094845 | 16770033
tctcaagatgagtcttgacagggcc

SEQ ID NO: 444 - DNA, 25 bp, Artificial Sequence
  >Female | AK094845 | 16770033
gacagggccttttgagcaaagaagc

SEQ ID NO: 445 - DNA, 25 bp, Artificial Sequence
  >Female | AK094845 | 16770033
aaatctgctatgtttggctgggtgc

SEQ ID NO: 446 - DNA, 25 bp, Artificial Sequence
  >Female | AK094845 | 16770033
ggtgagaaatgggaactacaactga

SEQ ID NO: 447 - DNA, 25 bp, Artificial Sequence
  >Female | AK094845 | 16770033
gcgtaaccagcaacctgtcagaggt

SEQ ID NO: 448 - DNA, 25 bp, Artificial Sequence
  >Female | AK094845 | 16770033
catggttgttcttcagtctcattac

SEQ ID NO: 449 - DNA, 25 bp, Artificial Sequence
  >Female | AK094845 | 16770033
aggccaaggtacagccacggtaacg

SEQ ID NO: 450 - DNA, 25 bp, Artificial Sequence
  >Female | AK094845 | 16770033
aaggtacagccacggtaacgctgga

SEQ ID NO: 451 - DNA, 25 bp, Artificial Sequence
  >Female | AK094845 | 16770033
tacagccacggtaacgctggacgca

SEQ ID NO: 452 - DNA, 25 bp, Artificial Sequence
  >Female | AK094845 | 16770033
catggtaactgtgcgtcctggtcta

SEQ ID NO: 453 - DNA, 25 bp, Artificial Sequence
  >Female | AK094845 | 16770033
gatcaactttccgtctgtgccaacg

SEQ ID NO: 454 - DNA, 25 bp, Artificial Sequence
  >Female | AK094845 | 16770033
tagcatgtaaagtccacgagcacag

SEQ ID NO: 455 - DNA, 25 bp, Artificial Sequence
  >Female | AK094845 | 16770033
ggaagtgaaaccaaagacgggcagc

SEQ ID NO: 456 - DNA, 25 bp, Artificial Sequence
  >Female | AK094845 | 16770033
tgtaacgtatttctggcaaccacag

SEQ ID NO: 457 - DNA, 25 bp, Artificial Sequence
  >Female | AK094845 | 16770033
tagtgcagaaacctgacccaatggc

SEQ ID NO: 458 - DNA, 25 bp, Artificial Sequence
  >Female | AK094845 | 16770033
taatctgccatgttaaagacactgt

SEQ ID NO: 459 - DNA, 25 bp, Artificial Sequence
  >Female | AK094845 | 16770033
cacaggaaagcatcaatgggaggca

SEQ ID NO: 460 - DNA, 25 bp, Artificial Sequence
  >Female | AK094845 | 16770033
gcatgacttgcttccgtgtgactcg

SEQ ID NO: 461 - DNA, 25 bp, Artificial Sequence
  >Female | AK094845 | 16770033
gcattgcaggtaggatgggccccat

SEQ ID NO: 462 - DNA, 25 bp, Artificial Sequence
  >Female | AK094845 | 16770033
cagggaggatgtgcctttcagcaaa

SEQ ID NO: 463 - DNA, 25 bp, Artificial Sequence
  >Female | AK094845 | 16770033
tatgaatgaagcgagaagcttgtcc

SEQ ID NO: 464 - DNA, 25 bp, Artificial Sequence
  >Female | AK094845 | 16770033
aaggtcacatggtaaacagcagcgc

SEQ ID NO: 465 - DNA, 25 bp, Artificial Sequence
  >Female | AK094845 | 16770033
tgcatttactgttctcttggtcccg

SEQ ID NO: 466 - DNA, 25 bp, Artificial Sequence
  >Female | AK094845 | 16770033
gggtcacctccagaactgggtcatc

SEQ ID NO: 467 - DNA, 25 bp, Artificial Sequence
  >Female | AK094845 | 16770033
tcccattttgtctggtaacaggatc

SEQ ID NO: 468 - DNA, 25 bp, Artificial Sequence
  >Female | AK094845 | 16770033
tgtggttcagtagggctcacactgc

SEQ ID NO: 469 - DNA, 25 bp, Artificial Sequence
  >Female | ENST00000257359 | 16746216
ttgaaatggatccacccctgcaggt

SEQ ID NO: 470 - DNA, 25 bp, Artificial Sequence
  >Female | ENST00000257359 | 16746216
cagttgatgatagggtctgccgccc

SEQ ID NO: 471 - DNA, 25 bp, Artificial Sequence
  >Female | ENST00000257359 | 16746216
ttcctgcaggagttgcctttgcccc

SEQ ID NO: 472 - DNA, 25 bp, Artificial Sequence
  >Female | ENST00000257359 | 16746216
gcatttgtccagcttccgaggcgag

SEQ ID NO: 473 - DNA, 25 bp, Artificial Sequence
  >Female | ENST00000257359 | 16746216
gagattcccgtccatgtcagtgtaa

SEQ ID NO: 474 - DNA, 25 bp, Artificial Sequence
  >Female | ENST00000257359 | 16746216
gcatgactggtacttggctctccga

SEQ ID NO: 475 - DNA, 25 bp, Artificial Sequence
  >Female | ENST00000257359 | 16746216
tcacggtgtgaaaactgtactcctc

SEQ ID NO: 476 - DNA, 25 bp, Artificial Sequence
  >Female | ENST00000257359 | 16746216
cagtatctgtgtcactgggtggcca

SEQ ID NO: 477 - DNA, 25 bp, Artificial Sequence
  >Female | ENST00000257359 | 16746216
taatgactgtgtggcctgcatggct

SEQ ID NO: 478 - DNA, 25 bp, Artificial Sequence
  >Female | ENST00000257359 | 16746216
gaaatccggcccaaagatctgcctg

SEQ ID NO: 479 - DNA, 25 bp, Artificial Sequence
  >Female | ENST00000257359 | 16746216
gctctgtgagatacatggcgctgca

SEQ ID NO: 480 - DNA, 25 bp, Artificial Sequence
  >Female | ENST00000257359 | 16746216
catcacgtggtgcttgcccatgggc

SEQ ID NO: 481 - DNA, 25 bp, Artificial Sequence
  >Female | ENST00000257359 | 16746216
acaaatggtcccgatgtctgccaca

SEQ ID NO: 482 - DNA, 25 bp, Artificial Sequence
  >Female | ENST00000257359 | 16746216
gttgaaacgccgctgccagttgcag

SEQ ID NO: 483 - DNA, 25 bp, Artificial Sequence
  >Female | ENST00000257359 | 16746216
tgcttgtagattcgggctgccacag

SEQ ID NO: 484 - DNA, 25 bp, Artificial Sequence
  >Female | ENST00000257359 | 16746216
caaaccgcttggtcctactcgtggc

SEQ ID NO: 485 - DNA, 25 bp, Artificial Sequence
  >Female | ENST00000257359 | 16746216
ggatggtgaactcctcgccgtccag

SEQ ID NO: 486 - DNA, 25 bp, Artificial Sequence
  >Female | ENST00000257359 | 16746216
cgatcttgaactcgggcgctaggaa

SEQ ID NO: 487 - DNA, 25 bp, Artificial Sequence
  >Female | ENST00000257359 | 16746216
aagcccttgccgaaggcggacaggt

SEQ ID NO: 488 - DNA, 25 bp, Artificial Sequence
  >Female | ENST00000257359 | 16746216
gaatcaatcgggtgcaaggccgact

SEQ ID NO: 489 - DNA, 25 bp, Artificial Sequence
  >Female | ENST00000257359 | 16746216
aagaggctcgtgcactggtctcagc

SEQ ID NO: 490 - DNA, 25 bp, Artificial Sequence
  >Female | ENST00000504429 | 16972455
gatagagctatgtccacgaagggcc

SEQ ID NO: 491 - DNA, 25 bp, Artificial Sequence
  >Female | ENST00000504429 | 16972455
tcttatggttatgaggaggtagcca

SEQ ID NO: 492 - DNA, 25 bp, Artificial Sequence
  >Female | ENST00000504429 | 16972455
gtgaagcatctgttaaacacttgca

SEQ ID NO: 493 - DNA, 25 bp, Artificial Sequence
  >Female | ENST00000504429 | 16972455
ttcaaccagaaaagagagcagagtg

SEQ ID NO: 494 - DNA, 25 bp, Artificial Sequence
  >Female | ENST00000504429 | 16972455
tagccactgagaccggcgtttcgag

SEQ ID NO: 495 - DNA, 25 bp, Artificial Sequence
  >Female | ENST00000504429 | 16972455
aagtttgccgcaataacgtgagcca

SEQ ID NO: 496 - DNA, 25 bp, Artificial Sequence
  >Female | ENST00000504429 | 16972455
caaggtcttcgtagggactggtgtc

SEQ ID NO: 497 - DNA, 25 bp, Artificial Sequence
  >Female | ENST00000504429 | 16972455
caaaatcgcccaaggtcttcgtagg

SEQ ID NO: 498 - DNA, 25 bp, Artificial Sequence
  >Female | ENST00000504429 | 16972455
gaggtgcccgcacttcaaaatcgcc

SEQ ID NO: 499 - DNA, 25 bp, Artificial Sequence
  >Female | ENST00000504429 | 16972455
taaacctgctttccacagatgcccg

SEQ ID NO: 500 - DNA, 25 bp, Artificial Sequence
  >Female | ENST00000504429 | 16972455
caaccactttgtcggcggtgagcaa

SEQ ID NO: 501 - DNA, 25 bp, Artificial Sequence
  >Female | ENST00000504429 | 16972455
cagagctatcagagtgtcgcaagaa

SEQ ID NO: 502 - DNA, 25 bp, Artificial Sequence
  >Female | ENST00000504429 | 16972455
ggagaggactggtttcggttataca

SEQ ID NO: 503 - DNA, 25 bp, Artificial Sequence
  >Female | ENST00000504429 | 16972455
tagactgcgaaagtgaagatcccca

SEQ ID NO: 504 - DNA, 25 bp, Artificial Sequence
  >Female | ENST00000504429 | 16972455
tggagtcacaggcagtcgtagactg

SEQ ID NO: 505 - DNA, 25 bp, Artificial Sequence
  >Female | ENST00000504429 | 16972455
aacctatggcttgagagtggacacc

SEQ ID NO: 506 - DNA, 25 bp, Artificial Sequence
  >Female | ENST00000504429 | 16972455
gaagcagtatctggaaaggctccct

SEQ ID NO: 507 - DNA, 25 bp, Artificial Sequence
  >Female | ENST00000504429 | 16972455
tggaaagctggcgacctaaatcggg

SEQ ID NO: 508 - DNA, 25 bp, Artificial Sequence
  >Female | ENST00000504429 | 16972455
gctggtaaggacacgacactggttt

SEQ ID NO: 509 - DNA, 25 bp, Artificial Sequence
  >Female | ENST00000504429 | 16972455
gagaagggaaatccagcaaaccgct

SEQ ID NO: 510 - DNA, 25 bp, Artificial Sequence
  >Female | ENST00000504429 | 16972455
tctgctgatacaaactaggctggcc

SEQ ID NO: 511 - DNA, 25 bp, Artificial Sequence
  >Female | ENST00000504429 | 16972455
aatcacagcagctaatattgtccca

SEQ ID NO: 512 - DNA, 25 bp, Artificial Sequence
  >Female | ENST00000504429 | 16972455
tttgacaccaattgttacactatgc

SEQ ID NO: 513 - DNA, 25 bp, Artificial Sequence
  >Female | ENST00000504429 | 16972455
gattaataacggttaagttgccatg

SEQ ID NO: 514 - DNA, 25 bp, Artificial Sequence
  >Female | ENST00000504429 | 16972455
gcagtttcctgttttatttagtcca

SEQ ID NO: 515 - DNA, 25 bp, Artificial Sequence
  >Female | ENST00000504429 | 16972455
gaatgttctatgagcacttgggtct

SEQ ID NO: 516 - DNA, 25 bp, Artificial Sequence
  >Female | ENST00000504429 | 16972455
tctaagggttcaagaacatgggctc

SEQ ID NO: 517 - DNA, 25 bp, Artificial Sequence
  >Female | ENST00000504429 | 16972455
tgcaggcagtatcatggcagccact

SEQ ID NO: 518 - DNA, 25 bp, Artificial Sequence
  >Female | ENST00000504429 | 16972455
ccagaacgggtgtatgaggcgctaa

SEQ ID NO: 519 - DNA, 25 bp, Artificial Sequence
  >Female | NM_001142553 | 16980805
aatgagcccaatctcgagttgctgg

SEQ ID NO: 520 - DNA, 25 bp, Artificial Sequence
  >Female | NM_001142553 | 16980805
catcagtttccccagataggcagga

SEQ ID NO: 521 - DNA, 25 bp, Artificial Sequence
  >Female | NM_001142553 | 16980805
gagtcagcactgaataccccacagg

SEQ ID NO: 522 - DNA, 25 bp, Artificial Sequence
  >Female | NM_001142553 | 16980805
tgagtcacaattacaccaggcaaag

SEQ ID NO: 523 - DNA, 25 bp, Artificial Sequence
  >Female | NM_001142553 | 16980805
tacagtcgtattagaaagcctgggc

SEQ ID NO: 524 - DNA, 25 bp, Artificial Sequence
  >Female | NM_001142553 | 16980805
tggtgagctcgtaatctagaatcgc

SEQ ID NO: 525 - DNA, 25 bp, Artificial Sequence
  >Female | NM_001142553 | 16980805
tagagcacagggaaagaactccatc

SEQ ID NO: 526 - DNA, 25 bp, Artificial Sequence
  >Female | NM_001142553 | 16980805
catgtgaatgaccaagagacccgtg

SEQ ID NO: 527 - DNA, 25 bp, Artificial Sequence
  >Female | NM_001142553 | 16980805
tattgccagcatccatatcagaggc

SEQ ID NO: 528 - DNA, 25 bp, Artificial Sequence
  >Female | NM_001142553 | 16980805
aattcaaatgaagcacctggcatga

SEQ ID NO: 529 - DNA, 25 bp, Artificial Sequence
  >Female | NM_001142553 | 16980805
ggtgtgccatcatccagtgccagaa

SEQ ID NO: 530 - DNA, 25 bp, Artificial Sequence
  >Female | NM_001142553 | 16980805
cattgaagacatacaccagggttcc

SEQ ID NO: 531 - DNA, 25 bp, Artificial Sequence
  >Female | NM_001142553 | 16980805
aaattgggaggcagatctagagaac

SEQ ID NO: 532 - DNA, 25 bp, Artificial Sequence
  >Female | NM_001142553 | 16980805
tttcccttcagaggcataggtctag

SEQ ID NO: 533 - DNA, 25 bp, Artificial Sequence
  >Female | NM_001142553 | 16980805
tcagtaactgagacgtaaaccgcca

SEQ ID NO: 534 - DNA, 25 bp, Artificial Sequence
  >Female | NM_001142553 | 16980805
aagtctgtcccactaaaggcagcag

SEQ ID NO: 535 - DNA, 25 bp, Artificial Sequence
  >Female | NM_001142553 | 16980805
cattttgcaagaatccgtcctcggg

SEQ ID NO: 536 - DNA, 25 bp, Artificial Sequence
  >Female | NM_001142553 | 16980805
gagcagagaccatcaacgaaagtgt

SEQ ID NO: 537 - DNA, 25 bp, Artificial Sequence
  >Female | NM_001142553 | 16980805
gccttagcagaggtaaaaacatctc

SEQ ID NO: 538 - DNA, 25 bp, Artificial Sequence
  >Female | NM_001142553 | 16980805
tccaggtccacacgaacaaaggctt

SEQ ID NO: 539 - DNA, 25 bp, Artificial Sequence
  >Female | NM_001142553 | 16980805
tcaccagggctaaatgtgtcattct

SEQ ID NO: 540 - DNA, 25 bp, Artificial Sequence
  >Female | NM_001142553 | 16980805
tcatgagggtcgatccggaatgcct

SEQ ID NO: 541 - DNA, 25 bp, Artificial Sequence
  >Female | NM_001142553 | 16980805
tgaacactatagcaccccagagctc

SEQ ID NO: 542 - DNA, 25 bp, Artificial Sequence
  >Female | NM_001142553 | 16980805
tacacctcatatacacaggcatcag

SEQ ID NO: 543 - DNA, 25 bp, Artificial Sequence
  >Female | NM_001142553 | 16980805
gattttgacaaaggcaacttgagca

SEQ ID NO: 544 - DNA, 25 bp, Artificial Sequence
  >Female | NM_001142553 | 16980805
caaaagatggtccacactctgcggt

SEQ ID NO: 545 - DNA, 25 bp, Artificial Sequence
  >Female | NM_001142553 | 16980805
gacccacatgactacagtgccaggg

SEQ ID NO: 546 - DNA, 25 bp, Artificial Sequence
  >Female | NM_001142553 | 16980805
tcattgaggtcagcgacccggagta

SEQ ID NO: 547 - DNA, 25 bp, Artificial Sequence
  >Female | NM_001142553 | 16980805
tccgtggccaccagtagtaactcat

SEQ ID NO: 548 - DNA, 25 bp, Artificial Sequence
  >Female | NM_001142553 | 16980805
cacgtgaattgctggccggttgtca

SEQ ID NO: 549 - DNA, 25 bp, Artificial Sequence
  >Female | NM_001142553 | 16980805
ctgtagcgcacgaagccattgggcc

SEQ ID NO: 550 - DNA, 25 bp, Artificial Sequence
  >Female | NM_001142553 | 16980805
gtcctgctcaaagaccggcgggttg

SEQ ID NO: 551 - DNA, 25 bp, Artificial Sequence
  >Female | NM_001142553 | 16980805
tccggtagcgcaactggaagaacgg

SEQ ID NO: 552 - DNA, 25 bp, Artificial Sequence
  >Female | NM_001142553 | 16980805
tgcacgtggaagtcgtccagcagcg

SEQ ID NO: 553 - DNA, 25 bp, Artificial Sequence
  >Female | NM_001142553 | 16980805
ggagtcctccgacagaaagaagccg

SEQ ID NO: 554 - DNA, 25 bp, Artificial Sequence
  >Female | NM_001142553 | 16980805
ggatgtcacctaccagcgtgtccgg

SEQ ID NO: 555 - DNA, 25 bp, Artificial Sequence
  >Female | NM_001142553 | 16980805
cagcttgtggcaggatcgcagaaaa

SEQ ID NO: 556 - DNA, 25 bp, Artificial Sequence
  >Female | NM_001142553 | 16980805
catctgcaactggtgaaagcgtcct

SEQ ID NO: 557 - DNA, 25 bp, Artificial Sequence
  >Female | NM_001142553 | 16980805
ggagattatatgaagcgcgcacaca

SEQ ID NO: 558 - DNA, 25 bp, Artificial Sequence
  >Female | NM_003211 | 16756127
cctgggcccgatggctggcagtacc

SEQ ID NO: 559 - DNA, 25 bp, Artificial Sequence
  >Female | NM_003211 | 16756127
tggaaacgtataaaaagcttgagct

SEQ ID NO: 560 - DNA, 25 bp, Artificial Sequence
  >Female | NM_003211 | 16756127
actgccatattaggagcttcagcca

SEQ ID NO: 561 - DNA, 25 bp, Artificial Sequence
  >Female | NM_003211 | 16756127
cagacagtctaaatttggagcccac

SEQ ID NO: 562 - DNA, 25 bp, Artificial Sequence
  >Female | NM_003211 | 16756127
tcaggtctccacaggcatcattcag

SEQ ID NO: 563 - DNA, 25 bp, Artificial Sequence
  >Female | NM_003211 | 16756127
ccatatggttcagctggacctcact

SEQ ID NO: 564 - DNA, 25 bp, Artificial Sequence
  >Female | NM_003211 | 16756127
agagatctttgctgccgggcgtggt

SEQ ID NO: 565 - DNA, 25 bp, Artificial Sequence
  >Female | NM_003211 | 16756127
tggagagatctttgctgccgggcgt

SEQ ID NO: 566 - DNA, 25 bp, Artificial Sequence
  >Female | NM_003211 | 16756127
gctcagcttgaactagatacatatg

SEQ ID NO: 567 - DNA, 25 bp, Artificial Sequence
  >Female | NM_003211 | 16756127
gtaatttctgtactagaatacgtcc

SEQ ID NO: 568 - DNA, 25 bp, Artificial Sequence
  >Female | NM_003211 | 16756127
tgtaatttctgtactagaatacgtc

SEQ ID NO: 569 - DNA, 25 bp, Artificial Sequence
  >Female | NM_003211 | 16756127
tacattgcccataatgttagcaaag

SEQ ID NO: 570 - DNA, 25 bp, Artificial Sequence
  >Female | NM_003211 | 16756127
cgaggaaactgagcacatcttgcac

SEQ ID NO: 571 - DNA, 25 bp, Artificial Sequence
  >Female | NM_003211 | 16756127
gtatattgcacctcttgaacgtcca

SEQ ID NO: 572 - DNA, 25 bp, Artificial Sequence
  >Female | NM_003211 | 16756127
gctgcatggattttctccgtaagca

SEQ ID NO: 573 - DNA, 25 bp, Artificial Sequence
  >Female | NM_003211 | 16756127
ttagcccatttgaagagaagccaca

SEQ ID NO: 574 - DNA, 25 bp, Artificial Sequence
  >Female | NM_003211 | 16756127
ggaggaaaatgcaactaggatggcc

SEQ ID NO: 575 - DNA, 25 bp, Artificial Sequence
  >Female | NM_003211 | 16756127
taaaatagttaagcaagcttccgga

SEQ ID NO: 576 - DNA, 25 bp, Artificial Sequence
  >Female | NM_003211 | 16756127
cccgggatcgaggagaggcatatat

SEQ ID NO: 577 - DNA, 25 bp, Artificial Sequence
  >Female | NM_003211 | 16756127
gagccaccgtatcagcttatttgaa

SEQ ID NO: 578 - DNA, 25 bp, Artificial Sequence
  >Female | NM_003211 | 16756127
tgcccattaggaatgccactgaaag

SEQ ID NO: 579 - DNA, 25 bp, Artificial Sequence
  >Female | NM_003211 | 16756127
taaatgactgggtcatccactgccc

SEQ ID NO: 580 - DNA, 25 bp, Artificial Sequence
  >Female | NM_003211 | 16756127
taagcagagctgagaagcaccattc

SEQ ID NO: 581 - DNA, 25 bp, Artificial Sequence
  >Female | NM_003211 | 16756127
ctgccaccccagagtagttaattgg

SEQ ID NO: 582 - DNA, 25 bp, Artificial Sequence
  >Female | NM_024638 | 16944179
ccagtgcagagccaatcagggagta

SEQ ID NO: 583 - DNA, 25 bp, Artificial Sequence
  >Female | NM_024638 | 16944179
cactaccacgtgttgcaaaattctc

SEQ ID NO: 584 - DNA, 25 bp, Artificial Sequence
  >Female | NM_024638 | 16944179
ttttatctcagaggtgtcggcgacg

SEQ ID NO: 585 - DNA, 25 bp, Artificial Sequence
  >Female | NM_024638 | 16944179
tttcagcagaggctagtcgaaaggg

SEQ ID NO: 586 - DNA, 25 bp, Artificial Sequence
  >Female | NM_024638 | 16944179
gatttatctttgctccatgggccat

SEQ ID NO: 587 - DNA, 25 bp, Artificial Sequence
  >Female | NM_024638 | 16944179
ggaaccccgtggatattatgcagcg

SEQ ID NO: 588 - DNA, 25 bp, Artificial Sequence
  >Female | NM_024638 | 16944179
ctggatcgtgcagggagcagtacaa

SEQ ID NO: 589 - DNA, 25 bp, Artificial Sequence
  >Female | NM_024638 | 16944179
tctgagggatacaccataggctgac

SEQ ID NO: 590 - DNA, 25 bp, Artificial Sequence
  >Female | NM_024638 | 16944179
tctccatcggagaggcactggaacc

SEQ ID NO: 591 - DNA, 25 bp, Artificial Sequence
  >Female | NM_024638 | 16944179
tgcagccgcagacagttatccaaga

SEQ ID NO: 592 - DNA, 25 bp, Artificial Sequence
  >Female | NM_024638 | 16944179
gccgcttggctgtctctcgtgctga

SEQ ID NO: 593 - DNA, 25 bp, Artificial Sequence
  >Female | NM_024638 | 16944179
caagcgtagtctagcctccagggtt

SEQ ID NO: 594 - DNA, 25 bp, Artificial Sequence
  >Female | NM_024638 | 16944179
gaataagaacagtgacatgaggaca

SEQ ID NO: 595 - DNA, 25 bp, Artificial Sequence
  >Female | NM_024638 | 16944179
tggccgactaacaccagatatgagc

SEQ ID NO: 596 - DNA, 25 bp, Artificial Sequence
  >Female | NM_024638 | 16944179
taatcaaaactgaaagtcagggcac

SEQ ID NO: 597 - DNA, 25 bp, Artificial Sequence
  >Female | NM_024638 | 16944179
tgatcagataagaagtggccattgg

SEQ ID NO: 598 - DNA, 25 bp, Artificial Sequence
  >Female | NM_024638 | 16944179
tcttggttgcaaccagttgtttcaa

SEQ ID NO: 599 - DNA, 25 bp, Artificial Sequence
  >Female | NM_024638 | 16944179
ccttcagattaatttcaaatgatgt

SEQ ID NO: 600 - DNA, 25 bp, Artificial Sequence
  >Female | NM_024638 | 16944179
tcttctgacaagacgaagtctacaa

SEQ ID NO: 601 - DNA, 25 bp, Artificial Sequence
  >Female | NM_024638 | 16944179
tggctccagtcttctgacaagacga

SEQ ID NO: 602 - DNA, 25 bp, Artificial Sequence
  >Female | NM_024638 | 16944179
cagcagatggtggatgtatgcccga

SEQ ID NO: 603 - DNA, 25 bp, Artificial Sequence
  >Female | NM_024638 | 16944179
cactttttagtgcttcccggatgta

SEQ ID NO: 604 - DNA, 25 bp, Artificial Sequence
  >Female | NM_024638 | 16944179
ctctaatcgttaggccaggcagggc

SEQ ID NO: 605 - DNA, 25 bp, Artificial Sequence
  >Female | NM_033637 | 16708482
tgagtgccttctcttgcagcaccgc

SEQ ID NO: 606 - DNA, 25 bp, Artificial Sequence
  >Female | NM_033637 | 16708482
gtttctccagagagcttcctccgct

SEQ ID NO: 607 - DNA, 25 bp, Artificial Sequence
  >Female | NM_033637 | 16708482
ggttatacaggcatcgcagcgaagg

SEQ ID NO: 608 - DNA, 25 bp, Artificial Sequence
  >Female | NM_033637 | 16708482
tggaaagctgtgagtgcgccagtcc

SEQ ID NO: 609 - DNA, 25 bp, Artificial Sequence
  >Female | NM_033637 | 16708482
caaggttggatggtgcaacagagcc

SEQ ID NO: 610 - DNA, 25 bp, Artificial Sequence
  >Female | NM_033637 | 16708482
ggttcgccattattacagtcttctc

SEQ ID NO: 611 - DNA, 25 bp, Artificial Sequence
  >Female | NM_033637 | 16708482
gggttcgccattattacagtcttct

SEQ ID NO: 612 - DNA, 25 bp, Artificial Sequence
  >Female | NM_033637 | 16708482
tggtttaagcagagtctggcacagc

SEQ ID NO: 613 - DNA, 25 bp, Artificial Sequence
  >Female | NM_033637 | 16708482
tctcagtcttcatagcagtgcttgc

SEQ ID NO: 614 - DNA, 25 bp, Artificial Sequence
  >Female | NM_033637 | 16708482
tgagagtttccgttgcttgggcaca

SEQ ID NO: 615 - DNA, 25 bp, Artificial Sequence
  >Female | NM_033637 | 16708482
taagatacgagtttatgtgcccatg

SEQ ID NO: 616 - DNA, 25 bp, Artificial Sequence
  >Female | NM_033637 | 16708482
tcagcaatatgatccaatccccgag

SEQ ID NO: 617 - DNA, 25 bp, Artificial Sequence
  >Female | NM_033637 | 16708482
tcttccacagcatgccatcagaggt

SEQ ID NO: 618 - DNA, 25 bp, Artificial Sequence
  >Female | NM_033637 | 16708482
cacttcggcagtgaattctctgtaa

SEQ ID NO: 619 - DNA, 25 bp, Artificial Sequence
  >Female | NM_033637 | 16708482
tgttgtctcgaaggccgcttactat

SEQ ID NO: 620 - DNA, 25 bp, Artificial Sequence
  >Female | NM_033637 | 16708482
tatggcctgtgagaattcgcttgca

SEQ ID NO: 621 - DNA, 25 bp, Artificial Sequence
  >Female | NM_033637 | 16708482
tgaccgtggaatccgatgatcctgt

SEQ ID NO: 622 - DNA, 25 bp, Artificial Sequence
  >Female | NM_033637 | 16708482
gaacgatctttggagcaggtcacca

SEQ ID NO: 623 - DNA, 25 bp, Artificial Sequence
  >Female | NM_033637 | 16708482
tagtgttgtcagatgagccactcac

SEQ ID NO: 624 - DNA, 25 bp, Artificial Sequence
  >Female | NM_033637 | 16708482
tggccttctaacactcgtaaacatg

SEQ ID NO: 625 - DNA, 25 bp, Artificial Sequence
  >Female | NM_033637 | 16708482
gaatacaacgcaccaattcctcatg

SEQ ID NO: 626 - DNA, 25 bp, Artificial Sequence
  >Female | NM_033637 | 16708482
gcagccacaagatcccacactttaa

SEQ ID NO: 627 - DNA, 25 bp, Artificial Sequence
  >Female | NM_033637 | 16708482
caagggtccgtagacagagtgtccc

SEQ ID NO: 628 - DNA, 25 bp, Artificial Sequence
  >Female | NM_033637 | 16708482
tagtcgaaaaactcttccggaatgc

SEQ ID NO: 629 - DNA, 25 bp, Artificial Sequence
  >Female | NM_033637 | 16708482
cagctggatcatttaggaagtccca

SEQ ID NO: 630 - DNA, 25 bp, Artificial Sequence
  >Female | NM_033637 | 16708482
caagtatgaggtcagtgtatggtta

SEQ ID NO: 631 - DNA, 25 bp, Artificial Sequence
  >Female | NM_033637 | 16708482
ctgggcaagtatgaggtcagtgtat

SEQ ID NO: 632 - DNA, 25 bp, Artificial Sequence
  >Female | NM_033637 | 16708482
cccaaacggcaggagaaagttccat

SEQ ID NO: 633 - DNA, 25 bp, Artificial Sequence
  >Female | NM_033637 | 16708482
gactaggcttaccacacaagtagga

SEQ ID NO: 634 - DNA, 25 bp, Artificial Sequence
  >Female | NM_033637 | 16708482
tcttggcaaagatacaggcacctgg

SEQ ID NO: 635 - DNA, 25 bp, Artificial Sequence
  >Female | NM_033637 | 16708482
tagattggagagcaaaaccctgggc

SEQ ID NO: 636 - DNA, 25 bp, Artificial Sequence
  >Female | NM_033655 | 17094394
gaagtgccaggagttcagtccacgc

SEQ ID NO: 637 - DNA, 25 bp, Artificial Sequence
  >Female | NM_033655 | 17094394
tcacgatgatagagacagccacagc

SEQ ID NO: 638 - DNA, 25 bp, Artificial Sequence
  >Female | NM_033655 | 17094394
gtaactttctctgttgatagatgcg

SEQ ID NO: 639 - DNA, 25 bp, Artificial Sequence
  >Female | NM_033655 | 17094394
tatggctatggcagtgatgcaaagc

SEQ ID NO: 640 - DNA, 25 bp, Artificial Sequence
  >Female | NM_033655 | 17094394
taaagcgataatgacaagcaccagg

SEQ ID NO: 641 - DNA, 25 bp, Artificial Sequence
  >Female | NM_033655 | 17094394
caccaggtcattcagggccttgtta

SEQ ID NO: 642 - DNA, 25 bp, Artificial Sequence
  >Female | NM_033655 | 17094394
ctccgatgacagcagagtctcttct

SEQ ID NO: 643 - DNA, 25 bp, Artificial Sequence
  >Female | NM_033655 | 17094394
tctgtctgcattaaccaagggctct

SEQ ID NO: 644 - DNA, 25 bp, Artificial Sequence
  >Female | NM_033655 | 17094394
cgagaggcagccagtgaagccacta

SEQ ID NO: 645 - DNA, 25 bp, Artificial Sequence
  >Female | NM_033655 | 17094394
agccagtgaagccactagtcgccgc

SEQ ID NO: 646 - DNA, 25 bp, Artificial Sequence
  >Female | NM_033655 | 17094394
gatggctggctctctgcaagtaaca

SEQ ID NO: 647 - DNA, 25 bp, Artificial Sequence
  >Female | NM_033655 | 17094394
tccggaggattacagaaaagcgact

SEQ ID NO: 648 - DNA, 25 bp, Artificial Sequence
  >Female | NM_033655 | 17094394
tctgagtatatacttcgttgctgaa

SEQ ID NO: 649 - DNA, 25 bp, Artificial Sequence
  >Female | NM_033655 | 17094394
tgcctttgaatacaccatccttgaa

SEQ ID NO: 650 - DNA, 25 bp, Artificial Sequence
  >Female | NM_033655 | 17094394
gaaacaacaggcaaagcagggcttg

SEQ ID NO: 651 - DNA, 25 bp, Artificial Sequence
  >Female | NM_033655 | 17094394
gattatatgtacactcaggcaagag

SEQ ID NO: 652 - DNA, 25 bp, Artificial Sequence
  >Female | NM_033655 | 17094394
tcccaatatgagagatttgacggcg

SEQ ID NO: 653 - DNA, 25 bp, Artificial Sequence
  >Female | NM_033655 | 17094394
ggcgttgaattctgtccctgaggac

SEQ ID NO: 654 - DNA, 25 bp, Artificial Sequence
  >Female | NM_033655 | 17094394
ttagatgtcccatgagaagcaaaca

SEQ ID NO: 655 - DNA, 25 bp, Artificial Sequence
  >Female | NM_033655 | 17094394
taagcaattcctatgatgccatcag

SEQ ID NO: 656 - DNA, 25 bp, Artificial Sequence
  >Female | NM_033655 | 17094394
cataatggaaggatctataattggc

SEQ ID NO: 657 - DNA, 25 bp, Artificial Sequence
  >Female | NM_033655 | 17094394
catgaaaaagatggaactggctgtt

SEQ ID NO: 658 - DNA, 25 bp, Artificial Sequence
  >Female | NM_033655 | 17094394
tgaaacataaaaccaagcactgctg

SEQ ID NO: 659 - DNA, 25 bp, Artificial Sequence
  >Female | NM_033655 | 17094394
tgacttatggaagagcagcactgaa

SEQ ID NO: 660 - DNA, 25 bp, Artificial Sequence
  >Female | NM_033655 | 17094394
ttgacttttgcatttgtgggattac

SEQ ID NO: 661 - DNA, 25 bp, Artificial Sequence
  >Female | NM_033655 | 17094394
catgaccacggcttcttctctgtta

SEQ ID NO: 662 - DNA, 25 bp, Artificial Sequence
  >Female | NM_033655 | 17094394
ggtgaagttgcccatcagccatgtt

SEQ ID NO: 663 - DNA, 25 bp, Artificial Sequence
  >Female | NM_033655 | 17094394
tacagcaataagctcggagttcgtg

SEQ ID NO: 664 - DNA, 25 bp, Artificial Sequence
  >Female | NM_033655 | 17094394
tatgtcattgaggagccagttgcga

SEQ ID NO: 665 - DNA, 25 bp, Artificial Sequence
  >Female | NM_152891 | 16823203
tcagggtgctgccagaatccagtgc

SEQ ID NO: 666 - DNA, 25 bp, Artificial Sequence
  >Female | NM_152891 | 16823203
aattggtttgcccatcactgcgtgc

SEQ ID NO: 667 - DNA, 25 bp, Artificial Sequence
  >Female | NM_152891 | 16823203
gagtcagagctggtgatccccaaag

SEQ ID NO: 668 - DNA, 25 bp, Artificial Sequence
  >Female | NM_152891 | 16823203
agaagctgacgcgagcctgaatcca

SEQ ID NO: 669 - DNA, 25 bp, Artificial Sequence
  >Female | NM_152891 | 16823203
tatatgtggccacactggtgtagac

SEQ ID NO: 670 - DNA, 25 bp, Artificial Sequence
  >Female | NM_152891 | 16823203
cactggtgtagacccctggacggtt

SEQ ID NO: 671 - DNA, 25 bp, Artificial Sequence
  >Female | NM_152891 | 16823203
agactgcaggcaggtcagaggtccc

SEQ ID NO: 672 - DNA, 25 bp, Artificial Sequence
  >Female | NM_152891 | 16823203
aggcagcacaatgcgctcagcctgg

SEQ ID NO: 673 - DNA, 25 bp, Artificial Sequence
  >Female | NM_152891 | 16823203
agcggcacccttactccttgtagcg

SEQ ID NO: 674 - DNA, 25 bp, Artificial Sequence
  >Female | NM_152891 | 16823203
gcggcacccttactccttgtagcgg

SEQ ID NO: 675 - DNA, 25 bp, Artificial Sequence
  >Female | NM_152891 | 16823203
gcacccttactccttgtagcggtcg

SEQ ID NO: 676 - DNA, 25 bp, Artificial Sequence
  >Female | NM_152891 | 16823203
ccttgtagcggtcgccactctggga

SEQ ID NO: 677 - DNA, 25 bp, Artificial Sequence
  >Female | NM_152891 | 16823203
cccagccggtgacccggcatggtgt

SEQ ID NO: 678 - DNA, 25 bp, Artificial Sequence
  >Female | NM_152891 | 16823203
aggcgcacgcggtactcagctggca

SEQ ID NO: 679 - DNA, 25 bp, Artificial Sequence
  >Female | NM_152891 | 16823203
gcgcacgcggtactcagctggcagt

SEQ ID NO: 680 - DNA, 25 bp, Artificial Sequence
  >Female | NM_152891 | 16823203
cgcacgcggtactcagctggcagtg

SEQ ID NO: 681 - DNA, 25 bp, Artificial Sequence
  >Female | NM_152891 | 16823203
gcggtactcagctggcagtgccctc

SEQ ID NO: 682 - DNA, 25 bp, Artificial Sequence
  >Female | NM_152891 | 16823203
cacgtgtgccccacgatgctggatg

SEQ ID NO: 683 - DNA, 25 bp, Artificial Sequence
  >Female | NM_152891 | 16823203
tgtgccccacgatgctggatgctcg

SEQ ID NO: 684 - DNA, 25 bp, Artificial Sequence
  >Female | NM_152891 | 16823203
acgatgctggatgctcgcctgccac

SEQ ID NO: 685 - DNA, 25 bp, Artificial Sequence
  >Female | NM_152891 | 16823203
ccaacgatccgactggacatgcggg

SEQ ID NO: 686 - DNA, 25 bp, Artificial Sequence
  >Male | ENST00000440123 | 16708531
ttttttaaaagctgcgtcacatgca

SEQ ID NO: 687 - DNA, 25 bp, Artificial Sequence
  >Male | ENST00000440123 | 16708531
cttttttaaaagctgcgtcacatgc

SEQ ID NO: 688 - DNA, 25 bp, Artificial Sequence
  >Male | ENST00000440123 | 16708531
ccttttttaaaagctgcgtcacatg

SEQ ID NO: 689 - DNA, 25 bp, Artificial Sequence
  >Male | ENST00000440123 | 16708531
ggagagagatacaccacactgccca

SEQ ID NO: 690 - DNA, 25 bp, Artificial Sequence
  >Male | ENST00000440123 | 16708531
tggagagagatacaccacactgccc

SEQ ID NO: 691 - DNA, 25 bp, Artificial Sequence
  >Male | ENST00000440123 | 16708531
gtggagagagatacaccacactgcc

SEQ ID NO: 692 - DNA, 25 bp, Artificial Sequence
  >Male | ENST00000440123 | 16708531
ggtggagagagatacaccacactgc

SEQ ID NO: 693 - DNA, 25 bp, Artificial Sequence
  >Male | ENST00000440123 | 16708531
gggtggagagagatacaccacactg

SEQ ID NO: 694 - DNA, 25 bp, Artificial Sequence
  >Male | ENST00000440123 | 16708531
cagcctagggtagggacgcgaaaca

SEQ ID NO: 695 - DNA, 25 bp, Artificial Sequence
  >Male | ENST00000440123 | 16708531
atccagcctagggtagggacgcgaa

SEQ ID NO: 696 - DNA, 25 bp, Artificial Sequence
  >Male | ENST00000440123 | 16708531
catccagcctagggtagggacgcga

SEQ ID NO: 697 - DNA, 25 bp, Artificial Sequence
  >Male | ENST00000440123 | 16708531
ccatccagcctagggtagggacgcg

SEQ ID NO: 698 - DNA, 25 bp, Artificial Sequence
  >Male | ENST00000440123 | 16708531
tctccgaagccctcaaaggacagca

SEQ ID NO: 699 - DNA, 25 bp, Artificial Sequence
  >Male | ENST00000440123 | 16708531
atctccgaagccctcaaaggacagc

SEQ ID NO: 700 - DNA, 25 bp, Artificial Sequence
  >Male | ENST00000440123 | 16708531
catctccgaagccctcaaaggacag

SEQ ID NO: 701 - DNA, 25 bp, Artificial Sequence
  >Male | ENST00000440123 | 16708531
tcatctccgaagccctcaaaggaca

SEQ ID NO: 702 - DNA, 25 bp, Artificial Sequence
  >Male | ENST00000440123 | 16708531
tctcatctccgaagccctcaaagga

SEQ ID NO: 703 - DNA, 25 bp, Artificial Sequence
  >Male | ENST00000440123 | 16708531
ttctcatctccgaagccctcaaagg

SEQ ID NO: 704 - DNA, 25 bp, Artificial Sequence
  >Male | TCONS_00025321-XLOC_012127 | 16831561
atgccctccttattaactcatcaca

SEQ ID NO: 705 - DNA, 25 bp, Artificial Sequence
  >Male | TCONS_00025321-XLOC_012127 | 16831561
ggccaggacccgagctcattctgca

SEQ ID NO: 706 - DNA, 25 bp, Artificial Sequence
  >Male | TCONS_00025321-XLOC_012127 | 16831561
acagtgctggccagatgtcccatgg

SEQ ID NO: 707 - DNA, 25 bp, Artificial Sequence
  >Male | TCONS_00025321-XLOC_012127 | 16831561
atgatcccatggaaagatgggctcc

SEQ ID NO: 708 - DNA, 25 bp, Artificial Sequence
  >Male | TCONS_00025321-XLOC_012127 | 16831561
gaaggactctaatgatcccatggaa

SEQ ID NO: 709 - DNA, 25 bp, Artificial Sequence
  >Male | TCONS_00025321-XLOC_012127 | 16831561
caacagctgcaagagaaggactcta

SEQ ID NO: 710 - DNA, 25 bp, Artificial Sequence
  >Male | TCONS_00025321-XLOC_012127 | 16831561
ccaacagctgcaagagaaggactct

SEQ ID NO: 711 - DNA, 25 bp, Artificial Sequence
  >Male | TCONS_00025321-XLOC_012127 | 16831561
gtccacacatcattcctgtctgcga

SEQ ID NO: 712 - DNA, 25 bp, Artificial Sequence
  >Male | TCONS_00025321-XLOC_012127 | 16831561
agtccacacatcattcctgtctgcg

SEQ ID NO: 713 - DNA, 25 bp, Artificial Sequence
  >Male | TCONS_00025321-XLOC_012127 | 16831561
gcaagtccacacatcattcctgtct

SEQ ID NO: 714 - DNA, 25 bp, Artificial Sequence
  >Male | TCONS_00025321-XLOC_012127 | 16831561
ggcaagtccacacatcattcctgtc

SEQ ID NO: 715 - DNA, 25 bp, Artificial Sequence
  >Male | TCONS_00025321-XLOC_012127 | 16831561
tggcaagtccacacatcattcctgt

SEQ ID NO: 716 - DNA, 25 bp, Artificial Sequence
  >Male | TCONS_00025321-XLOC_012127 | 16831561
atggcaagtccacacatcattcctg

SEQ ID NO: 717 - DNA, 25 bp, Artificial Sequence
  >Male | TCONS_00025321-XLOC_012127 | 16831561
catggcaagtccacacatcattcct

SEQ ID NO: 718 - DNA, 25 bp, Artificial Sequence
  >Male | TCONS_00025321-XLOC_012127 | 16831561
caccatggcaagtccacacatcatt

SEQ ID NO: 719 - DNA, 25 bp, Artificial Sequence
  >Male | TCONS_00025321-XLOC_012127 | 16831561
acaccatggcaagtccacacatcat

SEQ ID NO: 720 - DNA, 25 bp, Artificial Sequence
  >Male | TCONS_00025321-XLOC_012127 | 16831561
tgcacaccatggcaagtccacacat

SEQ ID NO: 721 - DNA, 25 bp, Artificial Sequence
  >Male | TCONS_00025321-XLOC_012127 | 16831561
gctcatgcacaccatggcaagtcca

SEQ ID NO: 722 - DNA, 25 bp, Artificial Sequence
  >Male | TCONS_00025321-XLOC_012127 | 16831561
ggctcatgcacaccatggcaagtcc

SEQ ID NO: 723 - DNA, 25 bp, Artificial Sequence
  >Male | ENST00000488290 | 16712992
ccagcccttcttggatgggcagagg

SEQ ID NO: 724 - DNA, 25 bp, Artificial Sequence
  >Male | ENST00000488290 | 16712992
cagcccttcttggatgggcagaggt

SEQ ID NO: 725 - DNA, 25 bp, Artificial Sequence
  >Male | ENST00000488290 | 16712992
cccttcttggatgggcagaggttac

SEQ ID NO: 726 - DNA, 25 bp, Artificial Sequence
  >Male | ENST00000488290 | 16712992
tcttggatgggcagaggttacagtc

SEQ ID NO: 727 - DNA, 25 bp, Artificial Sequence
  >Male | ENST00000488290 | 16712992
tggatgggcagaggttacagtctcc

SEQ ID NO: 728 - DNA, 25 bp, Artificial Sequence
  >Male | ENST00000488290 | 16712992
ggatgggcagaggttacagtctcct

SEQ ID NO: 729 - DNA, 25 bp, Artificial Sequence
  >Male | ENST00000488290 | 16712992
gatgggcagaggttacagtctcctt

SEQ ID NO: 730 - DNA, 25 bp, Artificial Sequence
  >Male | ENST00000488290 | 16712992
atgggcagaggttacagtctccttc

SEQ ID NO: 731 - DNA, 25 bp, Artificial Sequence
  >Male | ENST00000488290 | 16712992
ggcagaggttacagtctccttcagc

SEQ ID NO: 732 - DNA, 25 bp, Artificial Sequence
  >Male | ENST00000488290 | 16712992
gaggttacagtctccttcagcttgc

SEQ ID NO: 733 - DNA, 25 bp, Artificial Sequence
  >Male | ENST00000430988 | 16895114
taatcaaagtttgaaggcagccgca

SEQ ID NO: 734 - DNA, 25 bp, Artificial Sequence
  >Male | ENST00000430988 | 16895114
tgaaggcagccgcatttcctcaggc

SEQ ID NO: 735 - DNA, 25 bp, Artificial Sequence
  >Male | ENST00000430988 | 16895114
gctcaacatcgctgcctgggtggac

SEQ ID NO: 736 - DNA, 25 bp, Artificial Sequence
  >Male | ENST00000430988 | 16895114
tgtgcccagctgttggtggcgctca

SEQ ID NO: 737 - DNA, 25 bp, Artificial Sequence
  >Male | ENST00000430988 | 16895114
gtgcatgccatcatagccttcctgg

SEQ ID NO: 738 - DNA, 25 bp, Artificial Sequence
  >Male | ENST00000430988 | 16895114
catcatagccttcctggtgcaggga

SEQ ID NO: 739 - DNA, 25 bp, Artificial Sequence
  >Male | ENST00000430988 | 16895114
cctgtaagcaccatcaacatccaga

SEQ ID NO: 740 - DNA, 25 bp, Artificial Sequence
  >Male | ENST00000430988 | 16895114
gagaagattccatgcgtctttcggg

SEQ ID NO: 741 - DNA, 25 bp, Artificial Sequence
  >Male | ENST00000430988 | 16895114
aagattccatgcgtctttcgggagc

SEQ ID NO: 742 - DNA, 25 bp, Artificial Sequence
  >Male | ENST00000430988 | 16895114
tgcgtctttcgggagcttgcctaaa

SEQ ID NO: 743 - DNA, 25 bp, Artificial Sequence
  >Male | ENST00000430988 | 16895114
gcgtctttcgggagcttgcctaaac

SEQ ID NO: 744 - DNA, 25 bp, Artificial Sequence
  >Male | ENST00000430988 | 16895114
cgtctttcgggagcttgcctaaaca

SEQ ID NO: 745 - DNA, 25 bp, Artificial Sequence
  >Male | ENST00000430988 | 16895114
tctttcgggagcttgcctaaacacc

SEQ ID NO: 746 - DNA, 25 bp, Artificial Sequence
  >Male | ENST00000430988 | 16895114
ctttcgggagcttgcctaaacacca

SEQ ID NO: 747 - DNA, 25 bp, Artificial Sequence
  >Male | ENST00000430988 | 16895114
tttcgggagcttgcctaaacaccac

SEQ ID NO: 748 - DNA, 25 bp, Artificial Sequence
  >Male | ENST00000430988 | 16895114
caccagcgttgctctgtcatgtgaa

SEQ ID NO: 749 - DNA, 25 bp, Artificial Sequence
  >Male | ENST00000430988 | 16895114
gacacctcagtgtcgtaggtagcgg

SEQ ID NO: 750 - DNA, 25 bp, Artificial Sequence
  >Male | ENST00000430988 | 16895114
taggtagcggagatgcaagtgttcc

SEQ ID NO: 751 - DNA, 25 bp, Artificial Sequence
  >Male | ENST00000430988 | 16895114
tttctcggaaaaggaagccgatgct

SEQ ID NO: 752 - DNA, 25 bp, Artificial Sequence
  >Male | ENST00000430988 | 16895114
ttctcggaaaaggaagccgatgctg

SEQ ID NO: 753 - DNA, 25 bp, Artificial Sequence
  >Male | ENST00000430988 | 16895114
ttctattacaccaaacccagagcgg

SEQ ID NO: 754 - DNA, 25 bp, Artificial Sequence
  >Male | ENST00000430988 | 16895114
tctattacaccaaacccagagcggg

SEQ ID NO: 755 - DNA, 25 bp, Artificial Sequence
  >Male | ENST00000430988 | 16895114
tattacaccaaacccagagcgggca

SEQ ID NO: 756 - DNA, 25 bp, Artificial Sequence
  >Male | ENST00000430988 | 16895114
aagagactacagaagcacaggcgcc

SEQ ID NO: 757 - DNA, 25 bp, Artificial Sequence
  >Male | ENST00000430988 | 16895114
tacagaagcacaggcgcctgctggg

SEQ ID NO: 758 - DNA, 25 bp, Artificial Sequence
  >Male | ENST00000440657 | 16773468
gcagacatttaaacgttaccattca

SEQ ID NO: 759 - DNA, 25 bp, Artificial Sequence
  >Male | ENST00000440657 | 16773468
gcagcagacatttaaacgttaccat

SEQ ID NO: 760 - DNA, 25 bp, Artificial Sequence
  >Male | ENST00000440657 | 16773468
tagcagcagacatttaaacgttacc

SEQ ID NO: 761 - DNA, 25 bp, Artificial Sequence
  >Male | ENST00000440657 | 16773468
ttccgtagcagcagacatttaaacg

SEQ ID NO: 762 - DNA, 25 bp, Artificial Sequence
  >Male | ENST00000440657 | 16773468
gcttccgtagcagcagacatttaaa

SEQ ID NO: 763 - DNA, 25 bp, Artificial Sequence
  >Male | ENST00000440657 | 16773468
tgcttccgtagcagcagacatttaa

SEQ ID NO: 764 - DNA, 25 bp, Artificial Sequence
  >Male | ENST00000440657 | 16773468
tcttgcttccgtagcagcagacatt

SEQ ID NO: 765 - DNA, 25 bp, Artificial Sequence
  >Male | ENST00000440657 | 16773468
gaattttcttgcttccgtagcagca

SEQ ID NO: 766 - DNA, 25 bp, Artificial Sequence
  >Male | ENST00000440657 | 16773468
ccacacagggagtgaattttcttgc

SEQ ID NO: 767 - DNA, 25 bp, Artificial Sequence
  >Male | ENST00000440657 | 16773468
aacagaacacttctcagaatcagca

SEQ ID NO: 768 - DNA, 25 bp, Artificial Sequence
  >Male | ENST00000440657 | 16773468
tgggctggacttaaacagaacactt

SEQ ID NO: 769 - DNA, 25 bp, Artificial Sequence
  >Male | ENST00000440657 | 16773468
gatgggctggacttaaacagaacac

SEQ ID NO: 770 - DNA, 25 bp, Artificial Sequence
  >Male | ENST00000440657 | 16773468
gagaagatgggctggacttaaacag

SEQ ID NO: 771 - DNA, 25 bp, Artificial Sequence
  >Male | ENST00000440657 | 16773468
ggagtaccaagttctgcattcagta

SEQ ID NO: 772 - DNA, 25 bp, Artificial Sequence
  >Male | ENST00000440657 | 16773468
tggagtaccaagttctgcattcagt

SEQ ID NO: 773 - DNA, 25 bp, Artificial Sequence
  >Male | ENST00000440657 | 16773468
gatctggagtaccaagttctgcatt

SEQ ID NO: 774 - DNA, 25 bp, Artificial Sequence
  >Male | ENST00000440657 | 16773468
catttacttctgcagtttgatctgg

SEQ ID NO: 775 - DNA, 25 bp, Artificial Sequence
  >Male | ProbSetID_17118935 | 17118935
aggattacacacctcgcaaaccgct

SEQ ID NO: 776 - DNA, 25 bp, Artificial Sequence
  >Male | ProbSetID_17118935 | 17118935
taggattacacacctcgcaaaccgc

SEQ ID NO: 777 - DNA, 25 bp, Artificial Sequence
  >Male | ProbSetID_17118935 | 17118935
ctaggattacacacctcgcaaaccg

SEQ ID NO: 778 - DNA, 25 bp, Artificial Sequence
  >Male | ProbSetID_17118935 | 17118935
actaggattacacacctcgcaaacc

SEQ ID NO: 779 - DNA, 25 bp, Artificial Sequence
  >Male | ProbSetID_17118935 | 17118935
aactaggattacacacctcgcaaac

SEQ ID NO: 780 - DNA, 25 bp, Artificial Sequence
  >Male | ProbSetID_17118935 | 17118935
taactaggattacacacctcgcaaa

SEQ ID NO: 781 - DNA, 25 bp, Artificial Sequence
  >Male | ProbSetID_17118935 | 17118935
gtaactaggattacacacctcgcaa

SEQ ID NO: 782 - DNA, 25 bp, Artificial Sequence
  >Male | NM_007117 | 16945454
aaccaatgtagaacgcagacgggcg

SEQ ID NO: 783 - DNA, 25 bp, Artificial Sequence
  >Male | NM_007117 | 16945454
acacggagacgacggagaaacacag

SEQ ID NO: 784 - DNA, 25 bp, Artificial Sequence
  >Male | NM_007117 | 16945454
tagagggcgagacaaagaccgagat

SEQ ID NO: 785 - DNA, 25 bp, Artificial Sequence
  >Male | NM_007117 | 16945454
cgattaaacacaggcgcacgagaga

SEQ ID NO: 786 - DNA, 25 bp, Artificial Sequence
  >Male | NM_007117 | 16945454
gatctgttgacgagaacacgcgtgt

SEQ ID NO: 787 - DNA, 25 bp, Artificial Sequence
  >Male | NM_007117 | 16945454
tccgcagtcggcaggtcaggagtct

SEQ ID NO: 788 - DNA, 25 bp, Artificial Sequence
  >Male | NM_007117 | 16945454
cggtcaggttcagggtcaaagccag

SEQ ID NO: 789 - DNA, 25 bp, Artificial Sequence
  >Male | NM_007117 | 16945454
caccggtcaggttcagggtcaaagc

SEQ ID NO: 790 - DNA, 25 bp, Artificial Sequence
  >Male | NM_007117 | 16945454
cctggatgctgacgtttggagagcc

SEQ ID NO: 791 - DNA, 25 bp, Artificial Sequence
  >Male | NM_007117 | 16945454
tgtgctgggttacatcgactgacca

SEQ ID NO: 792 - DNA, 25 bp, Artificial Sequence
  >Male | NM_007117 | 16945454
ctgccgcttcgggacagcatatgca

SEQ ID NO: 793 - DNA, 25 bp, Artificial Sequence
  >Male | NM_007117 | 16945454
tttgagccttgggatctgccagcct

SEQ ID NO: 794 - DNA, 25 bp, Artificial Sequence
  >Male | NM_007117 | 16945454
gcgtttttcaggcatcaggtcttcc

SEQ ID NO: 795 - DNA, 25 bp, Artificial Sequence
  >Male | NM_007117 | 16945454
cagaaggcccgcttgaccataggct

SEQ ID NO: 796 - DNA, 25 bp, Artificial Sequence
  >Male | NM_007117 | 16945454
cgaccagggtgctgccgcttttcct

SEQ ID NO: 797 - DNA, 25 bp, Artificial Sequence
  >Male | NM_007117 | 16945454
ttagaccacaaactcgacttcaggg

SEQ ID NO: 798 - DNA, 25 bp, Artificial Sequence
  >Male | NM_007117 | 16945454
gctcaggcttatggtcagggatcta

SEQ ID NO: 799 - DNA, 25 bp, Artificial Sequence
  >Male | NM_007117 | 16945454
cagaaggaccatcttagccaaggct

SEQ ID NO: 800 - DNA, 25 bp, Artificial Sequence
  >Male | NM_007117 | 16945454
tggaagctggatttgcacacaacgc

SEQ ID NO: 801 - DNA, 25 bp, Artificial Sequence
  >Male | NM_007117 | 16945454
gtttacacatggagaatcctgccag

SEQ ID NO: 802 - DNA, 25 bp, Artificial Sequence
  >Male | NM_007117 | 16945454
tccaagcagtaacacagctgtgggt

SEQ ID NO: 803 - DNA, 25 bp, Artificial Sequence
  >Male | NM_007117 | 16945454
tacaaaccacaattcctaggcgatg

SEQ ID NO: 804 - DNA, 25 bp, Artificial Sequence
  >Male | XR_109422 | 16848054
ggtgtgtgagcactataggacctat

SEQ ID NO: 805 - DNA, 25 bp, Artificial Sequence
  >Male | XR_109422 | 16848054
taggcagcctgtaattgtcatcacc

SEQ ID NO: 806 - DNA, 25 bp, Artificial Sequence
  >Male | XR_109422 | 16848054
cctatggacagagggattaagaact

SEQ ID NO: 807 - DNA, 25 bp, Artificial Sequence
  >Male | XR_109422 | 16848054
taatcaccaagatccccagaattgt

SEQ ID NO: 808 - DNA, 25 bp, Artificial Sequence
  >Male | XR_109422 | 16848054
taggtggtccgagacattctgctga

SEQ ID NO: 809 - DNA, 25 bp, Artificial Sequence
  >Male | XR_109422 | 16848054
tctgctgattggacatagacaggct

SEQ ID NO: 810 - DNA, 25 bp, Artificial Sequence
  >Male | XR_109422 | 16848054
agtggtatggtaagtcaatttctcc

SEQ ID NO: 811 - DNA, 25 bp, Artificial Sequence
  >Male | XR_109422 | 16848054
tgtctcgggctttctgtccatttgg

SEQ ID NO: 812 - DNA, 25 bp, Artificial Sequence
  >Male | XR_109422 | 16848054
tgataacgtagagtggttcttccca

SEQ ID NO: 813 - DNA, 25 bp, Artificial Sequence
  >Male | XR_109422 | 16848054
taacgtagagtggttcttcccatgg

SEQ ID NO: 814 - DNA, 25 bp, Artificial Sequence
  >Male | XR_109422 | 16848054
aacgtagagtggttcttcccatgga

SEQ ID NO: 815 - DNA, 25 bp, Artificial Sequence
  >Male | XR_109422 | 16848054
gaaaagcccacataatctctggctg

SEQ ID NO: 816 - DNA, 25 bp, Artificial Sequence
  >Male | XR_109422 | 16848054
cctcagcgttgttcccgtgacttca

SEQ ID NO: 817 - DNA, 25 bp, Artificial Sequence
  >Male | XR_109422 | 16848054
tttttctttggcagatcgttccaca

SEQ ID NO: 818 - DNA, 25 bp, Artificial Sequence
  >Male | XR_109422 | 16848054
ttctttggcagatcgttccacaagg

SEQ ID NO: 819 - DNA, 25 bp, Artificial Sequence
  >Male | XR_109422 | 16848054
tctttggcagatcgttccacaaggc

SEQ ID NO: 820 - DNA, 25 bp, Artificial Sequence
  >Male | XR_109422 | 16848054
ctttggcagatcgttccacaaggcc

SEQ ID NO: 821 - DNA, 25 bp, Artificial Sequence
  >Male | XR_109422 | 16848054
tttggcagatcgttccacaaggcca

SEQ ID NO: 822 - DNA, 25 bp, Artificial Sequence
  >Male | XR_109422 | 16848054
ttggcagatcgttccacaaggccat

SEQ ID NO: 823 - DNA, 25 bp, Artificial Sequence
  >Male | XR_109422 | 16848054
tttatattcgaccactccctagacc

SEQ ID NO: 824 - DNA, 25 bp, Artificial Sequence
  >Male | ENST00000456944 | 17095583
tcagggaaagaggtacaatgcaatc

SEQ ID NO: 825 - DNA, 25 bp, Artificial Sequence
  >Male | ENST00000456944 | 17095583
tgcaatcagtagaaaggtcaccaga

SEQ ID NO: 826 - DNA, 25 bp, Artificial Sequence
  >Male | ENST00000456944 | 17095583
tacggtcattaccacgacaaaggga

SEQ ID NO: 827 - DNA, 25 bp, Artificial Sequence
  >Male | ENST00000456944 | 17095583
gagcacagaatttccagcaggcagg

SEQ ID NO: 828 - DNA, 25 bp, Artificial Sequence
  >Male | ENST00000456944 | 17095583
tccagcaggcaggatgcatccacag

SEQ ID NO: 829 - DNA, 25 bp, Artificial Sequence
  >Male | ENST00000456944 | 17095583
ccagcagaggccgtgagaaaagcct

SEQ ID NO: 830 - DNA, 25 bp, Artificial Sequence
  >Male | ENST00000456944 | 17095583
tcttgttagtaaatgcagcctgtct

SEQ ID NO: 831 - DNA, 25 bp, Artificial Sequence
  >Male | ENST00000456944 | 17095583
taaatgcagcctgtcttaatactgc

SEQ ID NO: 832 - DNA, 25 bp, Artificial Sequence
  >Male | ENST00000456944 | 17095583
tatgcattgtttccatccccaaatg

SEQ ID NO: 833 - DNA, 25 bp, Artificial Sequence
  >Male | ENST00000456944 | 17095583
gaacttgtgattaaaggtccatgca

SEQ ID NO: 834 - DNA, 25 bp, Artificial Sequence
  >Male | ENST00000456944 | 17095583
tgattaaaggtccatgcaacccaga

SEQ ID NO: 835 - DNA, 25 bp, Artificial Sequence
  >Male | ENST00000456944 | 17095583
gattaaaggtccatgcaacccagaa

SEQ ID NO: 836 - DNA, 25 bp, Artificial Sequence
  >Male | ENST00000456944 | 17095583
taaaggtccatgcaacccagaaatg

SEQ ID NO: 837 - DNA, 25 bp, Artificial Sequence
  >Male | ENST00000456944 | 17095583
tgttggaagccagaagtgacctgag

SEQ ID NO: 838 - DNA, 25 bp, Artificial Sequence
  >Male | ENST00000456944 | 17095583
ctggcctgctctccttcaaggtgaa

SEQ ID NO: 839 - DNA, 25 bp, Artificial Sequence
  >Male | ENST00000456944 | 17095583
tgaaacccactgtgccaagggttgg

SEQ ID NO: 840 - DNA, 25 bp, Artificial Sequence
  >Male | ENST00000456944 | 17095583
tgtgattctcaccaacatcttcagg

SEQ ID NO: 841 - DNA, 25 bp, Artificial Sequence
  >Male | ENST00000456944 | 17095583
taagcaaagtctctcccatgaaaca

SEQ ID NO: 842 - DNA, 25 bp, Artificial Sequence
  >Male | NM_080717 | 16757527
ctgtggctgcgcagacccggcactg

SEQ ID NO: 843 - DNA, 25 bp, Artificial Sequence
  >Male | NM_080717 | 16757527
acgtccggaacctgtggctgcgcag

SEQ ID NO: 844 - DNA, 25 bp, Artificial Sequence
  >Male | NM_080717 | 16757527
aagacgtccggaacctgtggctgcg

SEQ ID NO: 845 - DNA, 25 bp, Artificial Sequence
  >Male | NM_080717 | 16757527
ccaagacgtccggaacctgtggctg

SEQ ID NO: 846 - DNA, 25 bp, Artificial Sequence
  >Male | NM_080717 | 16757527
cattcctccggagaaagccgggttg

SEQ ID NO: 847 - DNA, 25 bp, Artificial Sequence
  >Male | NM_080717 | 16757527
ctcattcctccggagaaagccgggt

SEQ ID NO: 848 - DNA, 25 bp, Artificial Sequence
  >Male | NM_080717 | 16757527
tagagcggcgcctcggtattcattt

SEQ ID NO: 849 - DNA, 25 bp, Artificial Sequence
  >Male | NM_080717 | 16757527
tatgcaagtctgcaagagggcactg

SEQ ID NO: 850 - DNA, 25 bp, Artificial Sequence
  >Male | NM_080717 | 16757527
gcaaggcacattacggagaactccc

SEQ ID NO: 851 - DNA, 25 bp, Artificial Sequence
  >Male | NM_080717 | 16757527
gccactctgggacgaattgcattct

SEQ ID NO: 852 - DNA, 25 bp, Artificial Sequence
  >Male | NM_080717 | 16757527
tcggcgggccctggtacaataatta

SEQ ID NO: 853 - DNA, 25 bp, Artificial Sequence
  >Male | NM_080717 | 16757527
aaaatagagtgcctcgtgcctcggc

SEQ ID NO: 854 - DNA, 25 bp, Artificial Sequence
  >Male | NM_080717 | 16757527
cttagaaattgtgcccattgatcag

SEQ ID NO: 855 - DNA, 25 bp, Artificial Sequence
  >Male | NM_080717 | 16757527
gcttagaaattgtgcccattgatca

SEQ ID NO: 856 - DNA, 25 bp, Artificial Sequence
  >Male | NM_080717 | 16757527
tgcttagaaattgtgcccattgatc

SEQ ID NO: 857 - DNA, 25 bp, Artificial Sequence
  >Male | NM_080717 | 16757527
ctgcttagaaattgtgcccattgat

SEQ ID NO: 858 - DNA, 25 bp, Artificial Sequence
  >Male | NM_080717 | 16757527
aagtttgcgagcatccaccactgcg

SEQ ID NO: 859 - DNA, 25 bp, Artificial Sequence
  >Male | NM_080717 | 16757527
tagtgggtttccagcggtgcgcaaa

SEQ ID NO: 860 - DNA, 25 bp, Artificial Sequence
  >Male | NM_080717 | 16757527
tacgcggtacgttttgcaactcaac

SEQ ID NO: 861 - DNA, 25 bp, Artificial Sequence
  >Male | NM_080717 | 16757527
ggcgtctacgcggtacgttttgcaa

SEQ ID NO: 862 - DNA, 25 bp, Artificial Sequence
  >Male | NM_080717 | 16757527
tgggcaggcctagctcttctctcgg

SEQ ID NO: 863 - DNA, 25 bp, Artificial Sequence
  >Male | NM_080717 | 16757527
cgctctccggctctgtgctgggcag

SEQ ID NO: 864 - DNA, 25 bp, Artificial Sequence
  >Male | NM_080717 | 16757527
cagaatcctttgaatgccggtccag

SEQ ID NO: 865 - DNA, 25 bp, Artificial Sequence
  >Male | NM_080717 | 16757527
gaaagcgacagttctccgaaaggag

SEQ ID NO: 866 - DNA, 25 bp, Artificial Sequence
  >Male | NM_080717 | 16757527
tatcaacagcaatgggcccctttgg

SEQ ID NO: 867 - DNA, 25 bp, Artificial Sequence
  >Male | NM_080717 | 16757527
cattgggatccttctcagctgggcc

SEQ ID NO: 868 - DNA, 25 bp, Artificial Sequence
  >Male | TCONS_l2_00026656-XLOC_l2_013873 | 17058221
cccgcagagcctggaaaggcactga

SEQ ID NO: 869 - DNA, 25 bp, Artificial Sequence
  >Male | TCONS_l2_00026656-XLOC_l2_013873 | 17058221
ccgcagagcctggaaaggcactgac

SEQ ID NO: 870 - DNA, 25 bp, Artificial Sequence
  >Male | TCONS_l2_00026656-XLOC_l2_013873 | 17058221
cgcagagcctggaaaggcactgacc

SEQ ID NO: 871 - DNA, 25 bp, Artificial Sequence
  >Male | TCONS_l2_00026656-XLOC_l2_013873 | 17058221
gcagagcctggaaaggcactgaccc

SEQ ID NO: 872 - DNA, 25 bp, Artificial Sequence
  >Male | TCONS_l2_00026656-XLOC_l2_013873 | 17058221
ggaatacctctatgctgttttaagc

SEQ ID NO: 873 - DNA, 25 bp, Artificial Sequence
  >Male | TCONS_l2_00026656-XLOC_l2_013873 | 17058221
cccaactgggtatggttcagatctg

SEQ ID NO: 874 - DNA, 25 bp, Artificial Sequence
  >Male | TCONS_l2_00026656-XLOC_l2_013873 | 17058221
ccaactgggtatggttcagatctgc

SEQ ID NO: 875 - DNA, 25 bp, Artificial Sequence
  >Male | TCONS_l2_00026656-XLOC_l2_013873 | 17058221
caactgggtatggttcagatctgca

SEQ ID NO: 876 - DNA, 25 bp, Artificial Sequence
  >Male | TCONS_l2_00026656-XLOC_l2_013873 | 17058221
tgtgctgggtcggagtttgtcaacc

SEQ ID NO: 877 - DNA, 25 bp, Artificial Sequence
  >Male | TCONS_l2_00026656-XLOC_l2_013873 | 17058221
aggctccactccgaggaaaaaccag

SEQ ID NO: 878 - DNA, 25 bp, Artificial Sequence
  >Male | TCONS_l2_00026656-XLOC_l2_013873 | 17058221
gaggaaaaaccagcgcagctccagg

SEQ ID NO: 879 - DNA, 25 bp, Artificial Sequence
  >Male | TCONS_l2_00026656-XLOC_l2_013873 | 17058221
gcactgtagcgccactgtgacgtcg

SEQ ID NO: 880 - DNA, 25 bp, Artificial Sequence
  >Male | ExonID_5262586 | 17025653
gactttaagcaaacagacaggcctg

SEQ ID NO: 881 - DNA, 25 bp, Artificial Sequence
  >Male | ExonID_5262586 | 17025653
gagtctcttcatgcctctgcgctga

SEQ ID NO: 882 - DNA, 25 bp, Artificial Sequence
  >Male | ExonID_5262586 | 17025653
tttgagcacttgcatcgccgtcagg

SEQ ID NO: 883 - DNA, 25 bp, Artificial Sequence
  >Male | ExonID_5262586 | 17025653
tagctgcgtcagatatcgagtccca

SEQ ID NO: 884 - DNA, 25 bp, Artificial Sequence
  >Male | ExonID_5262586 | 17025653
tgcaatcatgctctgaggcctccca

SEQ ID NO: 885 - DNA, 25 bp, Artificial Sequence
  >Male | ExonID_5262586 | 17025653
tcttattgctgatgaccgtcctccg

SEQ ID NO: 886 - DNA, 25 bp, Artificial Sequence
  >Male | ExonID_5262586 | 17025653
ttagactcagaagcctaggagcctg

SEQ ID NO: 887 - DNA, 25 bp, Artificial Sequence
  >Male | ExonID_5262586 | 17025653
tccgtttgaagagagctcgcagcaa

SEQ ID NO: 888 - DNA, 25 bp, Artificial Sequence
  >Male | ExonID_5262586 | 17025653
gatgagagccatggtctccttcctg

SEQ ID NO: 889 - DNA, 25 bp, Artificial Sequence
  >Male | ExonID_5262586 | 17025653
tgtactcgatcgtcccgcagaagga

SEQ ID NO: 890 - DNA, 25 bp, Artificial Sequence
  >Male | ExonID_5262586 | 17025653
tggagatggtctaaagccaaggcca

SEQ ID NO: 891 - DNA, 25 bp, Artificial Sequence
  >Male | ExonID_5262586 | 17025653
gatccttgtcctaaaaccttcagca

SEQ ID NO: 892 - DNA, 25 bp, Artificial Sequence
  >Male | ExonID_5262586 | 17025653
caagtctgttcctgaatcggctgca

SEQ ID NO: 893 - DNA, 25 bp, Artificial Sequence
  >Male | ExonID_5262586 | 17025653
tcaagggacgagaattcagatcatc

SEQ ID NO: 894 - DNA, 25 bp, Artificial Sequence
  >Male | ExonID_5262586 | 17025653
gacttcctgcgcaggtacacagaga

SEQ ID NO: 895 - DNA, 25 bp, Artificial Sequence
  >Male | ExonID_5262586 | 17025653
cgagctgcggtcacaaagggcaggc

SEQ ID NO: 896 - DNA, 25 bp, Artificial Sequence
  >Male | ExonID_5262586 | 17025653
taattgttgatcagcaaacgcagcc

SEQ ID NO: 897 - DNA, 25 bp, Artificial Sequence
  >Male | ExonID_5262586 | 17025653
cagcttcttgtgtggcagcctgatc

SEQ ID NO: 898 - DNA, 25 bp, Artificial Sequence
  >Male | ExonID_5262586 | 17025653
ttatcaccttgtgggctgctgcgcc

SEQ ID NO: 899 - DNA, 25 bp, Artificial Sequence
  >Male | ExonID_5262586 | 17025653
tacctttgtcttgcaggcagctgag

SEQ ID NO: 900 - DNA, 25 bp, Artificial Sequence
  >Male | ExonID_5262586 | 17025653
aactgctcacagatatttaatttca

SEQ ID NO: 901 - DNA, 25 bp, Artificial Sequence
  >Male | ExonID_5262586 | 17025653
caatctccccaaacaaagcagagtg

SEQ ID NO: 902 - DNA, 25 bp, Artificial Sequence
  >Male | ExonID_5262586 | 17025653
gatctttttccatagttccagcaac

SEQ ID NO: 903 - DNA, 25 bp, Artificial Sequence
  >Male | ExonID_5262586 | 17025653
gttgagtctgaggatgccgctgcca

SEQ ID NO: 904 - DNA, 25 bp, Artificial Sequence
  >Male | ExonID_5262586 | 17025653
taggccatataggacgctggtcaaa

SEQ ID NO: 905 - DNA, 25 bp, Artificial Sequence
  >Male | AK293404 | 16868954
tgacttaccttacctgagcttcaga

SEQ ID NO: 906 - DNA, 25 bp, Artificial Sequence
  >Male | AK293404 | 16868954
acagacagagtgttccgggtcccct

SEQ ID NO: 907 - DNA, 25 bp, Artificial Sequence
  >Male | AK293404 | 16868954
ttgtgcttctgcaaggctcgccgga

SEQ ID NO: 908 - DNA, 25 bp, Artificial Sequence
  >Male | AK293404 | 16868954
gatgcttcgatacaggttcccgtgg

SEQ ID NO: 909 - DNA, 25 bp, Artificial Sequence
  >Male | AK293404 | 16868954
tgatgagcttttctctcgggcaagc

SEQ ID NO: 910 - DNA, 25 bp, Artificial Sequence
  >Male | AK293404 | 16868954
actgagacgcttggtgaggctgatc

SEQ ID NO: 911 - DNA, 25 bp, Artificial Sequence
  >Male | AK293404 | 16868954
tgtcaggagccccactgtagtaagg

SEQ ID NO: 912 - DNA, 25 bp, Artificial Sequence
  >Male | AK293404 | 16868954
ttgtccccatcccaaactgtaatca

SEQ ID NO: 913 - DNA, 25 bp, Artificial Sequence
  >Male | AK293404 | 16868954
tcttcttgggatccctcagtggcct

SEQ ID NO: 914 - DNA, 25 bp, Artificial Sequence
  >Male | AK293404 | 16868954
tttcctgaaagtagatagcggttcc

SEQ ID NO: 915 - DNA, 25 bp, Artificial Sequence
  >Male | AK293404 | 16868954
agaagttccgcagttctcggcagcg

SEQ ID NO: 916 - DNA, 25 bp, Artificial Sequence
  >Male | AK293404 | 16868954
ttcctccgcgcaggcctctgaagag

SEQ ID NO: 917 - DNA, 25 bp, Artificial Sequence
  >Male | AK293404 | 16868954
aaatcctgagggtggtcctgcagcc

SEQ ID NO: 918 - DNA, 25 bp, Artificial Sequence
  >Male | AK293404 | 16868954
tgttgaagctcagatcttgtaccgc

SEQ ID NO: 919 - DNA, 25 bp, Artificial Sequence
  >Male | AK293404 | 16868954
tgccgccgcagggagacactgtaca

SEQ ID NO: 920 - DNA, 25 bp, Artificial Sequence
  >Male | AK293404 | 16868954
agctctttgcctgctgtgcgctcca

SEQ ID NO: 921 - DNA, 25 bp, Artificial Sequence
  >Male | ENST00000338315 | 16877665
gcacggccgtgtaagctgcaggtca

SEQ ID NO: 922 - DNA, 25 bp, Artificial Sequence
  >Male | ENST00000338315 | 16877665
catttactgagtcagcacggccgtg

SEQ ID NO: 923 - DNA, 25 bp, Artificial Sequence
  >Male | ENST00000338315 | 16877665
ttgtacagaatgagaggcgaccggc

SEQ ID NO: 924 - DNA, 25 bp, Artificial Sequence
  >Male | ENST00000338315 | 16877665
aaggcatgagccgtccagaccctgt

SEQ ID NO: 925 - DNA, 25 bp, Artificial Sequence
  >Male | ENST00000338315 | 16877665
tagaaagtcgtgtaccagaggcctc

SEQ ID NO: 926 - DNA, 25 bp, Artificial Sequence
  >Male | ENST00000338315 | 16877665
gtgagcgctgtgtagggcacctgga

SEQ ID NO: 927 - DNA, 25 bp, Artificial Sequence
  >Male | ENST00000338315 | 16877665
gccggacacgatgagcccgtggaca

SEQ ID NO: 928 - DNA, 25 bp, Artificial Sequence
  >Male | ENST00000338315 | 16877665
cagggtggctggatgcatcccagaa

SEQ ID NO: 929 - DNA, 25 bp, Artificial Sequence
  >Male | ENST00000338315 | 16877665
actcctttcaaagggcacctgaccg

SEQ ID NO: 930 - DNA, 25 bp, Artificial Sequence
  >Male | ENST00000338315 | 16877665
ggtaagtcactacaaccacggcagc

SEQ ID NO: 931 - DNA, 25 bp, Artificial Sequence
  >Male | ENST00000338315 | 16877665
tcacccctaggcacagtaaactgat

SEQ ID NO: 932 - DNA, 25 bp, Artificial Sequence
  >Male | ENST00000338315 | 16877665
gatgaacaggaaggagatcaccagc

SEQ ID NO: 933 - DNA, 25 bp, Artificial Sequence
  >Male | ENST00000338315 | 16877665
ctgaacagcagcagagatgaacagg

SEQ ID NO: 934 - DNA, 25 bp, Artificial Sequence
  >Male | ENST00000338315 | 16877665
ggacagttagtaccaggccctggac

SEQ ID NO: 935 - DNA, 25 bp, Artificial Sequence
  >Male | ENST00000338315 | 16877665
agatcccaaaggctgacgtcttctt

SEQ ID NO: 936 - DNA, 25 bp, Artificial Sequence
  >Male | ENST00000338315 | 16877665
gatacaaaggccacgacatatgcca

SEQ ID NO: 937 - DNA, 25 bp, Artificial Sequence
  >Male | ENST00000338315 | 16877665
caggtttacatgaaggaggtgacac

SEQ ID NO: 938 - DNA, 25 bp, Artificial Sequence
  >Male | ENST00000338315 | 16877665
cacatgcgccagacagcttggtgaa

SEQ ID NO: 939 - DNA, 25 bp, Artificial Sequence
  >Male | ENST00000338315 | 16877665
gcttgcttgcagacccctgccttat

SEQ ID NO: 940 - DNA, 25 bp, Artificial Sequence
  >Male | ENST00000338315 | 16877665
ttaggccaggctgtagctggtcctc

SEQ ID NO: 941 - DNA, 25 bp, Artificial Sequence
  >Male | ENST00000338315 | 16877665
gaaaggtcacatactaaactgccag

SEQ ID NO: 942 - DNA, 25 bp, Artificial Sequence
  >Male | ENST00000338315 | 16877665
agggtcccctacacaagagtttctg

SEQ ID NO: 943 - DNA, 25 bp, Artificial Sequence
  >Male | ENST00000432646 | 17051908
tagacccagtcttgcctcctgagaa

SEQ ID NO: 944 - DNA, 25 bp, Artificial Sequence
  >Male | ENST00000432646 | 17051908
cctgaatacaatgcaagggagggag

SEQ ID NO: 945 - DNA, 25 bp, Artificial Sequence
  >Male | ENST00000432646 | 17051908
tgtcattccctaggcatgctcagga

SEQ ID NO: 946 - DNA, 25 bp, Artificial Sequence
  >Male | ENST00000432646 | 17051908
gcacattttgttctagatggagttc

SEQ ID NO: 947 - DNA, 25 bp, Artificial Sequence
  >Male | ENST00000432646 | 17051908
caacaagagaggtcggtgtgccaca

SEQ ID NO: 948 - DNA, 25 bp, Artificial Sequence
  >Male | ENST00000432646 | 17051908
ggttggtcaccaatccctgtggaat

SEQ ID NO: 949 - DNA, 25 bp, Artificial Sequence
  >Male | ENST00000432646 | 17051908
cttggaaggctgactcatgttgtct

SEQ ID NO: 950 - DNA, 25 bp, Artificial Sequence
  >Male | ENST00000432646 | 17051908
cctgcgtttctgtgccatggagtca

SEQ ID NO: 951 - DNA, 25 bp, Artificial Sequence
  >Male | ENST00000432646 | 17051908
ccttctaagttctctgcgacgctca

SEQ ID NO: 952 - DNA, 25 bp, Artificial Sequence
  >Male | ENST00000432646 | 17051908
aaatgcacggtgcaggatgctcccg

SEQ ID NO: 953 - DNA, 25 bp, Artificial Sequence
  >Male | ENST00000432646 | 17051908
gctgcgtcttccatgcgatccggat

SEQ ID NO: 954 - DNA, 25 bp, Artificial Sequence
  >Male | ENST00000432646 | 17051908
tagagtgatttggagaactgactcc

SEQ ID NO: 955 - DNA, 25 bp, Artificial Sequence
  >Male | ENST00000432646 | 17051908
acagttgaccggtccccaagatcag

SEQ ID NO: 956 - DNA, 25 bp, Artificial Sequence
  >Male | ENST00000432646 | 17051908
caaaagatacagcatgttgcatgag

SEQ ID NO: 957 - DNA, 25 bp, Artificial Sequence
  >Male | ENST00000432646 | 17051908
tcatcgtcattcctctggtaggcga

SEQ ID NO: 958 - DNA, 25 bp, Artificial Sequence
  >Male | ENST00000432646 | 17051908
tgcattcttctgcttgggagcgaca

SEQ ID NO: 959 - DNA, 25 bp, Artificial Sequence
  >Male | ENST00000432646 | 17051908
ctatctcgtatctttcttggcgact

SEQ ID NO: 960 - DNA, 25 bp, Artificial Sequence
  >Male | ENST00000432646 | 17051908
gattttctccaatgctccctcgctt

SEQ ID NO: 961 - DNA, 25 bp, Artificial Sequence
  >Male | ENST00000432646 | 17051908
tcttttagcttgcactttagttccc

SEQ ID NO: 962 - DNA, 25 bp, Artificial Sequence
  >Male | ENST00000432646 | 17051908
taagtttgtgggtcatgaattctcc

SEQ ID NO: 963 - DNA, 25 bp, Artificial Sequence
  >Male | ENST00000432646 | 17051908
gaatatcctgtgtcctccagaacaa

SEQ ID NO: 964 - DNA, 25 bp, Artificial Sequence
  >Male | ENST00000432646 | 17051908
tgagttttcgatcggcttcctcctg

SEQ ID NO: 965 - DNA, 25 bp, Artificial Sequence
  >Male | ENST00000432646 | 17051908
tgtcaggcagactcaagggagacct

SEQ ID NO: 966 - DNA, 25 bp, Artificial Sequence
  >Male | ENST00000432646 | 17051908
tctggcgtttctcagcagcttctgc

SEQ ID NO: 967 - DNA, 25 bp, Artificial Sequence
  >Male | ENST00000432646 | 17051908
tgtcatctgacaagccatcttctgg

SEQ ID NO: 968 - DNA, 25 bp, Artificial Sequence
  >Male | ENST00000432646 | 17051908
ggtatactgctccagtctgctgtca

SEQ ID NO: 969 - DNA, 25 bp, Artificial Sequence
  >Male | ENST00000432646 | 17051908
tatttggagtaagatggcccgggct

SEQ ID NO: 970 - DNA, 25 bp, Artificial Sequence
  >Male | ENST00000432646 | 17051908
cattgatgcggctagaaacccctac

SEQ ID NO: 971 - DNA, 25 bp, Artificial Sequence
  >Male | ENST00000432646 | 17051908
gagaaagacccactccggaagaaga

SEQ ID NO: 972 - DNA, 25 bp, Artificial Sequence
  >Male | ENST00000432646 | 17051908
gcagaaaaacatcgataggtggcca

SEQ ID NO: 973 - DNA, 25 bp, Artificial Sequence
  >Male | ENST00000432646 | 17051908
cagattgcttttcccagaggttccg

SEQ ID NO: 974 - DNA, 25 bp, Artificial Sequence
  >Male | ENST00000432646 | 17051908
tctgaaatactagtcttcccaatag

SEQ ID NO: 975 - DNA, 25 bp, Artificial Sequence
  >Male | ENST00000432646 | 17051908
aactgagctcgtcctgcgtcttgag

SEQ ID NO: 976 - DNA, 25 bp, Artificial Sequence
  >Male | ENST00000432646 | 17051908
tgacgggagtcaatgctacctggga

SEQ ID NO: 977 - DNA, 25 bp, Artificial Sequence
  >Male | ENST00000518932 | 17080053
catgcccatgcaagaggaatgtgat

SEQ ID NO: 978 - DNA, 25 bp, Artificial Sequence
  >Male | ENST00000518932 | 17080053
tcagttgcaagatgacgctcagtcg

SEQ ID NO: 979 - DNA, 25 bp, Artificial Sequence
  >Male | ENST00000518932 | 17080053
caataaagtgctcttcatagttcat

SEQ ID NO: 980 - DNA, 25 bp, Artificial Sequence
  >Male | ENST00000518932 | 17080053
tttctgtgatttcaggtgccacctg

SEQ ID NO: 981 - DNA, 25 bp, Artificial Sequence
  >Male | ENST00000518932 | 17080053
ggtgccacctgttcttcactattag

SEQ ID NO: 982 - DNA, 25 bp, Artificial Sequence
  >Male | ENST00000518932 | 17080053
tcctaaatgttgagataccccaagt

SEQ ID NO: 983 - DNA, 25 bp, Artificial Sequence
  >Male | ENST00000518932 | 17080053
ggttaccacatgaatgcagagagca

SEQ ID NO: 984 - DNA, 25 bp, Artificial Sequence
  >Male | ENST00000518932 | 17080053
gcctgtatgtcttctccaagttcca

SEQ ID NO: 985 - DNA, 25 bp, Artificial Sequence
  >Male | ENST00000518932 | 17080053
aagctaatcgcagaagccttcaggg

SEQ ID NO: 986 - DNA, 25 bp, Artificial Sequence
  >Male | ENST00000518932 | 17080053
aatcagctggcttaattaattgccc

SEQ ID NO: 987 - DNA, 25 bp, Artificial Sequence
  >Male | ENST00000518932 | 17080053
tccaccagatttttaccacaagttg

SEQ ID NO: 988 - DNA, 25 bp, Artificial Sequence
  >Male | ENST00000518932 | 17080053
ttccctgtgtagatgaatgaagcca

SEQ ID NO: 989 - DNA, 25 bp, Artificial Sequence
  >Male | ENST00000518932 | 17080053
tactgacacagaagcttgggagcaa

SEQ ID NO: 990 - DNA, 25 bp, Artificial Sequence
  >Male | ENST00000518932 | 17080053
catggatgggcgagttacttaacac

SEQ ID NO: 991 - DNA, 25 bp, Artificial Sequence
  >Male | ENST00000518932 | 17080053
taatcaatcagataatttacatcac

SEQ ID NO: 992 - DNA, 25 bp, Artificial Sequence
  >Male | ENST00000518932 | 17080053
caaaagagaaacaggcacctcttca

SEQ ID NO: 993 - DNA, 25 bp, Artificial Sequence
  >Male | ENST00000518932 | 17080053
caataaaagtgttgaaggtgcctcc

SEQ ID NO: 994 - DNA, 25 bp, Artificial Sequence
  >Male | ENST00000518932 | 17080053
cttaagctccactatgagagaagtg

SEQ ID NO: 995 - DNA, 25 bp, Artificial Sequence
  >Male | ENST00000518932 | 17080053
taagctccactatgagagaagtgtg

SEQ ID NO: 996 - DNA, 25 bp, Artificial Sequence
  >Male | ENST00000518932 | 17080053
tgtgaagaacttaataatcaccagc

SEQ ID NO: 997 - DNA, 25 bp, Artificial Sequence
  >Male | ENST00000518932 | 17080053
tggtatccggtgagcattaaactct

SEQ ID NO: 998 - DNA, 25 bp, Artificial Sequence
  >Male | ENST00000518932 | 17080053
aactctgttgtctcagtgtaactga

SEQ ID NO: 999 - DNA, 25 bp, Artificial Sequence
  >Male | ENST00000518932 | 17080053
cagtggtcctgtgtacttgctagtc

SEQ ID NO: 1000 - DNA, 25 bp, Artificial Sequence
  >Male | ENST00000518932 | 17080053
tctgctggtggattcattgtaggaa

SEQ ID NO: 1001 - DNA, 25 bp, Artificial Sequence
  >Male | ENST00000518932 | 17080053
gaatgcgtactacatactgtaagga

SEQ ID NO: 1002 - DNA, 25 bp, Artificial Sequence
  >Male | ENST00000518932 | 17080053
tgtgctgcggtcaagaataggtcga

SEQ ID NO: 1003 - DNA, 25 bp, Artificial Sequence
  >Male | NM_001033551 | 16842003
taaacttctaggacgagtggacagc

SEQ ID NO: 1004 - DNA, 25 bp, Artificial Sequence
  >Male | NM_001033551 | 16842003
tattggtagtgtcgtctcagcagcg

SEQ ID NO: 1005 - DNA, 25 bp, Artificial Sequence
  >Male | NM_001033551 | 16842003
tcacagggcgaagagggcatcctct

SEQ ID NO: 1006 - DNA, 25 bp, Artificial Sequence
  >Male | NM_001033551 | 16842003
gcagctttggctctttcttcaagga

SEQ ID NO: 1007 - DNA, 25 bp, Artificial Sequence
  >Male | NM_001033551 | 16842003
tcggtcctgagccacacctcaatgt

SEQ ID NO: 1008 - DNA, 25 bp, Artificial Sequence
  >Male | NM_001033551 | 16842003
gcaaatgataagaagcaggctcccg

SEQ ID NO: 1009 - DNA, 25 bp, Artificial Sequence
  >Male | NM_001033551 | 16842003
tgagtgtccactctcacattgcggg

SEQ ID NO: 1010 - DNA, 25 bp, Artificial Sequence
  >Male | NM_001033551 | 16842003
cattccttgggttataagccagctg

SEQ ID NO: 1011 - DNA, 25 bp, Artificial Sequence
  >Male | NM_001033551 | 16842003
gggttataagccagctgtctatggg

SEQ ID NO: 1012 - DNA, 25 bp, Artificial Sequence
  >Male | NM_001033551 | 16842003
tgtctagtgcagaagcaagtcctcc

SEQ ID NO: 1013 - DNA, 25 bp, Artificial Sequence
  >Male | NM_001033551 | 16842003
tctcgctgtaaggaatgggttcacc

SEQ ID NO: 1014 - DNA, 25 bp, Artificial Sequence
  >Male | NM_001033551 | 16842003
gcaaacatgtcaaagccgtcacggg

SEQ ID NO: 1015 - DNA, 25 bp, Artificial Sequence
  >Male | NM_001033551 | 16842003
tgagggtgccactgacgctctctgt

SEQ ID NO: 1016 - DNA, 25 bp, Artificial Sequence
  >Male | NM_001033551 | 16842003
gctgtgttccccaccattgggctca

SEQ ID NO: 1017 - DNA, 25 bp, Artificial Sequence
  >Male | NM_001033551 | 16842003
gcattttgaacggatcggccagacc

SEQ ID NO: 1018 - DNA, 25 bp, Artificial Sequence
  >Male | NM_001033551 | 16842003
gatcggccagacctgtatcgttcga

SEQ ID NO: 1019 - DNA, 25 bp, Artificial Sequence
  >Male | NM_001033551 | 16842003
aagaaatccctctgttatggcaaca

SEQ ID NO: 1020 - DNA, 25 bp, Artificial Sequence
  >Male | NM_001033551 | 16842003
tggcaacaatcttttcaagggaaaa

SEQ ID NO: 1021 - DNA, 25 bp, Artificial Sequence
  >Male | NM_001033551 | 16842003
tgaggtcatcgttcacatgcagcag

SEQ ID NO: 1022 - DNA, 25 bp, Artificial Sequence
  >Male | NM_001033551 | 16842003
tcctcattggacacgcgggagatga

SEQ ID NO: 1023 - DNA, 25 bp, Artificial Sequence
  >Male | NM_001033551 | 16842003
tagggaacacatgcacctctgggta

SEQ ID NO: 1024 - DNA, 25 bp, Artificial Sequence
  >Male | NM_001033551 | 16842003
ccatcacttggtacagactgcctca

SEQ ID NO: 1025 - DNA, 25 bp, Artificial Sequence
  >Male | NM_001033551 | 16842003
ttgtgaatggctcatgtccccaggc

SEQ ID NO: 1026 - DNA, 25 bp, Artificial Sequence
  >Male | NM_001033551 | 16842003
ctctcaaaaagctgcctgggccttg

SEQ ID NO: 1027 - DNA, 25 bp, Artificial Sequence
  >Male | NM_001033551 | 16842003
tgtgtttcctcgaacgacgtccagt

SEQ ID NO: 1028 - DNA, 25 bp, Artificial Sequence
  >Male | NM_001033551 | 16842003
cgaggaataggaaccagcacttgtc

SEQ ID NO: 1029 - DNA, 25 bp, Artificial Sequence
  >Male | NM_001033551 | 16842003
ggcatggtcgcagctggatccactt

SEQ ID NO: 1030 - DNA, 25 bp, Artificial Sequence
  >Male | NM_001033551 | 16842003
catatatgtgcacaacgccggtgag

SEQ ID NO: 1031 - DNA, 25 bp, Artificial Sequence
  >Male | NM_001033551 | 16842003
gactgcttcgaaaggcatcagccca

SEQ ID NO: 1032 - DNA, 25 bp, Artificial Sequence
  >Male | NM_001033551 | 16842003
gatgaaatctcggttggccacaagg

SEQ ID NO: 1033 - DNA, 25 bp, Artificial Sequence
  >Male | NM_001033551 | 16842003
tctgtagttccggttcccgttgagc

SEQ ID NO: 1034 - DNA, 25 bp, Artificial Sequence
  >Male | NM_001033551 | 16842003
tcttcagggctcgaatggcatcctt

SEQ ID NO: 1035 - DNA, 25 bp, Artificial Sequence
  >Male | NM_001033551 | 16842003
tgtcacagatctccatattcaacgt

SEQ ID NO: 1036 - DNA, 25 bp, Artificial Sequence
  >Male | NM_001033551 | 16842003
gaggcactgccccactggtgtgctg

SEQ ID NO: 1037 - DNA, 25 bp, Artificial Sequence
  >Male | NM_001033551 | 16842003
ggactcccgtcctgactgacacttg

SEQ ID NO: 1038 - DNA, 25 bp, Artificial Sequence
  >Male | NM_001033551 | 16842003
tctggaacgccgagcttagggcctt

SEQ ID NO: 1039 - DNA, 25 bp, Artificial Sequence
  >Male | NM_001105206 | 17022799
ccagtaggaattgcgtgtgctctca

SEQ ID NO: 1040 - DNA, 25 bp, Artificial Sequence
  >Male | NM_001105206 | 17022799
acaggagttgatgcttacggcgccg

SEQ ID NO: 1041 - DNA, 25 bp, Artificial Sequence
  >Male | NM_001105206 | 17022799
cacatggttcacttcagagtccaca

SEQ ID NO: 1042 - DNA, 25 bp, Artificial Sequence
  >Male | NM_001105206 | 17022799
cacagagactctgcttgggtgtaac

SEQ ID NO: 1043 - DNA, 25 bp, Artificial Sequence
  >Male | NM_001105206 | 17022799
aactgcttctgggacggacttcaaa

SEQ ID NO: 1044 - DNA, 25 bp, Artificial Sequence
  >Male | NM_001105206 | 17022799
gaagactttcttctaggactcggag

SEQ ID NO: 1045 - DNA, 25 bp, Artificial Sequence
  >Male | NM_001105206 | 17022799
catgccatgggaggaacgagttctc

SEQ ID NO: 1046 - DNA, 25 bp, Artificial Sequence
  >Male | NM_001105206 | 17022799
gagtttcagagcaacaggatcccat

SEQ ID NO: 1047 - DNA, 25 bp, Artificial Sequence
  >Male | NM_001105206 | 17022799
tgtggaccttttcagtataccgttg

SEQ ID NO: 1048 - DNA, 25 bp, Artificial Sequence
  >Male | NM_001105206 | 17022799
tactgagcactgattggtgagccac

SEQ ID NO: 1049 - DNA, 25 bp, Artificial Sequence
  >Male | NM_001105206 | 17022799
gacccactctaggttggataagcag

SEQ ID NO: 1050 - DNA, 25 bp, Artificial Sequence
  >Male | NM_001105206 | 17022799
gctaatgacgaagtgggacagccca

SEQ ID NO: 1051 - DNA, 25 bp, Artificial Sequence
  >Male | NM_001105206 | 17022799
tgtccattgaaatatgctctgcgag

SEQ ID NO: 1052 - DNA, 25 bp, Artificial Sequence
  >Male | NM_001105206 | 17022799
tcttttggaactggaagcccttcat

SEQ ID NO: 1053 - DNA, 25 bp, Artificial Sequence
  >Male | NM_001105206 | 17022799
tgtaagatttctggaggagctcctc

SEQ ID NO: 1054 - DNA, 25 bp, Artificial Sequence
  >Male | NM_001105206 | 17022799
gggtccttcagttgctctttagata

SEQ ID NO: 1055 - DNA, 25 bp, Artificial Sequence
  >Male | NM_001105206 | 17022799
gggccaccgctgaatccaaaatcat

SEQ ID NO: 1056 - DNA, 25 bp, Artificial Sequence
  >Male | NM_001105206 | 17022799
catcgaagaagtaactggcagcccg

SEQ ID NO: 1057 - DNA, 25 bp, Artificial Sequence
  >Male | NM_001105206 | 17022799
ggcagccaacaaagccaggcaggtt

SEQ ID NO: 1058 - DNA, 25 bp, Artificial Sequence
  >Male | NM_001105206 | 17022799
tgtgctacttagactcgggactgtt

SEQ ID NO: 1059 - DNA, 25 bp, Artificial Sequence
  >Male | NM_001105206 | 17022799
taagcaggccaggaactgacgggct

SEQ ID NO: 1060 - DNA, 25 bp, Artificial Sequence
  >Male | NM_001105206 | 17022799
ggtttcatgtacaggctcagagacg

SEQ ID NO: 1061 - DNA, 25 bp, Artificial Sequence
  >Male | NM_001105206 | 17022799
tcaaccgtacgaagctgatccagga

SEQ ID NO: 1062 - DNA, 25 bp, Artificial Sequence
  >Male | NM_001105206 | 17022799
tgatcagtctagactgccccaggcg

SEQ ID NO: 1063 - DNA, 25 bp, Artificial Sequence
  >Male | NM_001105206 | 17022799
tcactgagtctggttttaagggcac

SEQ ID NO: 1064 - DNA, 25 bp, Artificial Sequence
  >Male | NM_001105206 | 17022799
ctctggcttgattgaggaggttctc

SEQ ID NO: 1065 - DNA, 25 bp, Artificial Sequence
  >Male | NM_001105206 | 17022799
gaaggtcctgtgcatggtcaatagc

SEQ ID NO: 1066 - DNA, 25 bp, Artificial Sequence
  >Male | NM_001105206 | 17022799
tcagagagtccgcagatgtgctcag

SEQ ID NO: 1067 - DNA, 25 bp, Artificial Sequence
  >Male | NM_001105206 | 17022799
tgcttgaagcggacacatgaccact

SEQ ID NO: 1068 - DNA, 25 bp, Artificial Sequence
  >Male | NM_001105206 | 17022799
tccaggacgacaggaaacagagtgc

SEQ ID NO: 1069 - DNA, 25 bp, Artificial Sequence
  >Male | NM_001105206 | 17022799
catccacgagctcccgttgggtgaa

SEQ ID NO: 1070 - DNA, 25 bp, Artificial Sequence
  >Male | NM_001105206 | 17022799
tatcatgggcttgctctaccagctg

SEQ ID NO: 1071 - DNA, 25 bp, Artificial Sequence
  >Male | NM_001105206 | 17022799
taaacgtaaatcttcctggcatgtg

SEQ ID NO: 1072 - DNA, 25 bp, Artificial Sequence
  >Male | NM_001105206 | 17022799
taaactgtgggctctctgaatggac

SEQ ID NO: 1073 - DNA, 25 bp, Artificial Sequence
  >Male | NM_001105206 | 17022799
ttatactccttcctgcaattccagt

SEQ ID NO: 1074 - DNA, 25 bp, Artificial Sequence
  >Male | NM_001105206 | 17022799
tctacgtcagacagaaggcttttca

SEQ ID NO: 1075 - DNA, 25 bp, Artificial Sequence
  >Male | NM_001105206 | 17022799
tcattcacgtgcctatgagcggcgg

SEQ ID NO: 1076 - DNA, 25 bp, Artificial Sequence
  >Male | NM_001105206 | 17022799
tgccctagggaatcaagtggaccac

SEQ ID NO: 1077 - DNA, 25 bp, Artificial Sequence
  >Male | NM_001105206 | 17022799
ccatagtagccaggagcgcaacgtt

SEQ ID NO: 1078 - DNA, 25 bp, Artificial Sequence
  >Male | NM_001105206 | 17022799
gaaagcctctcgtgctctgtggaga

SEQ ID NO: 1079 - DNA, 25 bp, Artificial Sequence
  >Male | NM_001105206 | 17022799
tcgttacaaatgcaccgaacagctc

SEQ ID NO: 1080 - DNA, 25 bp, Artificial Sequence
  >Male | NM_001105206 | 17022799
ggtgctcccctgatggaatctccga

SEQ ID NO: 1081 - DNA, 25 bp, Artificial Sequence
  >Male | NM_001105206 | 17022799
ggcaacctgcaagaactgactgaaa

SEQ ID NO: 1082 - DNA, 25 bp, Artificial Sequence
  >Male | NM_001105206 | 17022799
ggaattgccattacagtcgcagggc

SEQ ID NO: 1083 - DNA, 25 bp, Artificial Sequence
  >Male | NM_001105206 | 17022799
aaatgcctttaacactgtcttatca

SEQ ID NO: 1084 - DNA, 25 bp, Artificial Sequence
  >Male | NM_001105206 | 17022799
gacaaaatgactactgggacacgca

SEQ ID NO: 1085 - DNA, 25 bp, Artificial Sequence
  >Male | NM_001105206 | 17022799
aagtttccgaactgacctagcccag

SEQ ID NO: 1086 - DNA, 25 bp, Artificial Sequence
  >Male | NM_001105206 | 17022799
cgaactgacctagcccaggtgaaac

SEQ ID NO: 1087 - DNA, 25 bp, Artificial Sequence
  >Male | NM_001105206 | 17022799
caggtgaaactctcaaggcactggg

SEQ ID NO: 1088 - DNA, 25 bp, Artificial Sequence
  >Male | NM_001105206 | 17022799
ggttcgctcgtctcaggcgggtctt

SEQ ID NO: 1089 - DNA, 25 bp, Artificial Sequence
  >Male | NM_001105206 | 17022799
ggtcttgcctgccaaccgctgagct

SEQ ID NO: 1090 - DNA, 25 bp, Artificial Sequence
  >Male | NM_001105206 | 17022799
aaccgctgagctcccttcaatgtca

SEQ ID NO: 1091 - DNA, 25 bp, Artificial Sequence
  >Male | NM_001105206 | 17022799
ttctccgctgacatccagtagtgct

SEQ ID NO: 1092 - DNA, 25 bp, Artificial Sequence
  >Male | NM_001105206 | 17022799
tctccgctgacatccagtagtgctc

SEQ ID NO: 1093 - DNA, 25 bp, Artificial Sequence
  >Male | NM_001105206 | 17022799
cagtagtgctcttccagggctcggg

SEQ ID NO: 1094 - DNA, 25 bp, Artificial Sequence
  >Male | NM_001105206 | 17022799
tgtgggtctccgtaggtctcccgcg

SEQ ID NO: 1095 - DNA, 25 bp, Artificial Sequence
  >Male | NM_001105206 | 17022799
tccgtgtgcagtatcccgaggtggc

SEQ ID NO: 1096 - DNA, 25 bp, Artificial Sequence
  >Male | NM_001105206 | 17022799
gaaataaagggaaagtgcgagagta

SEQ ID NO: 1097 - DNA, 25 bp, Artificial Sequence
  >Male | NM_001105206 | 17022799
tcccgcagaggttctggctcaagaa

SEQ ID NO: 1098 - DNA, 25 bp, Artificial Sequence
  >Male | NM_001105206 | 17022799
tacggcatcaaaaggcagacggatt

SEQ ID NO: 1099 - DNA, 25 bp, Artificial Sequence
  >Male | NM_001105206 | 17022799
gctgtcctggcttccttctcacatt

SEQ ID NO: 1100 - DNA, 25 bp, Artificial Sequence
  >Male | NM_001105206 | 17022799
tggcttttcagacactgaggtccgc

SEQ ID NO: 1101 - DNA, 25 bp, Artificial Sequence
  >Male | NM_001105206 | 17022799
cagggtgcccactttcttgagcaag

SEQ ID NO: 1102 - DNA, 25 bp, Artificial Sequence
  >Male | NM_182480 | 16786369
tctgtccagctgaaatgaccgtggg

SEQ ID NO: 1103 - DNA, 25 bp, Artificial Sequence
  >Male | NM_182480 | 16786369
aaccagacgccaaagctagaaaggg

SEQ ID NO: 1104 - DNA, 25 bp, Artificial Sequence
  >Male | NM_182480 | 16786369
ctacgtagtgcgtccggagcagagc

SEQ ID NO: 1105 - DNA, 25 bp, Artificial Sequence
  >Male | NM_182480 | 16786369
cacggtgtctgttgaggcgccggac

SEQ ID NO: 1106 - DNA, 25 bp, Artificial Sequence
  >Male | NM_182480 | 16786369
tctttgggcaagtcgtgctagggct

SEQ ID NO: 1107 - DNA, 25 bp, Artificial Sequence
  >Male | NM_182480 | 16786369
gatggacccacatgcctcaaggatg

SEQ ID NO: 1108 - DNA, 25 bp, Artificial Sequence
  >Male | NM_182480 | 16786369
agagtgacttcacaaggacctgggc

SEQ ID NO: 1109 - DNA, 25 bp, Artificial Sequence
  >Male | NM_182480 | 16786369
tcatgttgcagatatggtcccaggc

SEQ ID NO: 1110 - DNA, 25 bp, Artificial Sequence
  >Male | NM_182480 | 16786369
tgcattcgccgaaaggctctgtatc

SEQ ID NO: 1111 - DNA, 25 bp, Artificial Sequence
  >Male | NM_182480 | 16786369
gtggactccgatatcttaagacaga

SEQ ID NO: 1112 - DNA, 25 bp, Artificial Sequence
  >Male | NM_182480 | 16786369
tcaaacattatcagggcctctgagc

SEQ ID NO: 1113 - DNA, 25 bp, Artificial Sequence
  >Male | NM_182480 | 16786369
tcccaatgaatgcaaggtggaagat

SEQ ID NO: 1114 - DNA, 25 bp, Artificial Sequence
  >Male | NM_182480 | 16786369
cagaggatttctttatggtggacac

SEQ ID NO: 1115 - DNA, 25 bp, Artificial Sequence
  >Male | NM_182480 | 16786369
gagaggattgttaagccactgcacc

SEQ ID NO: 1116 - DNA, 25 bp, Artificial Sequence
  >Male | NM_182480 | 16786369
tgctcctgtagagaaccgtcactcg

SEQ ID NO: 1117 - DNA, 25 bp, Artificial Sequence
  >Male | NM_182480 | 16786369
taaatcgaaaaccagagtccctaga

SEQ ID NO: 1118 - DNA, 25 bp, Artificial Sequence
  >Male | NM_182480 | 16786369
ctaagacggcccatgagattgctcc

SEQ ID NO: 1119 - DNA, 25 bp, Artificial Sequence
  >Male | NM_182480 | 16786369
tactccggagttgtgaccatctgca

SEQ ID NO: 1120 - DNA, 25 bp, Artificial Sequence
  >Male | NM_182480 | 16786369
tatgaataaagtccccagatggcag

SEQ ID NO: 1121 - DNA, 25 bp, Artificial Sequence
  >Male | NM_182480 | 16786369
ggaagaaatctctgccaggctacgt

SEQ ID NO: 1122 - DNA, 25 bp, Artificial Sequence
  >Male | NM_182480 | 16786369
gggaacttacaaacagcctgggcag

SEQ ID NO: 1123 - DNA, 25 bp, Artificial Sequence
  >Male | NM_182480 | 16786369
tcatgggacgtggaccaaaccaagg

SEQ ID NO: 1124 - DNA, 25 bp, Artificial Sequence
  >Male | NM_182480 | 16786369
aaaggcagagttaacggcatccaca

SEQ ID NO: 1125 - DNA, 25 bp, Artificial Sequence
  >Male | NM_182480 | 16786369
taagccccatgctgaaattcgctcg

SEQ ID NO: 1126 - DNA, 25 bp, Artificial Sequence
  >Male | NM_182480 | 16786369
caccagctgtgtcgatgaagtccgt

SEQ ID NO: 1127 - DNA, 25 bp, Artificial Sequence
  >Male | NM_182480 | 16786369
aacagaactcggcttttggcatcca

SEQ ID NO: 1128 - DNA, 25 bp, Artificial Sequence
  >Male | NM_182480 | 16786369
ccgtactgaggtgatgggccaagct

SEQ ID NO: 1129 - DNA, 25 bp, Artificial Sequence
  >Male | NM_182480 | 16786369
gagtggagacactgcatttgtggcc

SEQ ID NO: 1130 - DNA, 25 bp, Artificial Sequence
  >Male | NM_182480 | 16786369
aaatatgtatgatgggtcctgggca

SEQ ID NO: 1131 - DNA, 25 bp, Artificial Sequence
  >Male | ENST00000481363 | 16920377
gcaaagcagcatagcaacaatcgtg

SEQ ID NO: 1132 - DNA, 25 bp, Artificial Sequence
  >Male | ENST00000481363 | 16920377
gttgtggtcacaaccaacgtagtaa

SEQ ID NO: 1133 - DNA, 25 bp, Artificial Sequence
  >Male | ENST00000481363 | 16920377
gatttcactgtgtctgcattgctcc

SEQ ID NO: 1134 - DNA, 25 bp, Artificial Sequence
  >Male | ENST00000481363 | 16920377
tgggaacgccgtcagtagcacttgg

SEQ ID NO: 1135 - DNA, 25 bp, Artificial Sequence
  >Male | ENST00000481363 | 16920377
catctgcactgatacccgactggga

SEQ ID NO: 1136 - DNA, 25 bp, Artificial Sequence
  >Male | ENST00000481363 | 16920377
gcgttattcacaacggaggtggccc

SEQ ID NO: 1137 - DNA, 25 bp, Artificial Sequence
  >Male | ENST00000481363 | 16920377
taaaagctcgcccacaaatgttgca

SEQ ID NO: 1138 - DNA, 25 bp, Artificial Sequence
  >Male | ENST00000481363 | 16920377
tgtcgagggtcccacaaatgtgcca

SEQ ID NO: 1139 - DNA, 25 bp, Artificial Sequence
  >Male | ENST00000481363 | 16920377
gataaacgtggaagggagactgctc

SEQ ID NO: 1140 - DNA, 25 bp, Artificial Sequence
  >Male | ENST00000481363 | 16920377
tcatcatggcagatagcgccggtgc

SEQ ID NO: 1141 - DNA, 25 bp, Artificial Sequence
  >Male | ENST00000481363 | 16920377
cattcgttgggatcagtggtggcct

SEQ ID NO: 1142 - DNA, 25 bp, Artificial Sequence
  >Male | ENST00000481363 | 16920377
tgtcctggaactcggcaaacagctg

SEQ ID NO: 1143 - DNA, 25 bp, Artificial Sequence
  >Male | ENST00000481363 | 16920377
aacctgctgagacatgtggctgccc

SEQ ID NO: 1144 - DNA, 25 bp, Artificial Sequence
  >Male | ENST00000481363 | 16920377
tttaggtacaccacagactccgcat

SEQ ID NO: 1145 - DNA, 25 bp, Artificial Sequence
  >Male | ENST00000481363 | 16920377
gaagtcttctgaaggcacaggcccc

SEQ ID NO: 1146 - DNA, 25 bp, Artificial Sequence
  >Male | ENST00000481363 | 16920377
tacacattgcaactccgaacttggg

SEQ ID NO: 1147 - DNA, 25 bp, Artificial Sequence
  >Male | ENST00000481363 | 16920377
gatgcctggaagtctctcgaagcta

SEQ ID NO: 1148 - DNA, 25 bp, Artificial Sequence
  >Male | ENST00000481363 | 16920377
tcaggtataccccatcatcaagata

SEQ ID NO: 1149 - DNA, 25 bp, Artificial Sequence
  >Male | ENST00000481363 | 16920377
gcatatctcagacccagcagctaag

SEQ ID NO: 1150 - DNA, 25 bp, Artificial Sequence
  >Male | ENST00000481363 | 16920377
cacaagacattcacacgagcataca

SEQ ID NO: 1151 - DNA, 25 bp, Artificial Sequence
  >Male | ENST00000481363 | 16920377
tcacacgagcatacaatgatctagg

SEQ ID NO: 1152 - DNA, 25 bp, Artificial Sequence
  >Male | ENST00000481363 | 16920377
tgactcttaaaacagcagcagctct

SEQ ID NO: 1153 - DNA, 25 bp, Artificial Sequence
  >Male | ENST00000481363 | 16920377
aggccaccactggtaaataccgcaa

SEQ ID NO: 1154 - DNA, 25 bp, Artificial Sequence
  >Male | ENST00000481363 | 16920377
ttaggaagtcggaaatcaaagatgg

SEQ ID NO: 1155 - DNA, 25 bp, Artificial Sequence
  >Male | ENST00000481363 | 16920377
taggaagtcggaaatcaaagatggc

SEQ ID NO: 1156 - DNA, 25 bp, Artificial Sequence
  >Male | ENST00000481363 | 16920377
aaggttagggcgaagatcggcaggc

SEQ ID NO: 1157 - DNA, 25 bp, Artificial Sequence
  >Male | ENST00000481363 | 16920377
tggtcctcctccgagttgatgtgct

SEQ ID NO: 1158 - DNA, 25 bp, Artificial Sequence
  >Male | ENST00000481363 | 16920377
cgggagagccgcagttatttgccct

SEQ ID NO: 1159 - DNA, 25 bp, Artificial Sequence
  >Male | NM_138375 | 16851430
taccctgtcgtttatctcataagca

SEQ ID NO: 1160 - DNA, 25 bp, Artificial Sequence
  >Male | NM_138375 | 16851430
cataaactgggaccaatgtggacag

SEQ ID NO: 1161 - DNA, 25 bp, Artificial Sequence
  >Male | NM_138375 | 16851430
tgagtgaacgagttgaggcgtcccc

SEQ ID NO: 1162 - DNA, 25 bp, Artificial Sequence
  >Male | NM_138375 | 16851430
tgagtcattcaaacaccaggaagaa

SEQ ID NO: 1163 - DNA, 25 bp, Artificial Sequence
  >Male | NM_138375 | 16851430
gaggcttcagaccactccaaactca

SEQ ID NO: 1164 - DNA, 25 bp, Artificial Sequence
  >Male | NM_138375 | 16851430
tatattcttgcatggcagcccctct

SEQ ID NO: 1165 - DNA, 25 bp, Artificial Sequence
  >Male | NM_138375 | 16851430
tccaaggaagatctctgggagatga

SEQ ID NO: 1166 - DNA, 25 bp, Artificial Sequence
  >Male | NM_138375 | 16851430
gggcgttctcctcaatatcttccag

SEQ ID NO: 1167 - DNA, 25 bp, Artificial Sequence
  >Male | NM_138375 | 16851430
gggtgaacctgagagagttcgacat

SEQ ID NO: 1168 - DNA, 25 bp, Artificial Sequence
  >Male | NM_138375 | 16851430
aaattctttggtctgggtgaacctg

SEQ ID NO: 1169 - DNA, 25 bp, Artificial Sequence
  >Male | NM_138375 | 16851430
cattcctggtatcgtgttgccgcat

SEQ ID NO: 1170 - DNA, 25 bp, Artificial Sequence
  >Male | NM_138375 | 16851430
ccattcctggtatcgtgttgccgca

SEQ ID NO: 1171 - DNA, 25 bp, Artificial Sequence
  >Male | NM_138375 | 16851430
cagaaggatcttctgccactgataa

SEQ ID NO: 1172 - DNA, 25 bp, Artificial Sequence
  >Male | NM_138375 | 16851430
acttgggtactgtcgcgatacggca

SEQ ID NO: 1173 - DNA, 25 bp, Artificial Sequence
  >Male | NM_138375 | 16851430
cagttgattgtcttcctccgtccaa

SEQ ID NO: 1174 - DNA, 25 bp, Artificial Sequence
  >Male | NM_138375 | 16851430
tctttcaaactcactgcaccagttg

SEQ ID NO: 1175 - DNA, 25 bp, Artificial Sequence
  >Male | NM_138375 | 16851430
tatttctccgggctccaaaggcatt

SEQ ID NO: 1176 - DNA, 25 bp, Artificial Sequence
  >Male | NM_138375 | 16851430
ctgcggtggctcaggttacggaact

SEQ ID NO: 1177 - DNA, 25 bp, Artificial Sequence
  >Male | NM_138375 | 16851430
ggtcatagtccataaagtctcccag

SEQ ID NO: 1178 - DNA, 25 bp, Artificial Sequence
  >Male | NM_138375 | 16851430
tcagaacgcgtttgtgtttgccaca

SEQ ID NO: 1179 - DNA, 25 bp, Artificial Sequence
  >Male | NM_138375 | 16851430
tgtcagcttaatgtgaggaaacttc

SEQ ID NO: 1180 - DNA, 25 bp, Artificial Sequence
  >Male | NM_138375 | 16851430
aagcttccgcatctctcgtttcaga

SEQ ID NO: 1181 - DNA, 25 bp, Artificial Sequence
  >Male | NM_138375 | 16851430
taacaccgggaattcaaaggcaatc

SEQ ID NO: 1182 - DNA, 25 bp, Artificial Sequence
  >Male | NM_138375 | 16851430
caagtggagggcgaattccaaggcc

SEQ ID NO: 1183 - DNA, 25 bp, Artificial Sequence
  >Male | NM_138375 | 16851430
tcatggacgtgcaaaaggagacctc

SEQ ID NO: 1184 - DNA, 25 bp, Artificial Sequence
  >Male | NM_005035 | 16866470
aaaagagctttatttacacactgac

SEQ ID NO: 1185 - DNA, 25 bp, Artificial Sequence
  >Male | NM_005035 | 16866470
ctggcttgggcaccgcctgcagtgt

SEQ ID NO: 1186 - DNA, 25 bp, Artificial Sequence
  >Male | NM_005035 | 16866470
gagcagaaccgcttgaccaggaatc

SEQ ID NO: 1187 - DNA, 25 bp, Artificial Sequence
  >Male | NM_005035 | 16866470
agaaccgcttgaccaggaatctgga

SEQ ID NO: 1188 - DNA, 25 bp, Artificial Sequence
  >Male | NM_005035 | 16866470
tggttcatgacggagacatcagctg

SEQ ID NO: 1189 - DNA, 25 bp, Artificial Sequence
  >Male | NM_005035 | 16866470
tgcgtgagtccagtaacagtcgtgc

SEQ ID NO: 1190 - DNA, 25 bp, Artificial Sequence
  >Male | NM_005035 | 16866470
gaagccgttcttctgcttacgtgtg

SEQ ID NO: 1191 - DNA, 25 bp, Artificial Sequence
  >Male | NM_005035 | 16866470
tcttctgcttacgtgtgttgggctt

SEQ ID NO: 1192 - DNA, 25 bp, Artificial Sequence
  >Male | NM_005035 | 16866470
accttggagtccaggcgatagggct

SEQ ID NO: 1193 - DNA, 25 bp, Artificial Sequence
  >Male | NM_005035 | 16866470
ccacagagcccatgtgggagatgag

SEQ ID NO: 1194 - DNA, 25 bp, Artificial Sequence
  >Male | NM_005035 | 16866470
gaagacctggcgtacgagatagtga

SEQ ID NO: 1195 - DNA, 25 bp, Artificial Sequence
  >Male | NM_005035 | 16866470
cgtacgagatagtgagaggcctccc

SEQ ID NO: 1196 - DNA, 25 bp, Artificial Sequence
  >Male | NM_005035 | 16866470
caccttgcgggtgatgaaaccttcc

SEQ ID NO: 1197 - DNA, 25 bp, Artificial Sequence
  >Male | NM_005035 | 16866470
cataatgctgcaggccgttgcaaga

SEQ ID NO: 1198 - DNA, 25 bp, Artificial Sequence
  >Male | NM_005035 | 16866470
gattgaccaggtggatcttgagcca

SEQ ID NO: 1199 - DNA, 25 bp, Artificial Sequence
  >Male | NM_005035 | 16866470
gctgagcaggaaagcaccagagtgc

SEQ ID NO: 1200 - DNA, 25 bp, Artificial Sequence
  >Male | NM_005035 | 16866470
cggaaggaatacacgtggtagagca

SEQ ID NO: 1201 - DNA, 25 bp, Artificial Sequence
  >Male | NM_005035 | 16866470
aacgatgcggcttgtccaggctgca

SEQ ID NO: 1202 - DNA, 25 bp, Artificial Sequence
  >Male | NM_005035 | 16866470
gaggtacttcctgtagtggttctgc

SEQ ID NO: 1203 - DNA, 25 bp, Artificial Sequence
  >Male | NM_005035 | 16866470
tacacctcgcgctctaggcggttct

SEQ ID NO: 1204 - DNA, 25 bp, Artificial Sequence
  >Male | NM_005035 | 16866470
catgtggagctgcttctcaaagagg

SEQ ID NO: 1205 - DNA, 25 bp, Artificial Sequence
  >Male | NM_005035 | 16866470
taggacagcaggtccggagtcaagc

SEQ ID NO: 1206 - DNA, 25 bp, Artificial Sequence
  >Male | NM_005035 | 16866470
taacacatataccagctccttgaag

SEQ ID NO: 1207 - DNA, 25 bp, Artificial Sequence
  >Male | NM_005035 | 16866470
gggtccgcttatccttctccagtat

SEQ ID NO: 1208 - DNA, 25 bp, Artificial Sequence
  >Male | NM_005035 | 16866470
tgggtggctggaggctaccatctcc

SEQ ID NO: 1209 - DNA, 25 bp, Artificial Sequence
  >Male | NM_005035 | 16866470
ccgcaaggccgtagggctcgtttga

SEQ ID NO: 1210 - DNA, 25 bp, Artificial Sequence
  >Male | NM_005035 | 16866470
tagggctcgtttgagccccgccgct

SEQ ID NO: 1211 - DNA, 25 bp, Artificial Sequence
  >Male | ENST00000503919 | 17000583
tgttcttcctagatgctgacaagtc

SEQ ID NO: 1212 - DNA, 25 bp, Artificial Sequence
  >Male | ENST00000503919 | 17000583
tgtatcagaccacgctcctctgggc

SEQ ID NO: 1213 - DNA, 25 bp, Artificial Sequence
  >Male | ENST00000503919 | 17000583
tcaagtatgaaagcaaggcacccgc

SEQ ID NO: 1214 - DNA, 25 bp, Artificial Sequence
  >Male | ENST00000503919 | 17000583
acaaacatctccgtggtcagcagca

SEQ ID NO: 1215 - DNA, 25 bp, Artificial Sequence
  >Male | ENST00000503919 | 17000583
tattgatggcgccagggttggactc

SEQ ID NO: 1216 - DNA, 25 bp, Artificial Sequence
  >Male | ENST00000503919 | 17000583
agaagagggccgtgaacttgccgat

SEQ ID NO: 1217 - DNA, 25 bp, Artificial Sequence
  >Male | ENST00000503919 | 17000583
aggaccagcatgatagccgcaccat

SEQ ID NO: 1218 - DNA, 25 bp, Artificial Sequence
  >Male | ENST00000503919 | 17000583
taattcccaggacgccaatgttggg

SEQ ID NO: 1219 - DNA, 25 bp, Artificial Sequence
  >Male | ENST00000503919 | 17000583
tagccccgcgatgatgcagcaaatg

SEQ ID NO: 1220 - DNA, 25 bp, Artificial Sequence
  >Male | ENST00000503919 | 17000583
ctcaatgatgcctgccagagtggcg

SEQ ID NO: 1221 - DNA, 25 bp, Artificial Sequence
  >Male | ENST00000503919 | 17000583
caaggtcaggacatagcagagcagc

SEQ ID NO: 1222 - DNA, 25 bp, Artificial Sequence
  >Male | ENST00000503919 | 17000583
ggaggtctctgtccaggctaacctg

SEQ ID NO: 1223 - DNA, 25 bp, Artificial Sequence
  >Male | ENST00000503919 | 17000583
agtgaggcccttgccccagcggtag

SEQ ID NO: 1224 - DNA, 25 bp, Artificial Sequence
  >Male | ENST00000503919 | 17000583
gaaggtgaggttgcgcaggtactgg

SEQ ID NO: 1225 - DNA, 25 bp, Artificial Sequence
  >Male | ENST00000503919 | 17000583
ccgggaagaaggaccaaggacatga

SEQ ID NO: 1226 - DNA, 25 bp, Artificial Sequence
  >Male | ENST00000503919 | 17000583
aaggaccaaggacatgaagagggta

SEQ ID NO: 1227 - DNA, 25 bp, Artificial Sequence
  >Male | ENST00000503919 | 17000583
gctcggtcgccagcagcttggaaga

SEQ ID NO: 1228 - DNA, 25 bp, Artificial Sequence
  >Male | ENST00000503919 | 17000583
ccgtatccgtgggtgccaaatatga

SEQ ID NO: 1229 - DNA, 25 bp, Artificial Sequence
  >Male | ENST00000503919 | 17000583
gggcagactccagttaccgtagatc

SEQ ID NO: 1230 - DNA, 25 bp, Artificial Sequence
  >Male | ENST00000503919 | 17000583
tagagtcagggatacacacacggac

SEQ ID NO: 1231 - DNA, 25 bp, Artificial Sequence
  >Male | ENST00000503919 | 17000583
acggaccaggtacagagacagagag

SEQ ID NO: 1232 - DNA, 25 bp, Artificial Sequence
  >Male | ENST00000503919 | 17000583
taaccatgtgctggtcgtggcccac

SEQ ID NO: 1233 - DNA, 25 bp, Artificial Sequence
  >Male | ENST00000503919 | 17000583
ggcacggcgatggtaccactgaagc

SEQ ID NO: 1234 - DNA, 25 bp, Artificial Sequence
  >Male | ENST00000503919 | 17000583
caagggattcccagagagctactgc

SEQ ID NO: 1235 - DNA, 25 bp, Artificial Sequence
  >Male | ENST00000503919 | 17000583
caagatattcctgcggcttccgtgg

SEQ ID NO: 1236 - DNA, 25 bp, Artificial Sequence
  >Male | ENST00000503919 | 17000583
cacaggtaccaaggtggcacgtcct

SEQ ID NO: 1237 - DNA, 25 bp, Artificial Sequence
  >Male | ENST00000503919 | 17000583
caaacttaggctctgtgggtagcgg

SEQ ID NO: 1238 - DNA, 25 bp, Artificial Sequence
  >Male | ENST00000503919 | 17000583
gatgacttgacaaaggccaaggagg

SEQ ID NO: 1239 - DNA, 25 bp, Artificial Sequence
  >Male | ENST00000503919 | 17000583
ccaaggaggaggactttactccaca

SEQ ID NO: 1240 - DNA, 25 bp, Artificial Sequence
  >Male | ENST00000503919 | 17000583
tactgctcccaatttccaaagttgc

SEQ ID NO: 1241 - DNA, 25 bp, Artificial Sequence
  >Male | NM_024807 | 17019044
tatacaacaggatggtggctacacc

SEQ ID NO: 1242 - DNA, 25 bp, Artificial Sequence
  >Male | NM_024807 | 17019044
agctttctaaggaggcagcggccag

SEQ ID NO: 1243 - DNA, 25 bp, Artificial Sequence
  >Male | NM_024807 | 17019044
tcttccaggtgggtcacgtgtagaa

SEQ ID NO: 1244 - DNA, 25 bp, Artificial Sequence
  >Male | NM_024807 | 17019044
ggtcacgtgtagaaggatcgctgca

SEQ ID NO: 1245 - DNA, 25 bp, Artificial Sequence
  >Male | NM_024807 | 17019044
gaaggatcgctgcacatgctgtagc

SEQ ID NO: 1246 - DNA, 25 bp, Artificial Sequence
  >Male | NM_024807 | 17019044
acccatagaccatgatcagcatcag

SEQ ID NO: 1247 - DNA, 25 bp, Artificial Sequence
  >Male | NM_024807 | 17019044
caagcacagtggagtaaacatcctg

SEQ ID NO: 1248 - DNA, 25 bp, Artificial Sequence
  >Male | NM_024807 | 17019044
cacagtggagtaaacatcctggtgc

SEQ ID NO: 1249 - DNA, 25 bp, Artificial Sequence
  >Male | NM_024807 | 17019044
tgctgaggtccccagacttagtgga

SEQ ID NO: 1250 - DNA, 25 bp, Artificial Sequence
  >Male | NM_024807 | 17019044
gagcctaggcaaggtgatgagtcct

SEQ ID NO: 1251 - DNA, 25 bp, Artificial Sequence
  >Male | NM_024807 | 17019044
tttcacccagactcgggcaaagcca

SEQ ID NO: 1252 - DNA, 25 bp, Artificial Sequence
  >Male | NM_024807 | 17019044
tccccttcaaggagcctcacttttg

SEQ ID NO: 1253 - DNA, 25 bp, Artificial Sequence
  >Male | NM_024807 | 17019044
tttgtgtatacactgtcagcagagg

SEQ ID NO: 1254 - DNA, 25 bp, Artificial Sequence
  >Male | NM_024807 | 17019044
ttgtgtatacactgtcagcagaggg

SEQ ID NO: 1255 - DNA, 25 bp, Artificial Sequence
  >Male | NM_024807 | 17019044
tgagacgcaaccctgtggccacagc

SEQ ID NO: 1256 - DNA, 25 bp, Artificial Sequence
  >Male | NM_024807 | 17019044
gacacaggatgtgccacctgggcct

SEQ ID NO: 1257 - DNA, 25 bp, Artificial Sequence
  >Male | NR_003697 | 17057414
tagggccagaggtctgtctgccaga

SEQ ID NO: 1258 - DNA, 25 bp, Artificial Sequence
  >Male | NR_003697 | 17057414
cttccagaagggcaacaagcgaggt

SEQ ID NO: 1259 - DNA, 25 bp, Artificial Sequence
  >Male | NR_003697 | 17057414
ggttccaaggaacagcctggcagcc

SEQ ID NO: 1260 - DNA, 25 bp, Artificial Sequence
  >Male | NR_003697 | 17057414
ctggcagccactgaaggtatcttct

SEQ ID NO: 1261 - DNA, 25 bp, Artificial Sequence
  >Male | NR_003697 | 17057414
gaaacactgacggatggcaggcact

SEQ ID NO: 1262 - DNA, 25 bp, Artificial Sequence
  >Male | NR_003697 | 17057414
cggtcgcctcccagtttcatggaca

SEQ ID NO: 1263 - DNA, 25 bp, Artificial Sequence
  >Male | NR_003697 | 17057414
ctggtagaaaatacaaaattcctcg

SEQ ID NO: 1264 - DNA, 25 bp, Artificial Sequence
  >Male | NR_003697 | 17057414
ctcgattagggacaagggaccactg

SEQ ID NO: 1265 - DNA, 25 bp, Artificial Sequence
  >Male | NR_003697 | 17057414
tcaaaacaatagcaatagccagagc

SEQ ID NO: 1266 - DNA, 25 bp, Artificial Sequence
  >Male | NR_003697 | 17057414
gcaatagccagagcatcagcatttt

SEQ ID NO: 1267 - DNA, 25 bp, Artificial Sequence
  >Male | NR_003697 | 17057414
gagccattggactactacaagaaag

SEQ ID NO: 1268 - DNA, 25 bp, Artificial Sequence
  >Male | NR_003697 | 17057414
gactactacaagaaaggagcgcagg

SEQ ID NO: 1269 - DNA, 25 bp, Artificial Sequence
  >Male | NR_003697 | 17057414
gagcgcaggactctaccctttcaca

SEQ ID NO: 1270 - DNA, 25 bp, Artificial Sequence
  >Male | NR_003697 | 17057414
aacgcacagcaagaatgcctgccct

SEQ ID NO: 1271 - DNA, 25 bp, Artificial Sequence
  >Male | NR_003697 | 17057414
gagttgctgtgacagtaagctcttc

SEQ ID NO: 1272 - DNA, 25 bp, Artificial Sequence
  >Male | NR_003697 | 17057414
ttccactttgagaccgtcacctcag

SEQ ID NO: 1273 - DNA, 25 bp, Artificial Sequence
  >Male | NR_003697 | 17057414
tttgagaccgtcacctcagccacgg

SEQ ID NO: 1274 - DNA, 25 bp, Artificial Sequence
  >Male | NR_003697 | 17057414
ggtggatgactagactgccgaagac

SEQ ID NO: 1275 - DNA, 25 bp, Artificial Sequence
  >Male | NR_003697 | 17057414
tggatgactagactgccgaagaccg

SEQ ID NO: 1276 - DNA, 25 bp, Artificial Sequence
  >Male | NR_003697 | 17057414
cgctgcgactacgaagtacggagta

SEQ ID NO: 1277 - DNA, 25 bp, Artificial Sequence
  >Male | NM_000786 | 17059640
ttaggccccgagttacaatttgaga

SEQ ID NO: 1278 - DNA, 25 bp, Artificial Sequence
  >Male | NM_000786 | 17059640
tatttggcaagagcgatgagtactc

SEQ ID NO: 1279 - DNA, 25 bp, Artificial Sequence
  >Male | NM_000786 | 17059640
cattttgatcttcgtttgtaacgga

SEQ ID NO: 1280 - DNA, 25 bp, Artificial Sequence
  >Male | NM_000786 | 17059640
ttttccccaatacaacgatgacgcc

SEQ ID NO: 1281 - DNA, 25 bp, Artificial Sequence
  >Male | NM_000786 | 17059640
gctccaaatggcacataggcaaact

SEQ ID NO: 1282 - DNA, 25 bp, Artificial Sequence
  >Male | NM_000786 | 17059640
taagtctttgattgacagtgggaga

SEQ ID NO: 1283 - DNA, 25 bp, Artificial Sequence
  >Male | NM_000786 | 17059640
taaaaactggctagataataggcaa

SEQ ID NO: 1284 - DNA, 25 bp, Artificial Sequence
  >Male | NM_000786 | 17059640
ggagttctggccattctcatcatga

SEQ ID NO: 1285 - DNA, 25 bp, Artificial Sequence
  >Male | NM_000786 | 17059640
tctctggccaaaaagaagcccatcc

SEQ ID NO: 1286 - DNA, 25 bp, Artificial Sequence
  >Male | NM_000786 | 17059640
gaggatgtatgctgccctgccaaga

SEQ ID NO: 1287 - DNA, 25 bp, Artificial Sequence
  >Male | NM_000786 | 17059640
tatccttgatttcccgatgagctct

SEQ ID NO: 1288 - DNA, 25 bp, Artificial Sequence
  >Male | NM_000786 | 17059640
caatggctagctgttaaaattatga

SEQ ID NO: 1289 - DNA, 25 bp, Artificial Sequence
  >Male | NM_000786 | 17059640
ttaaagtgggctatgttaaggccac

SEQ ID NO: 1290 - DNA, 25 bp, Artificial Sequence
  >Male | NM_000786 | 17059640
agtgcagcagcatcactccccagaa

SEQ ID NO: 1291 - DNA, 25 bp, Artificial Sequence
  >Male | NM_000786 | 17059640
gtgcagcagcatcactccccagaag

SEQ ID NO: 1292 - DNA, 25 bp, Artificial Sequence
  >Male | NM_000786 | 17059640
tctagaaattcaattggacttttcc

SEQ ID NO: 1293 - DNA, 25 bp, Artificial Sequence
  >Male | NM_000786 | 17059640
aatgctatggcatgcccaaggaatg

SEQ ID NO: 1294 - DNA, 25 bp, Artificial Sequence
  >Male | NM_000786 | 17059640
gcatggacaagaggttgccgcctgt

SEQ ID NO: 1295 - DNA, 25 bp, Artificial Sequence
  >Male | NM_000786 | 17059640
catggacaagaggttgccgcctgtc

SEQ ID NO: 1296 - DNA, 25 bp, Artificial Sequence
  >Male | NM_000786 | 17059640
ggaaacactgaaggccgaggtcgcc

SEQ ID NO: 1297 - DNA, 25 bp, Artificial Sequence
  >Male | NM_000786 | 17059640
aatcgacggaacgagagaagctggc

SEQ ID NO: 1298 - DNA, 25 bp, Artificial Sequence
  >Male | NM_000786 | 17059640
tgaagaggcgatcaatccctgagaa

SEQ ID NO: 1299 - DNA, 25 bp, Artificial Sequence
  >Male | NM_000786 | 17059640
gatcaatccctgagaatcgcgggcg

SEQ ID NO: 1300 - DNA, 25 bp, Artificial Sequence
  >Male | ExonID_5299845 | 17076434
cagggacctgaatgcaaaactagcc

SEQ ID NO: 1301 - DNA, 25 bp, Artificial Sequence
  >Male | ExonID_5299845 | 17076434
gaggtcaccttcaatcgaggcacga

SEQ ID NO: 1302 - DNA, 25 bp, Artificial Sequence
  >Male | ExonID_5299845 | 17076434
ggctcatgagagaagacggaatcct

SEQ ID NO: 1303 - DNA, 25 bp, Artificial Sequence
  >Male | ExonID_5299845 | 17076434
ttgaaaagttcctccacaggcacac

SEQ ID NO: 1304 - DNA, 25 bp, Artificial Sequence
  >Male | ExonID_5299845 | 17076434
catactccacgatgacatacaaggg

SEQ ID NO: 1305 - DNA, 25 bp, Artificial Sequence
  >Male | ExonID_5299845 | 17076434
tctgagatcaggtctgacaagtctt

SEQ ID NO: 1306 - DNA, 25 bp, Artificial Sequence
  >Male | ExonID_5299845 | 17076434
tgagactcatttacttgggaaggga

SEQ ID NO: 1307 - DNA, 25 bp, Artificial Sequence
  >Male | ExonID_5299845 | 17076434
tagtcagggcttcccaacaatggca

SEQ ID NO: 1308 - DNA, 25 bp, Artificial Sequence
  >Male | ExonID_5299845 | 17076434
gaaggcccctgtgcaatagatgatg

SEQ ID NO: 1309 - DNA, 25 bp, Artificial Sequence
  >Male | ExonID_5299845 | 17076434
tgcaagggccagctgagaagtcact

SEQ ID NO: 1310 - DNA, 25 bp, Artificial Sequence
  >Male | ExonID_5299845 | 17076434
caggacatcgagaggagaagttaca

SEQ ID NO: 1311 - DNA, 25 bp, Artificial Sequence
  >Male | ExonID_5299845 | 17076434
gagtccgatagagttacccgccaag

SEQ ID NO: 1312 - DNA, 25 bp, Artificial Sequence
  >Male | ExonID_5299845 | 17076434
tctaagagacgcagagcaagggaag

SEQ ID NO: 1313 - DNA, 25 bp, Artificial Sequence
  >Male | ExonID_5299845 | 17076434
catggatccacacaaagccaaggaa

SEQ ID NO: 1314 - DNA, 25 bp, Artificial Sequence
  >Male | ExonID_5299845 | 17076434
cgcatccgagctattaatccccgaa

SEQ ID NO: 1315 - DNA, 25 bp, Artificial Sequence
  >Male | ExonID_5299845 | 17076434
gatcgtacgtaactcaggacacagg

SEQ ID NO: 1316 - DNA, 25 bp, Artificial Sequence
  >Male | ExonID_5299845 | 17076434
atgaactccacgttgctacccaggg

SEQ ID NO: 1317 - DNA, 25 bp, Artificial Sequence
  >Male | ExonID_5299845 | 17076434
catttttcaaccagcgcagtgtggg

SEQ ID NO: 1318 - DNA, 25 bp, Artificial Sequence
  >Male | ExonID_5299845 | 17076434
acttagcagaacaggcaccgtgacc

SEQ ID NO: 1319 - DNA, 25 bp, Artificial Sequence
  >Male | ExonID_5299845 | 17076434
ttaatcagagcagatagggcaccca

SEQ ID NO: 1320 - DNA, 25 bp, Artificial Sequence
  >Male | ExonID_5299845 | 17076434
gagcagggataccaccacctgttca

SEQ ID NO: 1321 - DNA, 25 bp, Artificial Sequence
  >Male | ExonID_5299845 | 17076434
taagccgagtaccaagtccaaatgg

SEQ ID NO: 1322 - DNA, 25 bp, Artificial Sequence
  >Male | ExonID_5299845 | 17076434
cacctccgaggtgtgtcctggaagc

SEQ ID NO: 1323 - DNA, 25 bp, Artificial Sequence
  >Male | ExonID_5299845 | 17076434
tgctggttacgcaagcatagaggcc

SEQ ID NO: 1324 - DNA, 25 bp, Artificial Sequence
  >Male | ExonID_5299845 | 17076434
gactatattaggacgggaggccaca

SEQ ID NO: 1325 - DNA, 25 bp, Artificial Sequence
  >Male | ExonID_5299845 | 17076434
agaagcatctcaccgaaatcccggg

SEQ ID NO: 1326 - DNA, 25 bp, Artificial Sequence
  >Male | ExonID_5299845 | 17076434
gacggcctagcggtgcagagtgtgg

SEQ ID NO: 1327 - DNA, 25 bp, Artificial Sequence
  >Male | ExonID_5299845 | 17076434
tagaggttggtgacaaggctccaca

SEQ ID NO: 1328 - DNA, 25 bp, Artificial Sequence
  >Male | ExonID_5299845 | 17076434
aaagagcctaagagtgtggagccag

SEQ ID NO: 1329 - DNA, 25 bp, Artificial Sequence
  >Male | ExonID_5299845 | 17076434
tactgatccaacatacagggtggac

SEQ ID NO: 1330 - DNA, 25 bp, Artificial Sequence
  >Male | ExonID_5299845 | 17076434
tctatttctatagggcgccacagct

SEQ ID NO: 1331 - DNA, 25 bp, Artificial Sequence
  >Male | ExonID_5299845 | 17076434
taaacaagtcattagggaggcaggc

SEQ ID NO: 1332 - DNA, 25 bp, Artificial Sequence
  >Male | ExonID_5299845 | 17076434
gatgcggcccaaatcagtccttaaa

SEQ ID NO: 1333 - DNA, 25 bp, Artificial Sequence
  >Male | ExonID_5299845 | 17076434
cggcggcgaataacttggtgagatc

SEQ ID NO: 1334 - DNA, 25 bp, Artificial Sequence
  >Male | ExonID_5299845 | 17076434
ctcccgagcgcgagttggaggaaaa

SEQ ID NO: 1335 - DNA, 25 bp, Artificial Sequence
  >Male | ExonID_5299845 | 17076434
agctcggaccggagaaaagtccttg

SEQ ID NO: 1336 - DNA, 25 bp, Artificial Sequence
  >Male | TCONS_00017554-XLOC_008249 | 17114699
cattccatacacacaaacattccat

SEQ ID NO: 1337 - DNA, 25 bp, Artificial Sequence
  >Male | TCONS_00017554-XLOC_008249 | 17114699
attccatacacacaaacattccata

SEQ ID NO: 1338 - DNA, 25 bp, Artificial Sequence
  >Male | TCONS_00017554-XLOC_008249 | 17114699
ttccatacacacaaacattccatac

SEQ ID NO: 1339 - DNA, 25 bp, Artificial Sequence
  >Male | TCONS_00017554-XLOC_008249 | 17114699
tccatacacacaaacattccataca

SEQ ID NO: 1340 - DNA, 25 bp, Artificial Sequence
  >Male | TCONS_00017554-XLOC_008249 | 17114699
tacacacaaacattccatacacaca

SEQ ID NO: 1341 - DNA, 25 bp, Artificial Sequence
  >Male | TCONS_00017554-XLOC_008249 | 17114699
tacacacacatattccatacacaca

SEQ ID NO: 1342 - DNA, 25 bp, Artificial Sequence
  >Male | TCONS_00017554-XLOC_008249 | 17114699
atattccatacacacacattccata

SEQ ID NO: 1343 - DNA, 25 bp, Artificial Sequence
  >Male | TCONS_00017554-XLOC_008249 | 17114699
catacacagacacattctgtacaca

SEQ ID NO: 1344 - DNA, 25 bp, Artificial Sequence
  >Male | TCONS_00017554-XLOC_008249 | 17114699
agacacattctgtacacacagacac

SEQ ID NO: 1345 - DNA, 25 bp, Artificial Sequence
  >Male | TCONS_00017554-XLOC_008249 | 17114699
gacacattctgtacacacagacaca

SEQ ID NO: 1346 - DNA, 25 bp, Artificial Sequence
  >Male | TCONS_00017554-XLOC_008249 | 17114699
acagacacacattccatacacagac

SEQ ID NO: 1347 - DNA, 25 bp, Artificial Sequence
  >Male | TCONS_00017554-XLOC_008249 | 17114699
cacacattccatacacagacacatt

SEQ ID NO: 1348 - DNA, 25 bp, Artificial Sequence
  >Male | TCONS_00017554-XLOC_008249 | 17114699
acacattccatacacagacacattc